European Patent Specification EP 3 596 234 B1, published August 16, 2023. Title: METHODS FOR IDENTIFYING AND MONITORING PREGNANT WOMEN AT RISK OF PREECLAMPSIA. Applicant: Ramot at Tel-Aviv University Ltd. Mor Research Applications Ltd. The sequence listing filed with the application follows.

SEQUENCE LISTING (25 sequences)

SEQ ID NO: 1 - DNA, 68 bp, Homo sapiens
cagagaatagtttaaattagaatcttagctttgggtgctaatggtggagttaaagactttttctctga

SEQ ID NO: 2 - DNA, 70 bp, Homo sapiens
cactgtaaagctaacttagcattaaccttttaagttaaagattaagagaaccaacacctctttacagtga

SEQ ID NO: 3 - DNA, 112 bp, Homo sapiens
gctgcttgcctccccccgtttttggcaatggtagaactcacactggtgaggtaacaggatccggtggttctagacttgccaactatggggcgaggactcagccggcaccctg

SEQ ID NO: 4 - DNA, 110 bp, Homo sapiens
ccagaggttgtaacgttgtctatatataccctgtagaaccgaatttgtgtggtatccgtatagtcacagattcgattctaggggaatatatggtcgatgcaaaaacttca

SEQ ID NO: 5 - DNA, 12667 bp, Homo sapiens
caacccacaccgcccctgccagccaccatggggctgccactagcccgcctggcggctgtgtgcctggccctgtctttggcagggggctcggagctccagacagagggcagaacccgaaaccacggccacaacgtctgcagcacctggggcaacttccactacaagaccttcgacggggacgtcttccgcttccccggcccctgcgactacaacttcgcctccgactgccgaggctcctacaaggaatttgctgtgcacctgaagcggggtccgggccaggctgaggcccccgccggggtggagtccatcctgctgaccatcaaggatgacaccatctacctcacccgccacctggctgtgcttaacggggccgtggtcagcaccccgcactacagccccgggctgctcattgagaagagcgatgcctacaccaaagtctactcccgcgccggcctcaccctcatgtggaaccgggaggatgcactcatgctggagctggacactaagttccggaaccacacctgtggcctctgcggggactacaacggcctgcagagctattcagaattcctctctgacggcgtgctcttcagtcccctggagtttgggaacatgcagaagatcaaccagcccgatgtggtgtgtgaggatcccgaggaggaggtggcccccgcatcctgctccgagcaccgcgccgagtgtgagaggctgctgaccgccgaggccttcgcggactgtcaggacctggtgccgctggagccgtatctgcgcgcctgccagcaggaccgctgccggtgcccgggcggtgacacctgcgtctgcagcaccgtggccgagttctcccgccagtgctcccacgccggcggccggcccgggaactggaggaccgccacgctctgccccaagacctgccccgggaacctggtgtacctggagagcggctcgccctgcatggacacctgctcacacctggaggtgagcagcctgtgcgaggagcaccgcatggacggctgtttctgcccagaaggcaccgtatatgacgacatcggggacagtggctgcgttcctgtgagccagtgccactgcaggctgcacggacacctgtacacaccgggccaggagatcaccaatgactgcgagcagtgtgtctgtaacgctggccgctgggtgtgcaaagacctgccctgccccggcacctgtgccctggaaggcggctcccacatcaccaccttcgatgggaagacgtacaccttccacggggactgctactatgtcctggccaagggtgaccacaacgattcctacgctctcctgggcgagctggccccctgtggctccacagacaagcagacctgcctgaagacggtggtgctgctggctgacaagaagaagaatgtggtggtcttcaagtccgatggcagtgtactgctcaacgagctgcaggtgaacctgccccacgtgaccgcgagcttctctgtcttccgcccgtcttcctaccacatcatggtgagcatggccattggcgtccggctgcaggtgcagctggccccagtcatgcaactctttgtgacactggaccaggcctcccaggggcaggtgcagggcctctgcgggaacttcaacggcctggaaggtgacgacttcaagacggccagcgggctggtggaggccacgggggccggctttgccaacacctggaaggcacagtcaacctgccatgacaagctggactggttggacgatccctgctccctgaacatcgagagcgccaactacgccgagcactggtgctccctcctgaagaagacagagaccccctttggcaggtgccactcggctgtggaccctgctgagtattacaagaggtgcaaatatgacacgtgtaactgtcagaacaatgaggactgcctgtgcgccgccctgtcctcctacgcgcgcgcctgcaccgccaagggcgtcatgctgtggggctggcgggagcatgtctgcaacaaggatgtgggctcctgccccaactcgcaggtcttcctgtacaacctgaccacctgccagcagacctgccgctccctctccgaggccgacagccactgtctcgagggctttgcgcctgtggacggctgcggctgccctgaccacaccttcctggacgagaagggccgctgcgtacccctggccaagtgctcctgttaccaccgcggtctctacctggaggcgggggacgtggtcgtcaggcaggaagaacgatgtgtgtgccgggatgggcggctgcactgtaggcagatccggctgatcggccagagctgcacggccccaaagatccacatggactgcagcaacctgactgcactggccacctcgaagccccgagccctcagctgccagacgctggccgccggctattaccacacagagtgtgtcagtggctgtgtgtgccccgacgggctgatggatgacggccggggtggctgcgtggtggagaaggaatgcccttgcgtccataacaacgacctgtattcttccggcgccaagatcaaggtggactgcaatacctgcacctgcaagagaggacgctgggtgtgcacccaggctgtgtgccatggcacctgctccatttacgggagtggccactacatcacctttgacgggaagtactacgactttgacggacactgctcctacgtggctgttcaggactactgcggccagaactcctcactgggctcattcagcatcatcaccgagaacgtcccctgtggcactacgggcgtcacctgctccaaggccatcaagatcttcatggggaggacggagctgaagttggaagacaagcaccgtgtggtgatccagcgtgatgagggtcaccacgtggcctacaccacgcgggaggtgggccagtacctggtggtggagtccagcacgggcatcatcgtcatctgggacaagaggaccaccgtgttcatcaagctggctccctcctacaagggcaccgtgtgtggcctgtgtgggaactttgaccaccgctccaacaacgacttcaccacgcgggaccacatggtggtgagcagcgagctggacttcgggaacagctggaaggaggcccccacctgcccagatgtgagcaccaaccccgagccctgcagcctgaacccgcaccgccgctcctgggccgagaagcagtgcagcatcctcaaaagcagcgtgttcagcatctgccacagcaaggtggaccccaagcccttctacgaggcctgtgtgcacgactcgtgctcctgtgacacgggtggggactgtgagtgcttctgctctgccgtggcctcctacgcccaggagtgtaccaaagagggggcctgcgtgttctggaggacgccggacctgtgccccatattctgcgactactacaaccctccgcatgagtgtgagtggcactatgagccatgtgggaaccggagcttcgagacctgcaggaccatcaatggcatccactccaacatctccgtgtcctacctggagggctgctacccccggtgccccaaggacaggcccatctatgaggaggatctgaagaagtgtgtcactgcagacaagtgtggctgctatgtcgaggacacccactacccacctggagcatcggttcccaccgaggagacctgcaagtcctgcgtgtgtaccaactcctcccaagtcgtctgcaggccggaggaaggaaagattcttaaccagacccaggatggcgccttctgctactgggagatctgtggccccaacgggacggtggagaagcacttcaacatctgttccattacgacacgcccgtccaccctgaccaccttcaccaccatcaccctccccaccacccccaccaccttcaccactaccaccaccaccaccaccccgacctccagcacagttttatcaacaactccgaagctgtgctgcctctggtctgactggatcaatgaggaccaccccagcagtggcagcgacgacggtgaccgagaaacatttgatggggtctgcggggcccctgaggacatcgagtgcaggtcggtcaaggatccccacctcagcttggagcagctaggccagaaggtgcagtgtgatgtctctgttgggttcatttgcaagaatgaagaccagtttggaaatggaccatttggactgtgttacgactacaagatacgtgtcaattgttgctggcccatggataagtgtatcaccactcccagccctccaactaccactcccagccctccaccaaccagcacgaccacccttccaccaaccaccacccccagccctccaaccaccaccacaaccacccctccaccaaccaccacccccagccctccaataaccaccacgaccacccctccaccaaccaccactcccagccctccaataagcaccacaaccacccctccaccaaccaccactcccagccctccaaccaccactcccagccctccaaccaccactcccagccctccaacaaccaccacaaccacccctccaccaaccaccactcccagccctccaacgactacgcccatcactccaccagccagcactaccacccttccaccaaccaccactcccagccctccaacaaccaccacaaccacccctccaccaaccaccactcccagtcctccaacgactacgcccatcactccaccaaccagcactactacccttccaccaaccaccactcccagccctccaccaaccaccacaaccacccctccaccaaccaccactcccagccctccaacaaccaccactcccagtcctccaacaatcaccacaaccacccctccaccaaccaccactcccagccctccaacaaccaccacgaccacccttccaccaaccaccacttccagccctctaacaactactcctctacctccatcaataactcctcctacattttcaccattctcaacgacaacccctactaccccatgcgtgcctctctgcaattggactggctggctggattctggaaaacccaactttcacaaaccaggtggagacacagaattgattggagacgtctgtggaccaggctgggcagctaacatctcttgcagagccaccatgtatcctgatgttcccattggacagcttggacaaacagtggtgtgtgatgtctctgtggggctgatatgcaaaaatgaagaccaaaagccaggtggggtcatccctatggccttctgcctcaactacgagatcaacgttcagtgctgtgagtgtgtcacccaacccaccaccatgacaaccaccaccacagagaacccaactccgacaccaatcaccaccaccactacggtgaccccaaccccaacacccaccagcacacagagtacaacaccaacacccatcaccaccaccaatacggtaaccccaaccccaacccccactggcacacagaccccaaccccgacacccatcaccaccaccaccactatggtgaccccaacaccaacaatcaccagcacacagaccccaaccccgacacccatcaccaccactacggtgaccccaaccccaacacccaccagcacacagagaacaacaccgacatccatcaccaccaccaccacggtgaccccaaccccaacacccaccggcacacagaccccaaccacgacacccatcaccaccaccaccacggtgaccccaaccccaacacccaccggcacacagaccccaacaacgacacccatcaccaccaccaccatggtgaccccaaccccaacacccactggaacacagacccaaaccccaacacccatcaccaccaccactacggtgaccccaacccctacacccaccggcacacagaccccaacatcgacacccatcagcaccaccactacggtgaccccaacaccaacacccaccggcacacagaccccaaccctgacacccatcaccaccaccactacggtgaccccaaccccaacacccaccggcacacagaccccaaccacgacacccatcaccaccaccactacggtgaccccaaccccaacacccaccggcacaaagagtacaaccccgacatccatcaccaccaccactatggtgaccccaaccccaccacccactggcacacagaccccaaccacgacacccatcaccaccaccactacggtgaccccaaccccaacacccaccggcacacagaccccaaccccgacacccatcaccaccaccaccacggtgaccccaaccccaacacccaccggcacacagaccccaacatcgacacccatcaccaccaacactacggtgaccccaaccccaacaccaaccggcacaccgagtacaaccctgacacccatcaccaccaccactatggtgaccccaaccccaacacccaccggcacacagaccccaacatcgacacccatcagcaccaccactacggtgaccccaacctcaacacccaccggcacacagaccccaaccccgacacccatctccaccaccactacggtgaccccaaccccgacacccatctccaccaccactacagtgaccccaaccccaacacccaccggcacacagaccccaaccatgacacccatcaccaccaccaccacggtgaccccaaccccaacacccaccggcacacagaccccaacaacgacacccatcagcaccaccaccacagtgaccccaaccccaacacccaccggcacacagaccccaacatcgacacccatcaccaccaccactacggtgaccccaaccccaacacccaccggcacacagaccccaaccacgacacccatcaccaccaccaccacggtgaccccaaccccaacacccaccggcacacagagtacaaccctgacacccatcaccaccaccaccacggtgacaccaaccccaacacccaccggcacacagaccccaaccccgacacccatctccaccaccactacggtgaccccaaccccaacacccaccggcacacagaccccaaccacgacacccatcaccaccaccaccacggtgaccccaaccccaacacccaccggcacacagaccccaacaacgacacccatcagcaccaccaccacggtgaccccaaccccaacacccaccggcacacagaccccaacatcgacacccatcaccaccaccactacggtgaccccaaccccaacacccaccggcacacagaccccaaccacgacacccatcaccaccaccaccacggtgaccccaaccccaacacccactggcacacaggccccaaccccaacagccatcaccaccaccactacggtgaccccaaccccaacacccaccggcacacagaccccaacaacgacacccatcaccaccaccaccatggtgaccccaaccccaacacccaccggcacacagaccccaacatcgacacccatcaccaccaccactacggtgaccccaaccccaacacccaccggcacacagaccccaaccccgacacccatctccaccaccactacggtgaccccaaccccaacacccaccggcacacagaccccaaccatgacacccatcaccaccaccaccacggtgaccccaaccccaacacccaccggcacacagaccccaacaacgacacccatcagcaccaccaccacggtgaccccaaccccaacacccaccggcacacagaccccaacatcgacacccatcaccaccaccactacggtgaccccaaccccaacacccaccggcacacagaccccaaccccgacacccatcaccaccaccaccacggtgaccccaaccccaacacccaccggcacacagaccccaacatcgacacccatcaccaccaccactacggtgaccccaaccccaacacccaccggcacacagaccccaaccacgacacccatcaccaccaccaccacggtgaccccaaccccaacacccaccggcacacagagtacaaccctgacacccatcaccaccaccaccacggtgaacaccaacccccaacacccaccggcacacaaaaccccaacatcaacacccatcaccacccaccactacggttgaccccaacccccaaaacccaccggcacacagaccccaaccccaacacccattctccaccaccaataacgggtgaccccaaccccaacaacccaccggcacacagaccccaaccatgacacccatcaccaccaccaccacggtgaccccaaccccaacacccaccggcacacagaccccaacatcgacacccatcaccaccaccactacggtgaccccaaccccaacacccaccggcacacagaccccaaccatgacacccatcaccaccaccaccacggtgaccccaaccccaacacccactggcacacaggccccaaccccaacagccatcaccaccaccactacggtgaccccaaccccaacacccaccggcacacagaccccaaccacgacacccatcaccaccaccaccacggtgaccccaaccccaacacccaccggcacacagagtacaaccctgacacccatcaccaccaccaccacggtgacaccaaccccaacacccaccggcacacagaccccaaccccgacacccatctccaccaccactacggtgaccccaaccccaacacccaccggcacacagaccccaaccatgacacccatcaccaccaccaccacggtgaccccaaccccaacacccaccggcacacagaccccaacaacgacacccatcagcaccaccaccacggtgaccccaaccccaacacccaccggcacacagaccccaacatcgacacccatcaccaccaccactacggtgaccccaaccccaacacccaccggcacacagaccccaaccacgacacccatcaccaccaccaccacggtgaccccaaccccaacacccactggcacacaggccccaaccccaacagccatcaccaccaccagtacggtgaccccaaccccaacacccaccggcacacagaccccaaccacgacacccatcaccaccaccactacggtgacaccaaccccaacacccaccggcacacagtccccaaccccaacagccatcaccaccaccactacggtgaccccaaccccaacacccaccggcacacagaccccaacattgacgcccatcaccaccaccactacggtgaccccaaccccaacacccaccggcacacagaccccaaccccgacacccatctccaccaccactacggtgaccccaaccccaacacccaccggcacacagaccccaaccacgacacccatcaccaccaccaccacggtgaccccaaccccgacacccaccggcacacagaccccaaccacggtactcatcaccaccaccactacgatgaccccaaccccaacacccaccagcacaaagagtacaaccgtgacacccatcaccaccacaactacggtgaccgcaaccccaacacccaccggcacacagaccccaaccatgatacccatcagcaccaccactacggtgaccccaaccccaacacccaccactggaagcacggggccccccacccacacaagcacagcaccgattgctgagttgaccacatccaatcctccgcctgagtcctcaacccctcagacctctcggtccacctcttcccctctcacggagtcaaccacccttctgagtaccctaccacctgccattgagatgaccagcacggccccaccctccacacccacggcacccacgaccacgagcggaggccacacactgtctccaccgcccagcaccaccacgtcccctccaggcacccccactcgcggtaccacgactgggtcatcttcagcccccacccccagcactgtgcagacgaccaccaccagtgcctggacccccacgccgaccccactctccacacccagcatcatcaggaccacaggcctgaggccctacccttcctctgtgcttatctgctgtgtcctgaacgacacctactacgcaccaggtgaggaggtgtacaacggcacatacggagacacctgttatttcgtcaactgctcactgagctgtacgttggagttctataactggtcctgcccatccacgccctccccaacacccacgccctccaagtcgacgcccacgccttccaagccatcgtccacgccctccaagccgacgcccggcaccaagccccccgagtgcccagactttgatcctcccagacaggagaacgagacttggtggctgtgcgactgcttcatggccacgtgcaagtacaacaacacggtggagatcgtgaaggtggagtgtgagccgccgcccatgcccacctgctccaacggcctccaacccgtgcgcgtcgaggaccccgacggctgctgctggcactgggagtgcgactgctactgcacgggctggggcgacccgcactatgtcaccttcgacggactctactacagctaccagggcaactgcacctacgtgctggtggaggagatcagcccctccgtggacaacttcggagtttacatcgacaactaccactgcgatcccaacgacaaggtgtcctgcccccgcaccctcatcgtgcgccacgagacccaggaggtgctgatcaagaccgtgcatatgatgcccatgcaggtgcaggtgcaggtgaacaggcaggcggtggcactgccctacaagaagtacgggctggaggtgtaccagtctggcatcaactacgtggtggacatccccgagctgggtgtcctcgtctcctacaatggcctgtccttctccgtcaggctgccctaccaccggtttggcaacaacaccaagggccagtgtggcacctgcaccaacaccacctccgacgactgcattctgcccagcggggagatcgtctccaactgtgaggctgcggctgaccagtggctggtgaacgacccctccaagccacactgcccccacagcagctccacgaccaagcgcccggccgtcactgtgcccgggggcggtaaaacgaccccacacaaggactgcaccccatctcccctctgccagctcatcaaggacagcctgtttgcccagtgccacgcactggtgcccccgcagcactactacgatgcctgcgtgttcgacagctgcttcatgccgggctcgagcctggagtgcgccagtctgcaggcctacgcagccctctgtgcccagcagaacatctgcctcgactggcggaaccacacgcatggggcctgcttggtggagtgcccatctcacagggagtaccaggcctgtggccctgcagaagagcccacgtgcaaatccagctcctcccagcagaacaacacagtcctggtggaaggctgcttctgtcctgagggcaccatgaactacgctcctggctttgatgtctgcgtgaagacctgcggctgtgtgggacctgacaatgtgcccagagagtttggggagcacttcgagttcgactgcaagaactgtgtctgcctggagggtggaagtggcatcatctgccaacccaagaggtgcagccagaagcccgttacccactgcgtggaagacggcacctacctcgccacggaggtcaaccctgccgacacctgctgcaacattaccgtctgcaagtgcaacaccagcctgtgcaaagagaagccctccgtgtgcccgctgggattcgaagtgaagagcaagatggtgcctggaaggtgctgtcctttctactggtgtgagtccaagggggtgtgtgttcacgggaatgctgagtaccagcccggttctccagtttattcctccaagtgccaggactgcgtgtgcacggacaaggtggacaacaacaccctgctcaacgtcatcgcctgcacccacgtgccctgcaacacctcctgcagccctggcttcgaactcatggaggcccccggggagtgctgtaagaagtgtgaacagacgcactgtatcatcaaacggcccgacaaccagcacgtcatcctgaagcccggggacttcaagagcgacccgaagaacaactgcacattcttcagctgcgtgaagatccacaaccagctcatctcgtccgtctccaacatcacctgccccaactttgatgccagcatttgcatcccgggctccatcacattcatgcccaatggatgctgcaagacctgcacccctcgcaatgagaccagggtgccctgctccaccgtccccgtcaccacggaggtttcgtacgccggctgcaccaagaccgtcctcatgaatcattgctccgggtcctgcgggacatttgtcatgtactcggccaaggcccaggccctggaccacagctgctcctgctgcaaagaggagaaaaccagccagcgtgaggtggtcctgagctgccccaatggcggctcgctgacacacacctacacccacatcgagagctgccagtgccaggacaccgtctgcgggctccccaccggcacctcccgccgggcccggcgctcccctaggcatctggggagcgggtgagcggggtgggcacagcccccttcactgccctcgacagctttacctcccccggaccctctgagcctcctaagctcggcttcctctcttcagatatttattgtctgagtctttgttcagtccttgctttccaataataaactcagggggacatgctgt

SEQ ID NO: 6 - DNA, 84 bp, Homo sapiens
ggccagtgttgagaggcggagacttgggcaattgctggacgctgccctgggcattgcacttgtctcggtctgacagtgccggcc

SEQ ID NO: 7 - DNA, 560 bp, Homo sapiens
atgatgctgttgtggctgttggcaggaagcttcctcacattttcagtttaaatgcattcctcctgatctttccaaaagacggaggcagaacagctggttgccatactccgcataaagtcctttgggtaaattgaaggcatttagtgctataaatttccctctacacacagaaatacaaactaccatcagagaatactacaaacacctctacgcaaataaactagaaaatctagaagaaatggatacattcctcgacacatacactctcccaagactaaaccaggaagaagttgaatctctgaatcgaccaataacaggctctgaaattgtggcaataatcaatagtttaccaaccaaaaagagtccaggaccagatggattcacagccgaattctaccagaggtacaaggaggaactggtaccattccttctgaaactattccaatcaatagaaaaagagggaatcctccctaactcattttatgaggccagcatcattctgataccaaagccgggcagagacacaaccaaaaaagagaattttagaccaatatccttga

SEQ ID NO: 8 - DNA, 102 bp, Homo sapiens
tgtgttccctatcctccttatgtcccacccccactcctgtttgaatatttcaccagaaacaggagtggggggtgggacgtaaggaggatgggggaaagaaca

SEQ ID NO: 9 - DNA, 69 bp, Homo sapiens
gtaaatatagtttaaccaaaacatcagattgtgaatctgacaacagaggcttacgaccccttatttacc

SEQ ID NO: 10 - DNA, 205012 bp, Homo sapiens
ggaaggagcaataactgatttttctgcagtgtcttccttctgaaagcctttccccaacctgaatgtattaaataccatgtcatcatctaaatttcttatggacttggatgctgaaagtaaaataccttgagaaaacaaagaaaaagttagtattaatatataggaagagagattcatttttgccattcttagtttgatgtttgcatacagtcaaacaagaaagaaaatgaaaaatttctctgtcagcctgcttggtaaacgattctgtatctttatatattttctagcttgaatagaaagcacttcaaagaattatacttttcatcattttagaaatgactcattagattgaggctaacctttatgcagctgctaatacctacattgttttggttttagtgacacattgtttattttgagtgtgaattttctcagaatctgactaagatccttggtagaatgctttctgttgagtagattatagtctcttgaaaatgggttgttattaaggaagaccacaggacatcaggctctctctatattattgtttccttttgtgtattttctgattaagtaaagatattaaaactcaagttatttcactcaaggatgataaggataaagttttatttccttttaatcctgattaaactgaaataatcctcaaaagagactttcttttataaatacttgatatagtttttggtgattaaagtacatatgcctgtcagtgtgaacaaaaagccattcatgctatatcaaaaattgacctgtcaggtgtattttatctctgcatttacaaaaggataatatgtacaaatatttattaatgaatttagaaattaatgaattagtccatgaaaagaatatttatgtgcccataaacattacttttggatgatgagtttatgttgtatgacttttaattaaacatttcagagttaatttctaattttgaccccaatgaataagataatacattcttttatatgtcttctggtacatatatgtaagaatttttctagagtatatttctcagtatggaattactggatcatggagtatgtatatgttcagctttactaatgccaaaatgttttccaacatagttgtaagcgatttgtgccctcgataagcagggtatgagaatttccattgttccatgtcctagctgactcttgtgtctcattgtccttttaatttgtattttcctaattaccaaagaggttaagtgtcttcccatatgtttctgagccatttatgtttcctcttatgttaaatgctttttttttttttcttttttggctttgtccatttttctattgggttgtctttttctaatttatttatgggagttctttatatattctggatattaattgttagttatatatgtttcaattattttcgctcagtttgtgacatattttcaacccctctggtgtcttttggtgaaccaaactgattaattttaatgtttaaatatttttcttttttctttatggcaactacttttaatgtgttgtttttttttagaaatccttctcaatccttagattattaacgtgttttcatatattttcttctaaaagtttaaatattttgactttcatgtttaggtttgtaattcatctgtaattttgtgtatgatataagatagagatgtaattttactttttccaatgtccttatatatttcttgaagaagtcatcctgtccccactaatctgcagtgccatctctacagtatatcagatttctatatatgtgtgggctcctttcagaacgttctattccacagccaaatctacagtattaatataactttaaaataatttttaatatctggtcaaatttcccagccctctacttacccacatgtttttcttttacagcagttccttagctattcttagtcatttcttttccatataaatcttaaaatcagcttttcaagttccgtaagaacacttgacaggatattaaggttctagttaggtatcccttatctgaaatgcttaggaccagaagtatttttggatttgggatatttttttcagaatttggaacatttgcattatatcagttaagtatcccaaaatctgaaatctgaaatgcttcaatgaatatatattttttagcatattgttaatgcttaacaagtttcagattttggagcatttttggattttggcttttcagatttgggatgctcaacttataatcacattggttttatagatttatagattaattttggagaagaactgatatcctgaaggtaatttattatctatgagcatgacatttttctgtatttgcttagatcttctttaatctttttttcttctttaatcttttaatgacattttcttttcttcataaaggtcttgcatacctttgttgagagaattataattctttataatttaattgaatttcttatttttggttattataaattgtattttgaaatgatctttctaacattattgctggtatgtgcatgtgcatttggcttgtgcatagtaatttgataacagaaaaaaactttctaaactcttatttttttttctttttaattgtttataaatgtatagattctttgggattttgtatgaagacaattgatataaatgataaaataatggcattttatctctttctcctaacttcatctatattgtgtatacatgtctttgtgtctgttcatgtgttcatacacactggccaaagcctccagtaaatactgaaaatggagagaagagatatctttacagtgttactgattttacagataatgattttaatgcttcaccactgagcgtaatgtttgctgtaggtttcttatagatacttgctataaagtacaggatgttctcttttgtttctggcttactaatagtttttatcatgaattgttgttgaatattattgaatgctttttttgcatatattgagatgaccagatcattttctccttcagtctttggaaatattaacagatttttctaatgttaaactaaccatgtgttcatgaagaaacctttaaattatcggattcaatttggcaatatttgatttagtacattttacatttattatgagtaagattgatttgtaattttccttttttatattgactttggtttgatattaagtttgtaccaatttcttacattgagggcaagatttatccttctttcttttctctcttgttagactttgggtttggtgttttcttggtaggatttttgttgttaagaattgatgtactttcttcagtagctgtagtaacatttagcttctctgtttcttttttagtttgttttaggaatttacattattgtataatttgtccatttcacttaagtactttttatctgaggtagacttaactgctgattttctcggggactattaagatctttctcagtaaatgttttgtgattataattataaacaaaggactctgacatcccttgacttctttgatcttagagcttccttatctttttaatgttgttagttgtgccctactttgtttcccttggtttgaacctggtttggatgtgcctgtttaatctataaaagtccttgttaggctgggcacggtggctcacgcctgtaaccccagcaccatgggaggccgaggtgggtggatcacctgaggtcaggagtttgtgaccagcctggccaacatggtgaaaccccatctctactaaaaatataaaaattagctgggcatggtggtgggtgcctgtaattccagctactggagaggctgaggcaggagaattgcttgaacccaggagacggaggttgcagtgaaccaaacatggtgccattgcactccagcccaggcgacagagcgagactctgtctggaaaaaaaaaaaaaaaaaaaaaaaaaagtccttgttaatggaaatcttttttcttagatgctgttgtgggagggtaataaatattaataattatgtactttgttttaaatttccactggatgaattggcttggctgatcttcactcaaaattgggaccaaatccaaatgattttgacggtttagagaagttaatgttttattttgtttaaactgtcatagcctctgagcattatgaggttttgccataaccatttaattatggagatagtttccaatttttttaatgataactttttttaaaaaaaactttggttactgtgatgtgcagtggagcatagtagacttctttttcattgatgctgaaaatggtatgtccccaagtagtagaagggaactttggagaagtaaaactattgccagatgggcttgggtggttcagtaaaccttacaaaggcaaaaggcttatataaaatatgatcttcattttctgttgaactactgctaacactgtatatttgcaagtcactttattaaatttctctttgttccaattaacacatctttgctatgtgtcaccagtaaattaaatggcaattggccattggcttactgagaatcatcaatttcttagtggctaattgtatgagtgtaaaaacaagattgctcacttatataaattatcaaaagatataagaaaacttaaaattccttctcagatttctatagtaaacaacccatacactttcacctagcgtttaccattaacgttttacttctatcccttcatccctttattaatcatcttattcttttaatgcatttcaaaggatattgcatatatcagtatgcttttcatgaaatacttcaacatacgtatcattaactggaatttaatagttgtttacagcttttttttgaagtaaaatttatggaaagtaaaatgcataaactataagtgcatatttgctaatttttgacaaatgtgtttgcttatgaaacccaaagtcctttcaagatacaagacattgccatcaccccagaaagttatgtcttaccttgttagagtttacatgtaccaccattttccccactcccacccgtcattccaactctgctcttagacaatcactgttctaatttcttctgctgtgaattagttttgcctattttggaaatatacagtatgacgtcttttatggaaggcctctttcactcagcatgtttgacattcatctttaatgttgtaagaagcagtagttccttccttttttattaccgttgtataaatatactacaattgacttgtctcttttcctgttaatggactcttgaattgtatccagtttttggctattacgaataacactatctacattcttgcacaagtctttttgtggacatgtgtttttatttctcttgggtaaatatataggaatggaattgctaggatataagatagatgtatctttaattttgtaagaaattgttagattattttccaaagtgattgtaccattttatacttcaacaaagactgtattagagctttggttgctccacatcctcaccagcatttgatgttgtcagtcttaatcttagccattctggtagatgagtagtgatatcgtgttttaattacattttcctaataactaatgatgttgagcactttttcatgtgcttgttagctattcatatattttcttttgtgaagtgtctgtttagatcttttgttcattttgttgggcgagggatgtttctttttattactgagttgtaagagttatatatattacatatatattcctcccaccccagaaattccccccaaccccagaattttcttctctttatctatgtttccaactggagtgggccacatgagacattcctgtataagattggagagcagaagtgaagcagatgtcacgtacggttcacacatgatgtcgcttatctgctggctcatgtcgttggctctgcagcagtcagacctgcgactgctccactttcgctggatccactttcagtttctctgactcctgggacacatgtgtgcagttctgtgacaaaggagactagctgtcctgaggacatccataccattgaggtcagatgcagcaagatatgatatgagtttcagtctatcctcatgggtttcagctcatgctggtgaattccagtatgttcttcttcttccctactttacatccatctttccttcctggcagcctgccctgtggactccagcattagatggaatgatctgcttaatattgcttaattagctttcacaattgcatgagacagatttatgtaacaaattgtgtatatatttctgtatatgtgaatatgtatgtgtgttgttctgcttctgtgattgacttctgacggacacttcccaactctttttatgagtctagcataaatttggtaccaagacctgataatgctattacaagaagggaaaattataggccaatatttctaatgaacatggatgtaaaaatcctaaacaaaatgttatcaaatagaatccagttatgaaaaaggtaaaatttcatgaccaggtgaggtttatttcaggaatgtaaaattgaactttcagaaaaaaattggtaaaattcaccactgtaaatgaatacaggagacaaaaacacgatcatctcaaatatagaaaagcacaatgattggctgtgctgaatgctactggttgagtaagatgagaactgagaatttatctttgatttggctatgtgatagtcattgctgaccttaatgaagcagtttcaatgacactggtagagattcaaccttgataggagagaatttaataagaatggaaagagaacaaatggaaacagtgaatataaatagtatgtcaccgatttacactgaagaatgcagaaaaattagattgtagatggaagagagttggctattgctatttaaagatggaagatattgtagcatgataagaagtggctatgctgaatttgtgggactcaagtaacaaaaggatttacatgctgtaaacagtatggaataaaatagacattcatcctccttcccaactcttaagtatgtgtggtggtaatgggatcagtgaagtggagaacgctataagggtatttgttattcagaaggtatagtacaaagattggagagagaagagagaagaaacacagtgctgtttagagatgaaagtgtgggaggatagatatctagaggggctcatatctggatggagagcaagggtaagagagaacaaggtgtggtaatttggctagcaagggaattagtcctgacactcccttagaaggtgtgtgtgtgtgtgtgtgtgtgtgtgtgtgtgtgtgtggagttgatgtagttggcagggaagggtagctcctggtaggcgtttaggccactcagaattcagcaataaaattaggaggttatccttctgagacagtttgaatttggttggtaagttgacctccagtttttttttctttctttgagaagagtcaacttgagtttttttgtttgtttgtttttaatttgaaggctcagaagagagatccaaggcttccagcatgtgggcttgtagagagtacttagagacgcgagatatgggggccagctgagagtggtgaagatggttaagctcttgttttgctccaagaattggagtgggtaaggtatcttctcaccatgctcaatgcagttggtttgtgagatagtggggtgggagacacagggagagtttatgatgctccactgtaattagtccagtaactgtgagaccagttgagtaggaacgtggatatcctcaagctttgttccactgttacagctggtaaacatggatgaattgatttaaatatttattttgcaacaatgtggatttgaattatggatatagtttcctctttttggttaattatatgcacatttgaattcatctctgtctatgagtactagtggactagctgcttccctggatctcgttactggatggtatgttgctcttagtgtcatccaaacagaattattttaaaagtgaaatgaagaaaccagttgtagtgaattacacatcaccaatttttagagctgtagactaatatcttgaaaattgccttaacatctttttgccacaaatcaagatataagtaacattaagagttatgtaaggccaggcgtggtggctcacacctgtaatcccagcactttgggaggctgaagaggatggatcatctgaggtcaggagttaaagaccaacctggccaatatggtgaaaccccgtctctactaaaagtaaaaaaaacaaaattagccggctgtggtggcatgtgcctgtagtcccagctactcgggaggctgaggcacaagaatctcttgaatgcggacagtggaggttgcagtgagctgagaatgcaccactgcactctagcctgggcgacagagcaagattccatctcaattaaaaaaaaaaaaagttatgtgaacatgcttgaaatgatgttcatggctaaatttttcagttaccttgtaaagatgattcttggatattgttttgattctgagtacttttggagtcatctgatagtatgcttcgagaataacaatctgatgatagctttcaacattgggttaccaacaaagcttgttattttgtatacattgattcataatttcaggtttcttcaccattatggtaagtagtgtattgagtcttcattctaacacatgttaggaatttatgtttgtactcatggatgtctttaaccctcagacatttctacttatattgagaactctagactgaaaacattttgaaatgtagtggttttactatgtaggaggaacatgtgattcatttgttctgcttcattttcttctgtttgtgatagagattggatcagatgaaagtgtcttgataatgatatacatgccattcttttcattctatgtatttgtagtccttttttgccatcataactttgtttatgatattccctgctcttaaaataccctcatcttgtccctccacctatctatatctaaaatatccttcaagaccttccttttgcagctttctctgagtactacagccaaatcctcttgtctgaactccaacatgtgtaatacattatcatcctgtttaaatataattatttcttatatttattaatttatcaaggccctaaatatctgcataagcttgccttcatggtttcactttttcattgttctctatattcatgccatgtaactttggcatgccttcccactgtgggtggggtaacctgcccactgtttgactctggtttcaggcatgtgatttgctttaactaatgagatattatcagatatcatgcaagcagaggcttgaaatggtcttgcacattgggaattccctcttgagcctctgccaccaccatgaaaacattcccatgctagcctgctggagagagccacatggaggagagccatgctaccctaactgccatagctgaggctatcctcgatcagcacacatccattcaagcaccagacactggagaaagtccacttgaggtcagtagagctgcctagcagatgcccaactgacccaaaaagcataagacataaacatttattgttgtataccctctgaagttttgcatgtgttacaccatattactatagtaatagataattgatacaaatgtcctacatggcctggaccatgcattccttgctaaatttatttcttgctactctgtccctctttcgtcactctctagtgatattggccttctgtttttatgatatgccaagatcatttctgacgcaagactttttccctgctattctctttgtcaggagcatctttctcctgttatttatctgagcatttatcactcattattgtgatgctcagctcaaatatcatggtttctgagagtgcttccttgaccctatgagctaaaggagcccccttcccactcattctttccctattcctttcactcctttattttcttcactgtgcttctgtctaaaattatcttacttgtttacatgcttattgtccatttcctctaatgccagtgagggagatggtatcaagaacagagtatcaagaacagagtctggcacatagtagcctttcaataaacatgtaataaatgtatgaattattttttcattaagagaacagatggtagaaactatgataggttctagaatatgatagagtatttacttattacctaggtctgctgtgacaaattaccacaaacttgatggcttaaggcaacaaaagcccaaaatcaatgcgtggacaggactgtgtttcctccagagactctaggggagagcccttccttgcctcttccagcttctggtgactgttggcattcactgccttgtggtagcatcctctgctctgtcttcaatgaccttctcctctttgtgtctgttcctaatattcctctgcctctctcttataaggattcatgtgatggcatttagggcccaccaggattatctcctcatctcaagattcttagtcacatctgccaagactcttttaggggtaacattcaaaatgaataaagaaaactacaggacaatatgcctgatgaacacagatgcaaacctcctcaacgtaatactagcaaaccaaatacagcagcacataaaaaattgcttcaccatgatcaagtaagtttcatttctgagatgcaggttggctcaacatatgaaaatcaataaatatgattcaccacatatgcagaattaagaagaaaaaccatatgatcatctcagtagacacaggaaaagctttcagtaaaatccaacatcccttcatgataaaaaccctcaaaaaactaggcattgaagatacatacctcaaaaaataagcgccatctctgacaaacctacagacaacatcatactgaatggacaataactggaatcattccccttgagattggaataagacaaggatgcccactctcaccactcctgttcaaaatagtactggaagtccttgccagagcaatcaggcaagagaaagaaataaaaggcatgcgaataggagaaaaagtcgaactatcttcactgatgatataactcgatacttaggaaactaaagactctgccaaaaggctcctgaaactcataagcgcttcagtaaagtatgaggatacaaaattaacatacagaagtttgtagcatttctatacaccaataacattcaagctgaaagctaaatcaagaatgcaattccatttacaatacacatggacacacacacacgcctaggatacaaataaccaaagaggtaaaagatctccccaaggagaactacaaaacactgctgaaagaaatcccagatggaaacaaacaaatagaaaactattctacgctcacagattggaagaatcaatatcattaaaatagtcatactgtccaaagcgatctacaagtccaatgctattcctatcaagctatcaatatcatttttcacaaaactggaaaagactattctaaaatttatatggaacaacaacaacagaaagcccaaatagccaaagcaatcctaaacaaaaaaacaaagctggaagcatcaaattacctgacttcaaactatactataaggctacagtaaacaaaacagcatggcactggtgcaaaaacagaaacacatagaccagtggaacagaacagagaacccagaaataaagctgcacacctacagccacctgaccttcatcaaagttgacaaaaatagtcaatggggaaatgactccctattctataaatggttctgggatagctggctagtcacattgcaaaagaatgaaaccagacctctatatttcaccatatacaaaaattaacccaagagggattaaagtgtaagaccacaaattataagaattctagaagaaaacctaggaaacatctttctggagattggtcataggagagaacgtattactaagtcctcaaaagcaattgcaacaaaaccaaaaattgataagtgggacctgcataaactaaagagcttctgcacagcaaaataaactatcaacagaataaaaagacaacctacagaatgagagaaaatattcacaaactatgcatccaacaaaggtctaacatctagaatatataagaaacaaacagttgaacaagcaaaaaacaaatagccccattaaaaaatggagaaaatacatgaagagacacttctcaaaagaagacatacaagcagccaacaaacatttaaaaatgttcagcatcactagagaaatgcaaatcaaaaccacaatgagatgccttcttataccagttaaaatgggtattattaaaaagtcaaaaatcaacagatgccggcaaggctgtagagaaaagggaatgcttatacaccgttggtgggaatgtaaattagtttagcccctgtggaaagcagtttgcagatttctcaaagaacttgaaacagaactaccatttgacctagcaatcctattactggtatgcatccaaaagaaagtaagttgctctactaaaaagacatatgtactcatatgttcatcacaatgctattcataatagtaaagacatggagtcatctaggtgcccatcaaaagcagattagaaaaagagaatggggtattatacaccatggaatactatgcacccatagaaaaaaaattatgtcctttttagcaacatggaaacagctggaagccattatcctaagcaaattaacacaggaacaaaacaaaataccacatgttctcacttataagtgggagtaaaacaggtacttgtggacataaaggtgctaacagtagactcgggactactaggggagggagcaaggaaggcagggggtaggggctgaaaaattgttgggtactatgctcagtacttgggtgactcaagtaatctgcacatgtacaccctgaatctaaaaagttgaaattataaaaataataaaatatttttttaaaagatagcattcacagcttccagggattcagtgtgaatacttttgggggccattttttggcctgccagaagtataaacactatcaactctagtatataagaggcaaaacagtattatctgcacatgaccatgctgtttaagctctgtgcctacttgctctcctgcaaagcacagatatcaatagtacctatttccaaagattgttgtgaggattgatatgtaagtacccagtagtttctatgacataagtattcaataaatatcattacactgttaaacaatgcctactgaacatttcctatgtgccaagcttcgtcccaagtacatgtcatgccttagccaatttagtcctcacaacaatcctatgagtagagactgtctcttgctgaaggtcatatacctagtaagcggtggtgagattgaaacccagacactctgctccagaagtctgtgctcttaaccgctccagatgtggcctttctgaatgatgctactgttgttttaaaataattgctctaggctcggtgtggtggctcacacctgtaatcccaagactttgggaggctgaggcaggagaattgcttgagcccaggagtttgagaccagcttcagcaacatggtgagaccctatctctaccaaaaaaaaaaaaaaagaaaaaagccagatatggtggcacatgcctgtggtcccagctacttaggaagctgaggcagaaggatcgcttgagctcaggaggtcaagactgcggtaagacatgattgtgtcactgcactccagcctgtgcaacagagcaagaccctgtctcaattagtaataatagtaattgcttcagggccaggtgcaggggctcatgtttatagtcccagcactttgggaggctgaggctggaggatcacttcagtccaggagttcaaggacagcctgggcaataaagtgaggccccatctttacaaaaaattgaaaaaaaaaaaaaaaaaggcaggcctcttggtgtgcacctgtggtcccagctacttgggaggctgatctgggaggatcacttgagcccaggaggttgaggctgtagtgagccatgattacactaatgcattccagccttggcagcagatcaagaccctgtctcaaaaaaataaataaaaataaaataattgctgtgaaatttctattaacgtttttgggaaaaccagaggcttctgtgtgacatgtgaatcacagaggagaaatcatgaatctttatagccttgtgttaacatgacttccttttgttgatagagtggtttattagtctcaagacctttgaaatggcacatgaattgcttggacagattatggagacatccacccttctttagagatttaagtaagtagaaccagttagtgtgcctcttctgtttctcaccttgctcaatgcagaatgaacttggtgtatatccaccagaagcacctgcttatctactgtttgctgtcgttgcaggtatctgttgagattagctgtaacgagttgtatgtaattttataactaactgaattaagaaaagcctttgtaagattcagtatctgcttcaggtcattgaaatgtaaaattagaaagtaagctgagggcaggggatttttttctgttttattccatttattccctcaccacctttgccatccaccaccaacagtttcttttaaatttagcatccagagtagacctttgacaacgcaaatcagatcacttcatttgttcattaaaaaccttcaacaggtttcacattattcttaggattatatttaacatccttatacagtaatctccaagcctctccttgatctggtaccctctttccatctctaatctcttctttaacactcctatacttacttactcagccccaggcacattggcatatttgctgttgcctgaacatgcaaattccttgaacttgctgtttccttgcctgaaactctctttcctcagatatctgcctggccttcctcttaacctccaagtcttgtctcaaatatcattttttcagtgaggccttgcttggccagccctttccctcactatatcctgctccccaacaattgatttttacttatccatataacttttatccccctgtgtgctatatattttacttatttcttggttcattggctgtctccaccaaaatgtaagtgccatgaggacaggaattttattaatatcagtttgttcatttctatacctttagtgctttaaacagtatttagcacacagtaagcattcaataaatatgtattggactgggcacagtggctcatgcctgtaatcccagcactttgagaggccgaggcaggtggatcacctgaggtcaggagttcaagaccagtctggccagcagggtgaaaccccatttctactaaagagaccaaaatcagccagtcatggtggcatgtgcctgtagtcccagctactcggtaggctgaggcaggaagatcgctagaatccaggaggcagaggttgcagtgagtcgagatcaggccattgcactccagcctgggtgacagagcaagactctgtcttcaaaaaaaaaaaaaaaaagtattgaataattgaatgaatgttctgcaatgtaacagtccagttagctatatagcactgcttgggatgcagtgtggcctgcttgtctaacactattatggagatatttctatggatttatttgtattattaatgattgagtttataatcctatcttttaatgttgtgtacttcaaatgctattagttttctagatagccaaagatggctaaactctcttctgcccttctttaactacaatttagagaagtggaatttccatgtaagcaacctattgagcatctttactgaatatcttttatttgtgtatattttgggggtagtggggaaaagggacattttaatggcaaaacctaagttagggccccattctctacttgaaactctagacatttttaactgaatttttaataaaaaattactgaggctttgtagaaaaagatgagaatggggtagcatagagtagttgcgctagccacatttcaagtgctccagtgctgcatgtggctagtagctaccatattgaacagtgtagatatagaacattttcatcattacagaaagttctattatacagcactgctccaaacagtaggaactctgaacattgagctagataataagatataatcattttatgttttgtatccacagtggggaaatgtaaggaattgtgtcttgtaattctcttatactgtacctttatttgctcaacagatgtttgttttgcctctaataatatataccaggcactctactaggcactgggaattcaggggtagacacaatagcctcaggcctttctgtatggagcttgtattctcatggaagagcagtcattaagtagataatcatacaaataactatagtctctatagtgctggttgtatagtagatgtttaaatgactgttgattaattgactaatgtgtacagtcccatcatcttcttagatactgacaaatcataggaacaaaaagctagctagtaatttatagttaaggtctgcaagtaacattaaaatttcagtgcagtcaataaatttagttctgttcagactgtttttgttatttttcttatttttgacatagagcaaagattatgtcagttgccctgtggtttaaagccacagttattctagaagcacagttgccatcattgagtagtagctgatccaaaagaattccagccaaggtcttgccaatgatggaaagaaatgatgtgtcctggaagttgccaaaaattatgtttttcttgttgaagacaatctttgtatctttaagcccttcatatgttgtgacatgagcacatatgaatgttccctaaaaggcaacaattatgctgtcaaattcattcaagcagtagttatccctgtataatttgaagttatacagatgcctaataagtgttttgatgctgttgctactgatgttgctgatgacattacatagaaagttgcagaagataaaccatgaagattgacactttaccattattattttgattttgtttctctcttcacatcatcaagtcttgcttatgctgttaagccctagcagttctttaatatggaagggggtatgacatataatttccacctctgagaattattttctttttgttgatttttgcaacttcatccagacttctctaaaatggtgtatctgtgtgctttgtattgttggacactgacactgttgatgtaataatcaggggcttattgtaccagttaataattagccaaactcaggaggctgaggtgggaggatcacttgagcccaggagatcaaggctgcagtgagtcaagatcagatcactgcactccagcctgggcagcagcaagaccctgcctcaaaaacaataataacaataattataataattagcttagtaatagaaattcaaagtatgggtgtttaaataaatcagaattcagtttttctatgcaaagagaagtgtggaaataaattttttaacttcccaaatttttaaacacaagattttttaaaaacttgatcatctgataaaatagcctatacatttttagggaaataattctgcatagggtcttacctccagatagcaaaacatttttttaaagctatagtaattaaaatatggtacatatggaaccaggaataggtagataaatgaattgagtggaaagctcagaaatatacccaactgtttgttataatttattataagctaaaaattacactcaaatcaatgaggaaaagttattttgtacaatgactagtttaacataatggtctaatcgcttgggaaaaagtaaagttagaactctataagtccttatcagaaaatgcagtccaaacataattacaatcatatgccacttaatagggacatgctctgagaaatgctttgttaggtgattttgttctgaggactttatagattgtacttacccagatctagataatatagcctactacccacctagactatatggtatagactatttcacctaggctataaacctgtacagcatgttactgtactgaatactgtaggcaattgcaacatgatggtattgtgattgtgtatctagccatatctaaacatagacaaggtacagtaaaaatacagtttatatatatataaacagaataatgtatatataaacaaaatatatatatgtatatatatttaaaatggtatgcctgtataggacacttcccatgaatggagcttgcaggactggacgttgctctcagtgtcattgagtgagtggtgagtaaatatgaaggcctaggacattatactactgtagacttaagaagtctacatttaggttatactaaatttattttaaaaaattttctttcttcaataataaattaaccctagcttactttttttattttatgaattaaattttttaacattttatttttttgtaataacagcttaaaacacaaacacatagttcagctatacaaaaaatattttctttataaccttattctgtaagcttttttctatttttaaattttttatgtttttacttataattttttgttcaaaaactatgacacaaacgtacacattagcctaggcctacacagggtcaggatcattaatatcactggcttctacctccacatcttgtctcactgcaggatcgtcaggggcaacaatactcgtggagctgtcatttcctataatatcaatgccttctgtaatacctcttgatggacctgcctgagactatttacagttaacttttttttggaggtagaaggagtatactctaaaataatgattaaaagtatagtaaacacatacatcagtaagataatcatttattatgatcaaatatgtagtgtacataatcatatgcactgtacttttatatgactgggactgcagtggatttgtttataccagcatcaccacaaacatgtgagtcatgcattgcacgatgacatcactaggcaataggaattttccagcttcattataatcttatgggaccacctccatatctgcagtttgtcattgactgaaatgtcattatgcaacacatgactatatatttgtacacggaaaaaagcttttaatatattatttaaataattatttactatattatttaaagaaaaatacaaaaccattgtaagatacatttaaaaaacatcaagcatatatttctttctggtcgtgtatatgtttgtgtgtctcaaagactatacaatcattcctacctatcacaggacattggttccaggacaccaaaccaaaatccagggatgctcatgtcccttatataaaatggtgtaatatttgcatataacctatgcacattctctgagatactttaaatcaattctagatgacttacaacatctaatacaatataaatgctatgtcaatagttgttatatgtaatttttaaaatgtttattattattgtgttttttaaattgttttgttttagagtattttccattcacagttggttgaatctgtggatgcagacacacagggagaaccaagtatatggtaaaatatcagtagtgttatttctgggtagtgggattataggtagttaaaatacatgtatttacttttctttgtgcctatctgtattctgagttttctaaattaagccttgttataaaaaaagaactaaaaataagtgatctctattattgattatatcacaatgcatataggaaatatgctttgatgcaggaatagttgttaaaagttgatttataactcattttgttttcttatttaattatttttaagagatggggtctcactgtgttgcccaggctagagttgcctattcacaggcatgatcccactaccgatcagaacgggagtttcgatctgcttcatttccaacctgagtggttcactcctccttaggcaacctggtggtctcccactcctgggaggtcaccatgttgatgcctaacttagtgtgggcaccccatttgtatatagcacattacagcccagaactcccaggctcaagcgatcctcctgcctcggtcttcctagtagatgaaactacagttgtgtgccaatgtacctggcttacataacttattttatccccggctatccagtactgactcccggtgattccacagctccagattggcacttcttccccctgtaccaatgcgtaatttgatcagttttcttgattttcagtattcctgttgtgtgtgactagcagtttcccttttgccatgactttaaaactccccacacctggccgggcacggtggctcacgcctgtaatcccagcactttgggaggcggaggcgggcagatcacgaggtcaggagattgagaccatcctggctaacacggtgaaaccccgtctctaccaaaaatacaaaaaattagccgggcgtggtggcggcgcccgtagtcccagctactcgggaggctgaggcaggagaatggcgtgaacccgggaggcggagcttgcagtgagccgagatcgcgccactgcactccagcctgggcggcagagtgacactccgtctcaaaaaaaaaaaaacaaaaacaaacaaaaaaaaaactccccacacgtgatgatcaccctgtggtcagttttgtttgaatatgttccaacctacagagtagttgtgggtagttttgactgttcacgataatatttacaaagaattgaataaatattttttatttccaaatattggtggtggtcgtggtgattaagaatctgaatcggatgaaccagccttgcctttagagaaatgtccaagttacgtttggtttatgggggctctatattgggagaagtgaagaggcctaggacccaggatttccaagataaggttgttcagcagggctcatagagaacatcatttagaatttggcttgttcccaaatgattccctttataattcttaacagagaggctctgactgtatcagtatggtgtttctttattaagcaaaagctcatgccaagtgacttcaggtgcatttgacttcatatttagtcacagtgtgaatttctgtatgattaacttacccatcaccgtgatgaagaatgagatggtggtagtgatgctgtgattatattacctctttcatccttgatttttggtgattagtcttccttgaaactttctcttgacatggaccatcaatatggaaatctgaagcttccattgatggaggtggtctctgaactagcatccatccaagccaggaatagactgcaataaacttattgagaataacacaatccttaattgtatgtgtaatccatggctttcactgtctttaccacaccaaatggcattgccaagtcttatttttcctccttcctctgcttctcacacaacctcttttcttcatgcaattccattttccattccatttccattcaatgaatcttccaagcctaaaggtttaaatctggtcatccccctctcttccatgcagtttcatttctaagatggcattgaggatattgccatggttgtttcatacttagttgttattgttatgataggtaatatataattctgaactaaaattgctggctattttttgtcattgtgacaacaggttttagaaacatagcactccaattttgctactgaatgttttgattaaatgggagggactagaagactacaatttaagagcaggcttcagcaataatttttaaaaatagattcagagtcgatcatcttactatatttctatctaggcttatctcccttcatgcagttagttacaacacttggagggctgtttccaagactggcactaaagaggtcactttttccactctctctcccagaaaatatcaggaagtgcagtaaggttcatgaaaatttaagcttgaagtttagaaaactcaaaacaacccaaaccctcaaacattcagtttggtttgaatcttggacaaaggttttctatgcagctagtggagttatttcagtttaacggctgtagtaacttcatttcagggctaggggaaattatgaaaccataacttggatcttattttaacaaaaccaagaaataaaaacactggggaatctgcatgggaaaggggacctacctaaccccaattgctgctattttactgtggcagctcctcttactataggaattatgaaaccattctttccaattccttcagagagagctgacttttgaaaccgattgagtggcctgcatccaattaataaccctcctgatgtgcgcaacagggaagatctttcataggtgattaaatccaatagagttaaggtctgtcatcgtgatttccctcctggtcaactttcatttcaaaagtcatcccaggagaaccactgtagttctttacctagttgacttctgaaacaaaattttccacttcaaagagagcccaataatttagaccctatcctccttggatacaatttattttttccaagaataagaatttaatttaatgactatttattgagtggcttcattatatctggcataggataatatattccaggcagaggtatacaacatagggggaaaaatgtcctcaaagatcttttggaccagttcaataatcaacaatgaaacatcttagaacaaaaacaaattcaaaaaggatttattttgaaataatctagaaaacctcagttgatttttaaacatacccaatagagtatgtcacctcatttacagttgatcacttatcaaatactgcagagcaaaatgaggtcgagcctcaggctctgcagatgtggagcacagcctaaaggggcaaagcatcagcagcctgctgaatttctgaagcacacaatctcagaggatttccggactatttggggcttcagagcatccagaaatactgaaaatttaataaagttcgtgttttcttatttaggtagagacagatttgccagataatagaagtgacttaactaacaaggttccagttaataagtgccataaatattcccccaaagtatctatattcttatcaaactagcttgttctcttaattgaggatatacgtagtgattttagttggattatattaagcattcaccacccttttaagtgattatttctgctattatatggaatcatgttactatgaaatttgaattaactcacatgaaatctgaatcacagccagtgaaatgtggttaatggtatttgttgtaacttgaaattttcctttttttttttgcatttcttttaaaatattgttttaatattatgctttgatgatgtcagtatctaatttctttccttctttatgtactttagaactacagggagcaaatctgtttcttagaatataaatccatctagtaaacttttcaaaatttggagatctcctagaactattttctgaactaataatgatgcaataatgattacagttaatagtggaactgtaggaatatcatattctttaataacttgaaattttaaaatttgattctgaatatttatcaaaactattattgggcaaccaatacatactgtgtaaagttctgtacttagggattgaaccagtggttgaggaaatgaaacaaatctgaatgttaaatgcctattaagtggcagggacagtcaattccaaacaaggaagtaatcatttccagatggggatggtctgagtcctcatggaggaggtgaaattagtgttctcctttgaaaggtatatgcatttagagactagtgagcacgtgtttcagaggtgagaaattgatgcatcagaggctggaaaatgcatgctgtgtgtgtgaaggacaatgagaagacctctttgctgggcttaaacacagagttgatgtaggagagtagtgggtattagagcttaaaaggtaggataaagccggattttggaaggctgtgggctttttgtcatagatgcaaggagctgttttaagtttttgagatgaggattgaaatggtgaagtagtgttttaggaagataacgcaggtagtaacagggtaagtgggaaagaaaatggttgaagatacgacaattgattagaaaatttgcacttgcctaagaaaagatgataaaaaatctagtgtgtagtagtggctacagtgctggaaggagaaacattaggaagagaacaaggaatcaatataattttgagattgctagacatgggaagtgagggacaacttaaaaatgacaccttttggcttaatgtatgattttgaacctgcgtatcagggataatgattatcataaatgagaaatctggaaaataggtcaggttggggttaagggtagaaaataggctttgttttaagtgaattgctcttgagatagtggcatgtcttctaataagcaggtggaaatgcaggactcaattttatgagagagatcaggactagtaacaaaaaatggtgaccatttatatataagtaacaaccaaagttggagaggtaaatatcacctgaaggcttagaaatgctaaaaatggaaaagcaaatatctgagctgtgagatgtaggacacacgagatttaggtgatgaaaggtggaaaaaagacagtaaaagagacagaaaacaaagcaattgaaaggtaaagaaaagaaccagaatatgatagagtcatagaagtcaaacaagttatgagttttcaaaataatagtagtgattggcagtatctcatactttagacaggctatgcagaatggggaatggaaaacaccattgattatgtcaactaggagtctttgaagccaattaagtataattttcatagagtaggaagagcagagccaaattgtgtgagaaataaggaggcagtcgtggtaagcaggtatattcaaccctttgggaagaaaggagaaaaaagaacagtggcaagatgagtaccaggccctctccttttctccctccccaggcagattcaatctctttcatgtagaatcaccatttgtatgtcaataccttctggaattatatcacaaatatagaacatcgtccctaacaccctagctcccatatatcaacagctcttactttggtatcaatagatgccacttcaacttcaacatccgaaactaaatttataatttccccgtgctcctactaaaaaacaaaacaaaatacaaataagcataaataaacaacaaccaggtcttcttttagtgttttccatttcagtaagtaacatgacactctccccacttgctcacgctagaaagctcggggtcatttttgatacccccctttgctcttcatttctgtcatctaattcatcaccaaatcttgtaaacacacttctctccacatccactgccccactagttgaagactcggtcatctgaacaaactcagtaatatttcacgtgtctcctctgcatctcctcttgctcctcacagaagccagtgtaatcctttaaatccacaaacctgattactattaccctcctatttaataccttctagtggcctcttttttccttcaagccaagtgatgttatgaaaacaactattttagaatgaagcaactaactctgtatggaggaattagaaaaaccttcattaagatattggcatatggactggccttcagtgtcttcaggtggagaattctattagtgtgaagtatgggatgagagtgacagaagatcattccggcttgaggaacgtcatgtgccaaggtaggaagtaggtgttcagaaaagcgtgacaagttcagagggtgatgtcaagggatggggagtagctgtagaagccagtttttgaaagccctttgatgttggattttatggaggttttaaagcaagggataatataaagaaccaagctttttgtggcaaaggggaaagttgactgcaatgtttgagagtcttagagaagagagagcagtttagtgcctgttgtagggacccaagaaaggtgatagaggccaagacaaaggctgtggggctggggagaagattccaggcatatttagagtaggacctacagaagtaatgcaacatttgaggctagatgtccttgaataatgttattgtgagtgggtttatgtgcaaagcctatgatctgaccctaaattgacatgttattctgtggtctcatactctgtagaatgtattatttttgccacatgtaaaatgtactagagataaattacaattagtttgtttcctagtcaaagctacactaaaattacaacccagtaaaaatatttttaagaatccaaatatctggatttttcacagttctgtctctgataagttttagaaacttggtcaagtcatatactcagccggaggcttaaatttctcatttgcaaaaggaaggagttgactagactcactgaatgacctctaaggttccttcaagttccttggaaccagtgtcaacctctagggtatttttctgctttagttgattgacttgattctaactagcaggaagcagacggcttcagagtttcttgaaaacatagttatctccttgaagaactgtggtctagggagtgttctgagtagcattcgtagacccaccttgtcttataaaatgcattacatttataatccttctagaggatctttccaatctcccgtagctgggtaccaagcaaaaatcattccagttaataagagccatttgttggtaatagttctattatatttggtgtggcatattttcttttctccccaaggcttctcttaactaggagaaacttaaaagtacattcattgtcaagtcttcctaggcttttgatttcaagaacttgtgtagaattatgtgtttttttccttcaagtacaatttgcagaagggtagagacatatataatttaattgaacaaatttaaacttccactgtgtatgaagcattgtggagaaaaagcaggatgggtaaaggaatgtgccaagagggataaggcgcaatttctgtcttcaagtaagtatattatttaacaggagagcctacaatgttaatacatacttcaagtaggtatatgaaaatggtagtacagtagaagagagtgctacatgtaggatgagtatgattactccagccttgggcttgcaaattggaataactgtcttctggtaagcgctattcctaaattctgtctgagctggtgaatattggtatgaataacccaggtataggtctaaaataattgatcaacttgtctttggcaagtgtatataaagttttaagcaatctcttaaccacttcagattacagcgtattgctcatgtgagagataaaaatgaccaactgcttgaaaatggttgattggttataaatagacacagtctaaatttttggcaagagcatgataaaagcttttatgaagttatgaaattgtggcaacatattgtcaactgtggcacttgaagtcaagtcattagagaatcacatgaacagatttagtatactactaagctgacagacatactggcataaacagttattaagctgcagactaaactgaagatcaattttttaaaaatgatgctttgcagcatgttgtatgggtattacattttttatgtacatcatattcaactcctggatgagtgttatcttaaggttttctgggttgaatttaacataaagataacaggattccatttctaaagatggggcatttgtctcattcaatgtgagtgctaaaatattcttgttctataattcattcttctgagagataactatgatttctggtagtgtaaaggtgttcttccctgttttgtctttgtaccctgagaataaacaatcataggtaaaataaacttaaaataaattgtaggtgaaataaacttgcaggtttaaaaagcataagaaagctagtaagccaggaaactggtatgtatatatattttataaacctggtattatattttatgtcttcatctaattatgaaagtgattaaaaagtttaatatagtgaaaaatgtgtctaaattgtgacaaaagttctgatcccagatttatgtctgtatttgttctcacgctgctaataaagacatacccaagactgggtaatttataaaggaaagaggttcaatggactcacagttccacatggctggggaggcctcacaatcatggcagaagacaaaggaggagcaaagtcacatcttaggtagcggtggacaagagagcttgtgtagggaaactcccatttataaaaccatcagacctcgtgagacttattcaccatcatgaggacagcaccatcatgagaagagcatcattaaaacccgcccccaagttttaattacctcccaccaggtccctcccatgacacatgggaattatgggagctccaattcaagataagatttgggtggggacatagccaagccatatcagtgtcactaggcctttaagttggagcagtcctataagagggcatggaaaagtctaagtcaccttaaggtatgtttccaccagctctaagcctctattctccatcagtatgttaaggcatactgtttaaagaaatttttgttaaaatgaagtctgttgtctggcaggagtaagatcttaatattagctgacaattaagcacttaatttgtgcctaacattatgctaaggactgtacattggctctcttaatgcttattaaatatagtatggctatataatatatataatatataatacttatgaaattggtactattgtatttaatcatttttaagacacttttcacattttagcactctaaaattgggatgttttacaatcagtgactttttttgttgttgttattgttttgagacaaagtcttcctctgtcgcccagactccaggctggagtgcagtggcactatcttggctcactgaaggctccgcctcccgggatcacgtcattctcctgccttagcctcccgagtagctgggactacaggcgcccatcaccacgcccggctaatttttttgtatttttggtagagatggggtttcaccgtgttagccaggatggtctggatctcccgacctcgtgatctgcccgcctcggcctcccaaagtgctgggattacaggcgtgagccaccgcgcccggcctacaatcagtgacatcttacaaacataatttagagtattcttgttctgtaagtggcacataaaatcatggtgagagtgacaataagaaagcatcatagattagatgaaatatgatattagccaccatccccctttacccaatctgacctaaaaggaaccgaaacatgaagaagttaagtaatctgttcaatatcacagaactggtaaatgcttgagccaggattccacacaattgtttaactcaacccaggaacaatgcttccacacagcataccatgctgcctgctggtaatctaccagcacttcttaagctttggcgaaattggtgtatctgagtagccatcttcagagagctgcacactggagttgcagtggcacagtggagttgggaggagagagaatttgcaaggtccagaatggactgctgagtgaagaggcatggtggaagacccttggcagtcggggtaatcatgagtgaaatagaccctgaaaggacagaaaagttacaggaatgtagggaagccataaaggtggaggccacccattttactattttatccaggtccagacctgcgtgtgcaaatacatctatatgggacacagaaagaaaattcttatgtatcagggagagttatttatctatagctatatattatctatttttatatatttatccatatacgtatatctaaatccatatattttgagagacagaaaaaaaaagaaaaaagaaagttgtgcttttttttttttttttttatgatggaggcttactctgttgtcaagctggagagcagtggcatgatctctgcttactgcagcctccgcctcccaggttcaagcgattctcctgcctcagcctcccgagtagctgggactacaggtacacgccaccactctcagctaattttcgtatttttactagagatagggtttcaccatgttgggcaggatggtctcaatctcttgacctcgtgatctacccgcctcagcctcccaaagtttgtgcttttttaaagggaatattacattatgaataaatattttcttatcctacaattagaatttaagatttgatgtgttctgcatgtttcttttttatttgctttcccccccatagtgccatagcacaatttagtgtaaatattaggaagggcaagcatttattgaatacataaataataagaactctctctttacctcaaataccatacagaatcttggaagcttatttgagtttaacaaaaagatgctttaagtgggggtggggaacctcctaaagagttgtatcagttactgaaataacacagactagtgtaatttctattcctgcttgtcaagaaacaaggtaggcaaattaaagtcatcaggatctagcactgctgctctgcctccaacagaaaagatgagccaatgaaaagacaagccagtgaaaatacactgttactccctgtcagccccagtggccatatgcacaaacactatgcagaccaacacgtacacacacacacacacacacacacacacacatataaatttatgtattttcttttgcctatgtgtctagtcagcttaaatgggtcgactcgtgttttggctcctataaccaaaccagactctttggctcagctctacctgcaaactttctggcctgcttcagtatagtgaagtggtttaagtttctgagaacaaataattaggctctaggagaaggccaggattatacaaaacccattcgtttttgcttctgtgggttctgtgtctccgtaaaaaaggaaaacaaagttaggtaagaacagtgttcagctatgtgagcttcatgatatttctcctattatgttatcagaacacttatttaatttttgttgttctgaacctgagatacttagggattagtattttaagttacatctccttttaaccaacaatataaatcttagactcagaattagtgttggcatggaccggaatctgcccttatctttgttccctcaccttatctttgttacttatcttcactctttggacttaaaaggtaatgaagtttcaaactaggtttaggagcatcttcagctacagaaggcgagatataaggtatttatttatttatttatttaaacttactccactatctttctatggtactttctccatatcataaaaactttggagacctgtattattgggaagattgctcagctacaacagagactaagtgaggcactgacttcatcaagtgatttttggtgatcaagcagcaataaatgtgcccaatataaaccttctcttcctccagttcacaggcacaggatttaaatcaattttaagtggttttaaaatgtagcagagatttcactttttaggtattttttctttatcagagatataacttccaagagatttttctttattactccatttaggtgtttttccaaattatgaatcatctactatacttatttattaattgatactttagtgagttagagtgaactgcttgcgtcttcatttacccagaggtgaccactagtattatttttatagaagttacagatatttaatttcctaagaaaaccacaaccttgtctgttaagcttggagtgaggtagacagaggagagggcaggaagcacttttctcacattcaagctcaacatcatgtccagaggaaataggacagaaaccttctttcccagtcggggggctatttcctaagggaaagcagggaagtgagtgttcctttcctaagggaaagcagggaagggagtgttcccctcgatggctttattttctgtttttaatctagttcgtcagatggaattttatgattcaggaattatcagtgtcacctatgagttattaatagaatagcaagttattttgaccagtgaggtggaggaaaaggaaatgataataagagtaactgctcactttatgggacaaggagatgaggtcagaggagagtaaaaataatccatgtgaaagattatgtaaaagttagctagataggaattattctactcctttccccaaataacttttgtagggtaatcctaattccttaacttaaaaataaggacaaaattatgatagaaaactagtttaagccttagagaaccagagaagtgtgctttatctttcatttccatatttatcttcaccctttgctttttcaagctgtggacaaaaactccaccacctttagaggttctggcttatcctaataatttgaatctttccttattttggtttctaagctatcaattcattttcagcttaacctattctggagcttggtactgagactgcagagaagggaggtaagaaaacctcaacatttctaaagtttggaagtgaacattggacatattcctttatggttcaagtgcaatgttataactcttcaatggtgatttagtaacttgtcacatctgtgattttcatgtgtttattctgcttttttatttggagtgccagagagttttgcttgggtccttcaacaattgtcttggtctgatacctggcaacacaacataataatcaatctgggtttgtacttttcattggaatgctgaaaatgtacagtttggcaaagattggaagggcagttctatggaactacaccaactgaggtcattggccacatgaagatggccagatcttccaccagaaacagacaaatgatgagttttgaggtccaatgaagtggtcactctcataattatggcaaatttatgaactctgaaaacagttcaattgcatggccttcttggatttttgtacagcttgaatgacagacttgtagactctgaagctgatggtgacagagaagagagccatggtgaaataagaagccacagtgatgatgctgaaatctccagggaaagtagcatgatccatgtggggtgaagacaaactcagatttcttcactttttgtcaggaaaccagatggtgtattatacagaaagctgaagaacaggctcccaggcagcccctttatcacacctccttctcctgttgctgggcatggagtgtttgtccctcaaggacaaagaggaattagatggaattgagtggcctccaatagctttgccatgggctttttcagcaaggacaataggaaaagaaacaataaaataattacgccatgggttctcccaagtcccttcactctttccctccatgcttagacgccaactactagtaatgtcttgatagctgaccttctagattttattattttacataccattttgaacctttcttgcttaatatttcatttaaaaatctcttcggccattgtatttttcctcatcaaaaatattctccaaatgttttatttccaattgtctctctacccttgctccaatcccattccacacaggtagctaccagtaatattttgacttcaattattttatatgctaactggaattatagactgtgataactggaagagaccttggagatcatctttccatctttccctaccttctttcactgtcctaccactgcaggcttccagaagatatatagacaggctaaatgccccaccctaaatcccacctcagctaggaattgacatgggactagaacccaggtcttttcattgctagttaagggacctcaccaacctcatcccacaattttatatttttagtttgctggatgtcctaaagaagtagtttctgtaagacggatttgagtggtttatggccagattgaatttacaaggtgaccatccgtttttgaaggaaaaacaaacacacttctaaccaaatagaaatgactgtagttcatctattctgtccctcctttggcctccatgactggtcccacaggaccagcgttctgctttcctggagcagctttgttgtactgagattgtccttagatccatctatcacatggtaacgttggccttcttttctctttttttggtcacttgctttgggcataggcacagctctccatgcttttgcttcaaatgtttctagaaagatggaacttaaaccagctggctattggagttgctgatcttctgggtatcttctaaatattccacataaaaccaggattttctcctgatagagacattgtgtttttttattcatgtgccctcaactgagatttataatttgatcagtaaattcttacttaccttaaactctaggctggcctttttctttatatttatatatctatatctatatctatctatatatatatttatagattttttctttatatttttaagcagacccctccctagactttcactctaagttcaatttgaacacttctcacaccttcttttatagacataaaatgcacactttcacaaaataacactaataaaaaccttcagatctcattctacctccaccccctaaccattctcagaacttctcacttacctggcccacctagaagtcctaagatcactcttttccacactggcccagatctttggtctttgttcagggtccataatgtcttttgagttatattaagcatgcttactttaactatagtcagttctctgacacagacagaattcatagtgagttttggataaggtcttttgttttgttttgtttttttgtcaaggatccaaattgacccaacttgaatttttaaagaagaacatgtcaggggtggatgccaaagaggcccactctgcaaatatattttgcaattaacagagttcaagtgagctcttctgagtttggtggtggctgttgttgcttggggatctctttctttcacataagtctctgtctattgtttccctttgtgtgtgcttgtgtgtgtgctgtgggacatgataaacaagtatcattttgtttcatgtaattacagaatcatgcttttatgtttacctttcatatccactttaaggatagaatctgttttacaattgggactgcttctatgaccaattctgtagtgttgccttcagttcaggcacatgcctctgaaaccttaatcgcaaacagatgctgttctgaatcaagagtttccctctttggctactcagcctgagcaatgagctgcctgacttggatcctacaggcttcttgaaaaactccacaggctgccttactagcacactggtaacatgcagaagattgatattttccaggcccaagcaagactttgaaatagtacctagcagttgcagagagctatttattttcccctcctcccagaagtgttttcacatacatgatctcattttatccttcaaatagtccttggagttaagtaggaaaagcagtattttcccctaggaacctgaggtccagagatgttaagtaactcgctcaaggtcacacaattagccttgacttgtagtctgttattctttccaccaaaatgacactagcatttactttgtcttgtttcaaagttgttcaaagtcttttaggtgctggttggatccaagctgtcattcttatagctcagatttaaataaaatttgtaacatcttttagtgtttcatgtgtttttttttttcccctaggccttaagatgtgtctaaagtggtaattttgtggggccttaaaaattatgtgggagagagaacctttataaataaaagttgaaggaaaaaaattatttggggagcttgttcagtagatcatggttcaatagagcaaagatgcagtcgtaaatttggcattctataacaaaaaccacccatgtgattctgaattaggaggtctgtgtaatcactgttctcagagctaaagtaagcaaggcatgtaagacgtctgaggctcactttccttatttaaaaaacaaaggcaagactagaatcaattagtaaattgtctccagaaattaacatagattctaatctcctgtaaacttaacagctcgcatcagcattcttatgatggaagaaacagtatttgtctgaaaaaataccttggagttagaaagtcccccacaagggactgggttttctggagagggagggaggaagaatagaggagaatttattgaaagacatgaagttgggaactctgtaggttaaggaccaacagagaaatccctaggagtggatggccagaaaggactctggagaaagagggatgattggtatagagtttttaaatgtttgctctgtgatcttcatatagtcagtaaaatctatattttgtgtgactggtaactttcctataggaattcatgaagaggccgagctttgctttcagaatgacataatgcagaactgagcagaagagatactgagaatataagtcttgggaatttgcagaagtcttggggacagctttggatttctgcaaactagaactgaaggcttaaatcaacttcacttaactatccatgggatcaatgtgatccaggtgatgtctggggtaatatatgacaataagcatgaagatctagaaaatattatttaaaaaatactcttatggctttagaacaggggtctctggtaccccacagaggtaccggtctgtggtctcttaagaaccaggatgcacagcagaaggtgagctataagcaagtgagtgaagcttcatctctgctccccatcactcatagtacagcctgagatctgcctcctgtcagatcagtggcagcattagattctcatagaggtgtaaatcctagtgtgaactgtgcatgcaagggatctaggttgtgtgctccttctgataatctaatgcctgatgatctgtcactgtctctagtcaccctcagttaagaccatctagttgcaggaaaacaagctcagggctcctactgattctacattatggtgagttgtataattatttcattatatattacaatgtagtaataataaagtgcacaataaatgcaatgcatttgagtcatcctaaaactgtcttcctcccactggaccatggaaaaattgtcctccatgaaaccagtccctggtgcccaaatggttggaaactgctgctttagaaaaactaggataagattagatatctcataataaaggtgcacatcaagaaagtgaatgtgaacaaagatgtttgcaaacagagtacatgaagatcaagaaccttgagatgcagttccagctttggccagtttgcagaatgattttaactcagttttaatgtgtttgttccctttcccatgtaatttataatggtagttcacatggactgttgatgcttgtactctagcagccagaaccagaaaactgggaattttctacatctggaaatatttacctcgggatcttgagaaagagttcttggtctgaagaagcagaggatggggaggagcaaggcagagaacaacagaaccaaagtgttaatttccagtttagtaaagaacggacattttacatgaatgcaaggaacagaaatgtcctctttacagagaaataggcatccagatatgttgtcttaacgatactgggatactagactagtatactagagagtcgcaaatttagaggacaacaagattctactggaatgcttatgtcagatggtttcaatcctttcagtaaaaaaagggaattagcattatctgctgaaaagtaagggttgggattgtagaagtttgtggccttcaaaagaggtctgaactagttttggaagaatgaagctagggaggcagtgataaattaatgacaggacctgcccatgagtggctagggccaaagagttcctgtactgtcttatataaactgctaaaataaaaactccttctaccttcttactgtcaatgaaattcaattccctttgagaatactgcttacatggtttcttattctcaccaccctccctgcccagccccactccaccacagtgatggaaccaggagagaaaagcagagaaaataccaatattcctctggtgttctctttcaattattcttgcaattagcaaatatttgttgagtagctactagtctaggtgttctggtctaggtgctggaagaagcttattttaactcttttgataagaatacctcttttgaagcctatgctgtataaaaataccacctcttctttttgccatcttttaccaaattgcacatttgttgaaggtattgatgcttgtctttcaagtctggattatgggtatgagttgagtggagcattctttgagctgtccctctgctcttcagatgattgagaccataccctaaatctcttttcattaagccattgcatacaactgaaaagatttattggatatcacaatcttgctctgggacactttaacctattcagcaaatttaactatgagtgtaatggccatacccttgttttgatctttgcctcaaggttgagtcttgatcagcgtttgttgctcagttgtttattttaccttatgggattgaaaagcagttgctttctctaaccctgttaagtccccaaattcctggactttttcccttttattactgattgcatattggtcgatccttttctaagtacatttcttccttctaataccttgctatattcgttttctggagctgatgttacaaagtcacagaaactgggtggcctaaacactagaaatttattgtctcccatttctggaaactagaagtctgagattaaggcatcagcagagtgggtttcttctgagggctatgagggataatctatctgtttaagcctcttttctagcttttggtggtttactgacaatctttgctgtctcttgaccggtggatgaatctccctatttctgccttcaacttcacatggcactctccctgtatgcatgcctctgggtccaaatttcccctttgtataatgataccgattatattaggacttcctttaaataattatccgtatgtccaattctggtgtactggggattaaggatgacagtatatcttttttgaggagctaggaggacacagtttaatccgtgatacttaccaaatacagccaacagcaactacgacatgctactgacattctgttttctaacctttctttcctagggttacaagttagttaagtatatgatttgccttccaagttacctcaagcaaaagttttaacaaatgttaccagttttagcccgttctaaattttataaccaccaaaatacaggctcctaagccaatgccacgtattctttcacattccaatttgtggttctggagacaccaaaaaattaacataatattcacaatagttgccgatggaggctggaaaacatttgcaatattagactactaatattactcttaaatttataaatagtccatttgtactcttgctatctccctgcaaatgttagaggaggtgtttctgactccagatacttttttgcctgcaccagttattttagtttctttctttcttgctttctttctctttttttgtttttgtagttttgtacctgtactgtacttgtaggatcattttgaagagagaggaagtattacaattagtcctatgttcaaagaggtaaaagcaactagaaaagagaagtggcagcacagaaaagcagtagaaatatagaaccaattttctgagcatacagagaaagaacaaatgacttgtttaaaagggtccttttttaaaattatactttaagttctgggatgtatgtgcagaatgtgcaagtttgttacatatgtatacacgtgccatggtggtttgctgcatccatcaacccatcatctacattaggtattcctcctaatgctatccctcccctagccccccaccccctgacaggtcctggtgtgtaatgttccccttcctgtgtccatgtgttctcattgttcaattcccacttatgagtgaaaacatacagtgtttggttttctgttcctgtgttagtttgctgaggatgatggtttccagcttcacccatgtccctggaaaggacatgaactcatccatttttatggctgcatagtattccatggtgtatatgtgccacattttctttatccagtctatcactgatgggcatttgggttggttccaagtctttgctattgtgaacagtgctgcaataaacatacgtgtgcctctatctccttcagttctgctctgatcttagttatttcttgccttctgctagcttttgaatttgtttgctcttgcttctctggttcttttaattgtgatgttagggtgttgattttggatctttcctgctttcttttgtgggcatttagtgctataattttacacactgctttaaatgtgtcccagagattctggtgttgtatctttgttctcactggtttcaaagaacatctttatttctgccttcatttcattatttacccagtagttattcatgagcaggttgttcagtttccatgtagttgtgtggttttgagtgagcttcttaatcctgagttctaatttgattgtactgtggtctgagagacagtttgttgtgatttctcttcttttacatttgctgaggagtgctttacttccaactatgtggtcagtttttggaataagtgcgatgtggtgctaagaagaatgtatattctgttgatttggggtggagagttctgtagatatctattaagtctgcttagtgcagagctgagttcaagtcctggatatccttgttaaacttctgtctcattgatctgtctaatattgacagtggggtgttaatgtctcccattattattatttgggagtcgtaagtctctttgtaggtctctaaggacgtgctttatgaatctgggtgctcctgtattgggtgtatatatatttaggatagttagctcttcatgttgaattgatccctttactgttatgtaatggccttctttgtctcttttgatctttgttggtttaaactctgttttatcagagactaggattgcaacccctgcttttttttgctttccatttgcttgttagatcttcctccatccgtttattttgagtttagcaagactaataaagaaaaaaaagagagaagaatcaaatagacgcaataaaaaaatgataaaggggatatcaccaccaatcccacagaaatacaacctaccatcagagaatactataaacatctctatgcaaataaactagaaattctagaagaaatggataaattcctggacacatacaccatccgaagactaaatcaggaagaagttgaatctctgaatagaccaataacgggctctgaaattgaggcaataattatcccaccaaccaaaaaaactccaggaccagatggattcacagccgaattctaccagaggtacagagaggagctggtaccataccttctgaaaccattccaatcaatagaaaaagagagaatcctccctaactcattttatgaggccagtatcatcctgacaaaagcctggcagagacacaacaacaaaaaagagaattttagaccaatatccctgatgaacatcgttgtgaaaatcctcataaaatactggcaaactgaatccagcagcatatcaaaaagcttatccaccaagatcaagttggcttcatccctgggatgcaaagctggttcatcatacacaaatcagtaaacacaatccatcacataaacagaaccagtgacaaaagctacatgattatctcaatagatgcagaaaaggccttcgacaaaattcaacagcccttcatgctaaaaactctcaataaactaggtattgatggaatgtatctcaaaataataagagctatttatgacaaacccacagtcaatatcatactgaatgggcaaaaactggaagcattccctttgaaaactggcacaagacagggatgacctctctcaccactcctattcaacatagtgttggaagttctggccagggccatcaggcaagagaaagaaataaagggtattcaattaggaaaagaggaagtcaaattgtccctgtttgcagatgacatgactgtatatttagaaaaccccatcgtctcagcccacaatctccttaagctgataagcaatttcagcaaagtctcaggatacaaaatcaatgtgcaaaaatcacaagcattcttatacaccaataacagacaaatagagaggcaaatcatgagtgaactcccattcacaattgctacaaagagaataaaatacctagcaatctaacttacaagggatgtgaaggaccttttcaaggagaactacaaaccactgctcaatgaaataaaagaggatacaaagaaatggaagaaaattccatgctcttgggtaggaagaatcaatatcatgaaaatggccatactgcccaaggtaatttacagattcaatgccatccccatcaagctaccaatggctttcttcacagaagtggaaaaaaatactttaaagttcatatggaaccaaaaaagagcccgcattgccaagacaatcctaagcaaaaagaacaaagctggaggcatcatgctacctgacttcaaactatactacaaggctacggtaaccaaaacagcatggcactggtaccaaaacagatatatagaccaatgaaacagaacagaggcctcagaaataacaccacacatctacaacaatctgatctttgacaaacctgacaaaaacaagaaatggggaaaggatttcctatttaataaatggtggtgggaaaactggctagccatatgtagaaagctgaaactggatcccttccttacaccttatactaaaattaattcaagatggattaaagacttaaatgttagacctaaaaccataaaaaccctagaaaaaagcctaggcaatatcattcaggacataggcatgggcaaggacttcatgactgaaacaccaaaagcaatggcaacaaaagccaaaatgggatctaattaaactaaagagcttctgcacagcaaaagtactgccatcagagtgaacaggcaatgtacagaatgggagaaaatttttgcaatctacccatctgacaaagggctattatccagaatctacaaagaacttaaacaaatttacaagaaaaaatcaaataaccccatcaaaaagtgggcaaaggatatgaacagccacttttcaaaagaagacttttatgcagccaacaaacacatgaaaaagtgctcctcatcactggtcatcagagaaatgcaaatcaaaaccacagtgagataccatctcacaccagttagaatggcaatcattaaaaagacaggaaacaacagatgctggagaggatgtggagaaataggaacacttttacattgtttgtgggaacataaactagttcaaccattgtggaagacagtgtggcaattcctcaaggatctaaaactagaaataccatttgacccagcgatcccattactgtatatatactcaaaggattataatcatgctactatacagacacatgcacacctatgtttattgtgggactatacacaatagcaaagatttggatccaacccacatgtccatcaatgatagactggattaagaaaatgtggcatatatacaccatggaatactatgcagccataaaaaaggatgagttcatgtcctttgtagggacatggatgaagctggaaaccatcattctgagtaaactgtcacaaggacagaaaaccaaacaccgcatgttctcactgataggtgggaattgaacaatgagaacacttggacatagggcagggtacatgacacactggggcctgtcatggggtggagggatggtggagggatagcattaggagaagtacgtaatgtaaatgacgagttaatgggtgcagcaaaccaagatggcacatgtatacatatgcaacaaacctacactttgtgcacatgtaccctagaacttaaagtataataataaaaaataaaaattacaaaaacttaaaaaaagaaaataaaaataagaaaccatatgtttgcatgtgtcattatagtagactgatttatatttcagttactttctaatgcattgtgtcccagtagattagttcacatttgcctctttttttcctctatttattctgggccccataatctattacttgagcttgtccttcttcatcacccttaatactctcactttctgtttctctgctctgcttggcctgaaaaatgtcagcagcaaactatatctgatcattgtcatcctcctctgacatgcaacactattaaggatttatgaaggaaatacatagtaagctcctacacctttatgatgtttagttcaactgtgttctcaacactgctagggagtcttgcaagagttacctcactctctctcttttctctttatggatatgctgtataagcataagacacctcttaaagaataaccttgtttttgttatttattccactatgggaaacctgatctagtcagtaatttttcagtggttacttttagcttctgtaacattcttactacctgcatccatttgttccattttcctttctgtttcaatatccctcctcttgttcaattcagtcctttgccaaggtgttctatcctaccttctccacctctttaggagccttactccagcaaatgcctcctcttatccttcattttaaactctgactcttgattggctctttcacctgagcatactcattgctcagtttgtctctatctaaaaaatcatttttagactttatacctttattttctttgtaaatgtctttatatatattttcttataacctcccgtccctccttctttcttcccctctcccattgaaaatcaacaggatagtatttggagacttttgtttccctgggattgacacatctcacagctaagaatgaaagccatgaaatatctaatattctaagttcggagaaccactaggtcacctcctggacagtaaaatttcaatgtatgagcaacaaacaatcatgctaggatgtaaaatgattaaaatgtcactttctgagtattagacaattcatatggtttttaacaaacagtggctttatatccattgtaatgcctcttttagcatcaacattcagaaattcacattccatttttttggacacttcatgagattttgaaactactctttattctgagattctgttaattgtatttagaatggaccttgatagttttcctgctcataattttggtaaaactgtattgcattttgaggaagttaatatcaaatgttcctatataaactttgactagaaaatgatgtatggagatattcacacatctataaagtttggttatttaaatccaagagatgttttgtcatgaatatcttaactacagagacatggagctgcttggatagaacaaactctgtgctttaatggttgtatagtattcttttcatatgtatatctgtaattttacttctgtttagccattttcttctttttattatgtatacattttttatttctgtagcttttggggtacaagattttatttcatggatgaattgtatagcggtgaagtctgagattttagtgcacctgtcacccaagtagtgtacattgtatccaatatgtagctttctatcccttactcttggccccttctgagtttctaaagtccattataccacttggtatgccattacatacccatagcttagatcctacttataagtgaaaacatatggtattttgttttccaatcctgagtcactttacttagaataatggccctaagttccatccaagttgctgcaaaaaaaccccattatttcattcttttttaatggctgagtagtattccatggtgtatacatactgtattttcttaatccacacatcagttcgtggacacagattggttccatatctttgcaattgtgaatgaattgtgttgtgataaacaggcatgtgcacatctctttttgagataatgacttattttcctttcggtagatactcagtagtgggattgctggattgaatggtagatctacttttagttgtttaagaaatcttcatactgttttccatggagcttgtactagcttacattcccaacagcagtttaaacgttcccttttcaccacatttatgccaacatttgttgttttttgactttttaataatggtcactctggctgggttagatggtatctcattatggttttaatttgcatttctctaatcattagtgatgttaagcatttttcatttctttattggtcatttgtatatcttcttttgagaagtgtctattcatgtcatttttccactttttgatgggattatttgtttttttcttgctgatttgcttgaattccttgtagattctggatattagtccttggtcagatgcatagcttgcaaatattttctcccattatgtgggttgtctatttactctgatgattatttctttcgctatgcagaacattttagttcaattaggtcccatttttatttatttatttatttgcttttttgttcatttacttttggggtcttagtcataaattctttgtcgaggccaatgtccagaagagtttttccctaggctttcttctagaatttttaaggtttcatgtcttagattatgtctttaatcttgatttgattattgtatgtggtgagagatagggatccagtttcatccttctacatgtggctatccagtttcccagcacaatttactgaatagtgtgttctttctccaatttatgtttttgcacactttgtccaagattagttgcttgaaagtatttggctttatttgtgagttctttacactggtcccatggtttgtatctctccttttatatcagtaccatgctgttttggttactatagccttgtagtataatttgaagttgggtaatgtgatgcctcctaatttgttctttttgtttaggattgctttggctatctgggctcttttatggttccatatgaattctaggattgtttcttctaattctgtgaaaaatgatgttggtattttgataggaattgcattgaaaatgtagactgctttgggcagtttggtcattttcatgatattgattcttctaatccatgggcatggggtgtagttccattcatttgtgtcatctatgatttatttcagcagtgttttctagttctccttgtagaggtctttcacctccaaggttaagtatattcctatgtgttttatttatttatttttgcagcgattgtaaaagggattgagttcttgatttgattttcagcttggtcataagaagcaacagtatgcttccagtcgcctctgctcctttatgttattattgtcacacattttagttctacatatgttagaaattccacactacattattattatttttgctttacatagacaacaatcttttaaataaatgtttaaaaaaagaaaaagttatgtatttatatatatctttaccatttatggtgctcttattctttgacattgatacaattttcatctggtattatttttttctgtctgaaaaactttaatattctttaatactaatcttctgtgatgaatctctcaacatttatatgtctaagtgaaatatgttaatttttaattgtttttgaaggatatttttactatatataaaattttagattgacaatttttttttcttttagcaatttaaagatgttatttgattgtcttctagcttgcatagtttacaatgagaagtcttcaggtactcttgttttttgtttctctgttcattatgtgtctttttcccctctttggttgttttaagattttctttttatcatcagtttttggtaatttatttatgatatgctcagtttgctcctggatttgacattgcttgcttctagacctcagacagtttcttttcttgctatgtgtgtgagccaccacacctgaccgagtgtctttattttattgtcttccttcaataattgttgggctttgtttcagcaggtggttaattcacttggagatctggttgacatttttgaggaccattttaaaaacagatatagtgcatctagaatagtaactctggatcactagcatttctattgtttcttttcctgttggtttcagttgtttctatttccttttacactttataatttttaattgaatgataaacatcacatatgagaaaatcgtagagataatttgaccgtcttatagacacccctttttgctaaattttcagactctagaccctgtgacactaacgaatcagcaaatgtattcagagaaaaagagggacagaattttgtgttttatctcagttcacttcctggtttttgaagagctttatctttcatgtcctgactgccttgatagttttgaatgctttcaaacagatgttttaattttatcgaacttttctagcttttcttatagggaggtttgattcaatacaagcttttccatggaaatagaaattttttatattaattttgaacctaggcattttattaaattatcttatctataattactttttgtgtgttttccaactgtacaaattatttgcaaatgcttctcattttagaattttgcatttcttatttcaccagactagtccaattgaataggttagtactttcagaaaaattttagataatagttgtaaacaggaaaaactatattacatttatgtcacaaggttgttgtgatgactaaattaaaacatgtaaagtacctagaaaagaatgacggtaatgatagtgatgatgatgatggtgatgatgatgatggatatccttgtgttgtttctgactgtaacaggggtgttcctacggtttccccactaagaattatgttaaacatacaaggatacatttacctattctttttttaattaagaattttcatctcaaatcaatattgaattttatcaaatgtctttgtaggacatatggagaagaccatatgatttttcattttgattcattaatatggtgaattatatttattttctcatattgaatcagaactgtcttggtaggagccccatttaatcattttgtggtattctgtaaatatgctgctagattttaattttaataatttatttaaactgttttgtattactactcatatgtgaaattgatctatagtttttctttttgggctgctcatttcaggttttggttctattatgtttttataacaaatatttgataagttgttctttttcaatgctttgacacttttaattagcactcatgtcactggtttgtaaaagcttgggagaatttagttaattaaacccactgggcctggtacttttctttctctttctctctctcttttttttttttttttgtagggtgatcttaatttttttttttttattacatagtctatctcttttgggtcagttttggcagtctgttttcccagaaaacaatctatgtctttcaagatcccaagtttatttacatagaattgactcagttgattttctgtgtagacatgatgtgcaaaatgttgaaaacttagttggcatgggcattaataactcatagcagatgctacaaccaaccacaatatatatcaaacacaaatatctgatatggtcataatagtgcctattggctaagtattagccattgtatctgtatttattctctgtattattttcccattctcacttcttattttatgattttattctgtcctttttttgattaggtaagctaataatttatctatttcattattttaaacagtatgctcttggctttatttgttattttatcttttttcttgttttctaatgaatgaattgtttgtgccttatttaactcattttattttcatcaggtttacttcatttctctctttatgtcttgtgtgattttattttgttttatgaatatatgttttatgaatttatatcagattgatatatatacatatacaggtcattttatcccattaatgtaagacagataaatttttgtcatcatattttatatatatcgtgatttcagtttatattggttctttgtttaataatctttttatataatttgttttttattgcttttgtgtgtatgcatgtatgtattcacaggcacatctatgcatgcacatgcttccttgtaattcaaagatttattttaaattctgttagtggtcatcttaaaaccttgcaatttaatatgctttagcatttattccagccagtgtctgttgattcaccattagagcaatgacatttggtagtactcttctactttagtggttctcagcactggtccacattagtatcatctgggagcttttaaaaaataccagtgcctctaagattaagagataattattttcaaaaagtcccccatatgactttaaagagcagctatagttgagagccactgttttaccctctctcccctccaccaacaattttaatcaattatatattatttaaaaatttttttctagtctttatgtttttgaaagatgattggccgtatgtaggagaaaatacgcatacttgcacatcttctgtcttctctctttctcaccttcatctaatattatcattcattcttataatttgtaacctatgcattctgttttgctgccatctttatccgtgattaaatagattccatagtcactgtgagtaatttttctccattcattttttgattgactgaagtttattgtctagtaggttcttcagaagtgttcatggaagtcacatctatctgtttcctttatatttaaatgacagtttggctggatatagaaatcatggatcacatattattttcctgggttctttgtatcatatttctgtcttccagcatcaaatattgttgtgaactataaggtcagtctaatttttcttctttgtattaagtatgggaaagaaactaatactgtaacaaagtacaaaaatacagtgagttaactaagattcaaccttgtatcactctcatgtatcagtctggctggtctaagttatcagagcaactgctgcgcaaggtcacccagagagccatttcttccatgttgttgctccactatccctttttgggcattttgtcaccctcaaaatcaaaagtgggatgttggcaaatctaccttccagcttgcaaaagaggaaaagaggcaaaatacagagaaagcagattttctttaaattgcaaatgactttacatacttttgtacatattcaatattcagaacttgctcatggccaccgtagctaactgaaaaaaaaagctagaaaatgcagtatctagctgggtggccttagagttagaaatagaaaatttaggaagaacaaatatgagtccacttcaaacttgtaggttacttaataatcttagcctgaatgcccaaagtttttgttgttgttgttttgacatttgaagacctatactatcactaggaaatgtttcagcattgataaaattgcatgaggttttctgcttttttaattttggtaaggattttcggtttaagctataggttcttcaaaattatgtgttaaattttattttatgttttatttattgtgtgttccccccaccaccctattttttttttttttggtctgttttccatgtctattattttgcttgctttcctcaatcctgctcttttgtgccttagtatgaattcagtgatggctctttgtgctgcttaatgtagccttgatttcttggatggctttatttatttatttttctatttatttttcaagtctgccagctcatgtttcatctcctccagctgtctgctttgagctttttgattcattaggtgcctagtattcacggccatatttatttggtcatgatttttatctgggcagtgacaatattgttctggtgtgtattcatcacctgccacttgtttttcccacatttttcttccttttcctgaaagtaactttgtatagatccttggctggttctttttgtgttatttcttttgtgaatgaggttaattcctccagttattttcaagaggttccttcaggggagagaatagagtagtgttccaggcaagcagtaactcctccacagtaaagctccttatgactcaggggtgtgtgtgtgtgtatgtacactattttaaccttcgtttttctctagttcaaagaaatcagcaattgctggattactcataattcagatccatttccttcacccttcctcaaggatacactgcttctcagaaatgtgtgtgtttccttgttcagcctcaccttccctgcctgttctctgggctcagagaaggtccagataagctccctctaaagaccaggcatcctgttctcattgttctagacaaggtttgtggttttgcctctcatattgtgtcacatactttgaactgtactctacctggtttagttgagacttttttttttttcgagacggagtctcgccctgtcacccaggctggagtgcagtggcgggatctcggctctctgcaagctccgcctgccgggtccacgccattctcctgcctcagcctcccaggtagctgggactacaggcacccaccaccatgcccagctaatttttttgtagttttagtagagacaggatttcaccgttgttagccaggatggtctcgatctcctgactcgtgatctgcccaccttggcctcccagttagctgagattctcagccacagatgtctataggtatttccctgcactcctgtttgaacttccctgttggcagctcttactcaaatattgtagttcgaggttacagatgtgttataactttatcaaaaattattatttttttcttttttagttttcatcattggtttgagttgattttgtaaagaaaactatgtggagccatctttagtttggcatttcctaatcagctaccatgagtatttatttagagaaatccattattattttgttaggattcatttttctaagtggtaaatttacaaaatttcaagaattccaatctgcatttcaaaaagattatacaaatctatactcttctactcatatatcagagttactattttcctacacacttactaatatatagagagaactttgcctatttgatattctaacaaggtgtacctcttaagttgtacttttaattattaggggacaaataattatatcttcttctttttttttttttttttttttagtatttattgatcattcttgggtgtttctcggagagggggatttggcagggtcataggacaatagtggagggaaggtcggcagataaacacgtgaacaagggtctctggttttcctaggcagaggaccctgcggccttccgcagtgtttgtgttcctgggtacttgagattagggagtggtgatgactcttaaggagcatgctgccttcaagcatctgtttaacaaagcacatcttgcaccgcccttaatccatttaaccctgagttgacacagcacatgtttcagagagcacggggttgggggtaaagttatagattaacagcatcccaaggcagaagaatttttcttagtacagaacaaaatggagtctcctatgtctacttctttctacacagacacagtaacaatctgatctctctttcttttccccacatttcccccttttctattcgacaaaaccgccatcgtcatcatggcccgttctcagtgagctgttgggtacacctcccagacggggtggcggccgggcagaggggcccctcacctaccagatggggaggccgggcagaggcgccccccacctccctcttggacggggtggctggccgggctatatcttcttttgggaattttccattattatcctttagtgaatattgtttccttttgatgcctttgtcaacttcatatagatttatatgagctttttcttaaagatatgttgcatatatttttctgttagtaatttgcaagtttattttaatgtaatcttttaccaaatgaaaatatatttttatagcaagtttaatattttcccttgtggtttctactttaggactcattttctttaccacagcaaaattatatatccacgtatatattcctttagtgtttcaatgttgttttattttttgtacctaaatctttaataagtctggaatttgttttgaatatagtataaagtactaatctagcttatttttcccaaaattgttagttatgtatttcattaccatttatagagtaatgtcttcttccccacttatttaagatgccactactaacacattaatcttaggtttatacagaaacagttctaaactttaaattttatttcattgtttgcttgtttttatggcagcactgcaacattttaaccattattttatatattaatgcattttattttctagcagggcaaatctctaccattactagaattttcaaaatctcttacttagtttcatgtattattcttccagatgaactgtggaatcatttgttgagtttccagaaataaatcctcgaacccactgggattgtactgagtttatttatttatttgggaagaattaacatcttgacaatattaagtcttcttagctggtaacatgatatagttctccatttagacaagttttcttttatgttcttcaacaacaatattgtggttttcttcacagaggttctgcacatttctcatgagtttaactcttaggtgatatatattgttttgctattatgaatgcaatttattttccaatccattattgccaaatataagaaaagattgagctttatttattttgtaattactactctacaaatatttcttacaaatcctagttgcttttcaggttattcttttgagttttatatctagatagtaatgccattttcaaacttagtttttcctcgtgtccaatattcatactttttaacttgctttcttattcaattgcactggccaactttcccagaacaatgttaattaacaatagagttagcaggcatactttacttattcttgattatagtagaataaattgattgttttactgtcgttttgatgtttaatgtaaaagtacattgtgatggttttgcagtgcttgtgtagaccacacgaagttggatctaaaaaaattttaattttttttgcttaggattgtcttggctatatgggctctgttttggttctatatgaaatttaaagtagttttttctaattctgtgaagaaaatcaatggtagcttggtggggatagcattgaatctataaattactttgggcagtatggccattttcacgatattgattcttcctattcatgagcatggaatgtttttccatttgtttgtgtcctctcttatttcattgagcagtgttttgtagttctccttgaagagatccttcatatcccttgtaagttgtattactaggtgttttattctctttgtagcaattgtgaatgggagttcactcatgatttggctctctctttgcctattattggtgtataggaatgcttgtgatttttgcacattgattttgtatcctgagactttgctgaagttgctcatcagcttaaggagatttggggctaagacgatggggttttataaatatacagtcatgtcatctgcaaacagagacaatttgacttcctctctttctatttaaataccctttatttctttctcttgcctgattgccctggccagaacttccgatactatgttgaataggagtggtgagagagggcatccttgtcttgtgccagttttcaaagggaatgcttccagtttttgtccattcagtatgatattggctgtgggtttgtcatgaacagcttttattattttgaaatacattccatcaatgagatacattctagtttattgagagtttttagcatgaaggggtgttgaattttattgaaggccttttctgtatctattgagataatcatgtggtttttgtcattggttctgtttatgtgatggattatgtttgtttatttgcgtatgttgaatcagccttgcgtcccatggatgaagccaacttgattacagtggataagctttttgatgtgctgctggattcagtttgccagtattttattgaggattttcgcattgatgttcatcagggatattggcctgaaattttctttttttgttgcgtttctgccaggttttgctatcaggatgatgttggcctcgtaaaatgagttagagaggagtccctcttcttctattgtttggaatagtttcagaaggaatggtacaagctcctctttgtacctctggtagaatttggctgtgaatctgtctggtcctgggcttttttctggttggtaggctattaattactgcctcagtttcagaacttgttattggtctattcagggattcgacttcttcctggtttagtcttgggagagtgtatgtgtccaggaatttatccatttcttctagatattctagtttatttgcatagagatgtttatagtattctctaatggtagtttgtatttccgtggaataagtggtgatatcccctttatcattttttattgtgtctatttgattcttctctctttcttctttattagtctggctagcagtctatctattttgttaatcttttcaaaaaaccagctcctggattcatggattttttgaagggttttttgtgcctccatctccttcagttctgctatgatattagttatttcctatcttgtgatagcttttgaatttgtttgctcttgcttctctagttcttttaattgtgagcttagggtgtcaattttagatcttttctgctttctcctgtgggcacttagtgctataaatttccctctaaacactgctttagctgtgttccagagatcctggtacattgtgtctttgttctcattggtttcaaatagcttatttatttctgccttaattttgttatttacccagtattcattccggagcaggttgttcagtttccatgcagttgtgcaggttcgaatgagtttcttggtcctgagttctaatatgattgcaccgtgctctgagagactgcttttcatgatttccattcttttgcatttgctgaggagtgttttacttccaattatgtggtcagttttagaataagtgtgatgtggtgctgagaagaatgtatattctgttgatttggggtggagagttctgtagatgtctattaggttctctaggtccagagttgagttcaagtcctgaatatccttgttaattttctgtctcattgatctctctaatattgacagtggggtgttaaagtctcccactattattgtgtgggagtctaagctggaggcgtcatgctacctgacttcaaactatactacaaggctacagtaaccaaaacagcctggtactagtaccaaaacagatatatagaaaaatggaacagaacagaggcctcagaaataatgccacacatctacaaccatctgatctttgacaaacatgacaaaaagaagcaatgggtaaaggaatccctatttagtaaatggtgttgggaaaactggctagccctatgcagaaaactgaaactggaccccttccttacaccttatataaaaattaattcaagatggattaaatacttaaacataaaacctaaaaccgtaaaaccctagaagaaaacctaagcaataccattcaggacatagacataggcaaagacttcatgactaaaacaccaaaagcagtggcaataaaagctaaaactgacaaatggatctaattaaactaaagagcttcttctgcacatcaaaagaaactatcagagtgaacgggcaacctacagaatgggagaaaatttttcaatctatccatctgacaaagggtaatatccaaaatctacaaggaacttaaacaaatttataagaaaaaaaatcaaccccatcaaaaattgggcaaaggatatgaacagacacttctcaaaagaagacatttaggcaacccacaaacttgtgaaaaaaagctcatcatcactggtcattagagaaatgcaaatcaaaaccacaatgctgtaccatctcacgccagttagaatggcaatcattaaaaagtcaggaaacaacagatgctggagaggatatggagaagtaggaatgcttttacactggtggtgggagggttaattagttcaaccattacggaagacagtgtggcaattcctcaaggatctagaaccagaaataccatttgacccagcaatcctattactgggtatatacccaaaggattataaatcattctactataaagacacatgcacacgtatgtttattgcagcactgttcacaatagcaaagacttggaaccaacccaaatgcccatcaatgatagactggataaagaaaatgtggcacatatacacgatggaatactatgcagccataaaaaagatgagttcatgttctttgcatggacatggatgaaggtggaaaccatcattcttggcaaactaacacaggaacagaaaaccaaacacatgttctcactcataagtgggagctgaacaatgagaacacatggacacagggaggggaacaccacacactggggcctgtcaggtggtggggggcaaggggaggaataggattaggagaaatacctaatgtagatgatgggttgatgggtgcagcaaaccaccatggcacgtgtatacctatgtaacaaacttgcacgttctgcacatgtatcccagaacttaatgtataatacacacacacacacacacacgcacacacacgcacaaataaattcatacaattaagtgttttttaaaaagtattttaatttaaattcccatctaatcatttttttaaattggtgtgtcaattatttgcctttaaagtaactattggtttggttgcatttagatctacctttatattattactattattattattttacttatcctctctggttttgtcttctattctttttacctgctgtccttttctgatagtctatttttgatttctctattcacttgtgttctatatctctgtattttttagcacttgctctagagattatacacataactaagttatctttccaattaaaatgcagagcaaaatttggagccacatgatgttttggaccaaagaatgaaattaatctgattatgtcttaacaagataactttgttgttcttttgagaatagattttacaggtacaaaggctaaagttaggagatgaatgcaaatatacaggagtgtctttctattactctttactgagagtttttgtaaaatcaggaaacagtgttaattttataaactgctttctctgcttctattgaggtaattagtgaggtggccattttattctgttaatgtggtgaattatgttgatttaattttgaatgctaaatcaacgttgcatttctgagataaaccccacttgctcatgaggtactattctttgtatatattttctgatttgatatgctaattttttgtgaagatattttgagacaataagcatgagagatgtgggtctgtaattttccatgttttgcaaggttcttatctagttttagtattacggtgtgcttgtctcatacaatgaattccctcctcttctatgttctgaaagatctcacattagactaggattaatttttctttcaaagtttaaaagaattccccattgaagccatctgggcctggaatttattttatgtaaagaattttaattacaaattcaatatatcttttacagatacagtagtcctcccttacccatggtttcactttctgcagtttcagtggaacatgaacatggtcaacggtgatcagaaaatgttaaatggaaaatttcaggtataaacaattcgtaagtttcaaatcacacaccattttgagtatcataatgagatctgttgccatcctgctgtgtcccaccaggatgtgaaacagccctttgtccagctgtcagtactatatatgacacctacccattagccacttactatccctctcttatcagattgactgtgatggtgtcacattgcttgtgttcaaataacccttattttacttaataataaccccaaagcatgagcatagtgatgctggcaattaggatataccaaagagaagtcaaatatatgtcaaagagaagttgttaatctcttactgtggataatttataaagtaaacttaatcataggtatgcatgtatatgaaaaaccatagtatgtgtagggtttgatattgtctatggtttcaggcattccctgagggtgttgcaatgtatgcccagtggattaaaggggactaccttagaggagtattctgttttttttttttcttaactatcttcctgtgtcagttttgtaatttacgtgtttcaaggaatttgcccatttcttctgacttgtcaaattaattggcatttagctgttaataatattcccttattattatttaactatttgcatcatctatagtgatgtgccttccttcattccagatgctctctttctttttcttttttttccccttttattttttggtcagtcttggtaagatattaccaggtttattaaactttgcaaaaaactagcttttcgttttattaatttttctcttgtttgtgttctatttcattgatttccattattttattttttagttgcctacattttcatcctttaggtttaattttgtagagttttgagggaatttaagagttttcaacctttctccttttttctgaagtaagctagtaaagctacaaattaccttctacgtgcttctttagatgcctttcataatgtttattatgttttgttctcattttcatttatttcaaggtattttaaaatgtctttcatgatttcttctttgattttggatcctttagtactgtgttgcttaattttcagatatttggggtatttttttcaagatatatttttgttattgatttttaacttagttcctttattaatttctaatttagtatggtattaatccttttaaatttatgcccaatatatgacctatgttgattaatgtaccatgaatacttgaaggattatgtattctgtagttgtttggttatagtgttctataaatgtcaatcagatagtattggttgataatgattgtttcagttatctattgctatgtaacaaatgtcccccaaatagtagattaaaacaacagcatttatttggctcaaaattctgctattttggcaagtcttggtggtaacagtttagttatgttacattcagcatcagctggagtatctcaaaggcagactccactcagtgtcagctagtttgtgctgaattaaaggctataagctgggaatctctctctgttttaaaatgatctctttatatggcctctgcaatggctttggggaagcgactggcttagagctcctaagtttcatgtcacgagagagacagagccaagtagaaactgtatcaactttttgacctagtcttggaagtcatgcagccctacttctgctgtgttccatttgttttggtggtcacagagtactgtccattttgacaaagagaggggatatagacttcacctcttaatgagggtatgactaggtctggaagagtttgtgggacagtaaatcttgctgagaacatttttggaaagtacaattggtcataatattgatcaaatctttttctaatcttttttacccttccaataatggactgagatctttttctaatcataccaacttttagaaaattgatttctgggagtagtgttaaaatatcatactggatgtaggaacttgtacatttatttctttagttttgccagtttctgcatcatttatcttggcttgctattgattgcatacacattttagattatgtctttctgtttgttatacatatgttacaaatacaatgaaacacttttatatttgctttagccaatttttaaataaattgagaaatgagagtcatttatatttacccttttttttcccagtatacttcattcctcgtagatacaagtttctgcatggtatccttttccttttcttttttttttttttcttctttttttgagatggagtcttgctctgtcaccaggctggagtgcagtggtgtgatctcagctcactgtgacctccacctcctgggttcaagcgattctccttcctcagcctcctgagtagctgggactacaggcatgcaccactatgcccagctaatttttgtatttgtagtagagacagagtttcaccatgttggccaggatggtcttgatatcttgacctcatgatcggcccacctccacctcccgaagtgctggaatgacaggcatgagccaccgtgcccagccagtatcctttttcttaagcctaaggttcaggtcttgcccctatttatgaattctctcagattaaaaaaatctaaatatatttgttttgccttcaatatcaaaactttttttctgaatatagaattcttgttgattatgttttcagtactttaaatatgtcacattttattgtcatctggcttgtactgtttctgatgagaagacagcaatcattcctgttgctcacctgtatgtaatatgtcttttaccccttctgtgcccttttaacattttctctcactccttgtctttcagcagttttattgtagtgtgtccatgtgtggttttatttgtgtttatctgattagttaaacttcttggaaaatatgagactatagtgttttttaaatttccccctctgatatctttttcctctccctctagaactctaattacatatttgttagattatataatattgttccacaggccactgaggctgtgttcacttttctaatctaaatttcttctttctatgctttagattgggtagttcttttgtctaatctccaaagctaatctttctctggcaatgtatactctagtattaaggctattaggtgaaattttcatttcagataagttttttagttctagaattttcattcctttctccacccaagttttattctcttttcagtgtctgtatctgtttacttactacaatcatctttgtctttaatacttgaacatgtttaaagtccttgtcggttaattccaacattagtgccatctctgggcttccactgactttttcctcctgtttttggctcttgttttcctgcttcttcatatgtctagtaatttttattgtatgctggacatttatgatgctatgttgttacaaatttgatagagtatgccaagagcatgtattccattaagcaaggttgagttttgttgtggatggcaggaaatatattcagtcatctttatcctacttgattttaagctttctctgggtgggtctggaatagcccttaatctagtgatagagtaactcttcacttaagaaataccctttctgggatccaaactaaatgtccaaggtattcccaaatctcttcattctggcttatcaaaaattgaacatcttcggcattgtaagagctgtgaagtttgcattaatctcacagtcttttagtagttgttccctaaccgatctcttggagtcttgctctgtgcatgcatagcttaatattcatgcagatactaaagtggatctctatacaaacaaatgggactataattctatgcagctctctcttctctgttaacttgcctcacacatttcactttgctttctctattaggcaagatatctgctctctatttgtgatctacttctctgtgctactattcataaggtgcccacaggcaaaaaaccagggagaacatgaagtttaccttatggatttttttcttctctcaagaattgcacctgtactgttttcttccagtgtctgaaggccatttatttatttatttttgttgaattttagagttgtttgttgtaggaggataaatattatatgaattatttcatcatggcataaactatatatctagacatgttaaatctgagatgtctattagataaacagatagtgaggtgtgatagactgttgaatacatgaatttggagttcaagggtgaggtccatgctggagtcatacatttgagattcaccagcatatataattcatataaagttttgaagtgaatgagatcttctagggatttggtatagattgagagaagagataagggctgagcccctgggcagctttaaaatatcaggaagatcaggaaaaattagcaaactcagaaacagcaagtagataggagcaaaactagtagagtgtaatgacctagagaagaatatattttagggaaaaggtaatattcaactgtgtaaaatagtgctaattggtcgagtgagataagaatgtggactcaccattggatttgtcaaacactggggtcaaaatggtcttgacacaagcagttccagtagagtgctgggaatgaaggcctgattggaatggattcaaaataaacgtggggatggggaggattgaagacagagagtatgaagaacttgttcaaagagttttgctgtaaaattaagaatgtgaagattatgtgaaaaataatttaaatataaatagcaagcattgtaatacagtaatcacttgttcttgaatgtttgccagaactttactgggaaaccactggacctgagctactttggatagaggattaattccaggaatatgctggtaaatgttcaacaactaggtctctgaaaagaaaaaaccttgttttgtagccgttgccaatttctgtgatgtaaatattcccatcatggtagatttcaagctataaatgtgatgtcgctgaaaacagagttgggaagacatgcatgcaatccactctcaagagtttagtatatcactgagtaatttctggtcatcttttctaatttactgtatgattattggtatgtttagattttttttgagatagggtcttgctttattgcctagactggagtgcagtggcatgatcacagctcactgcagccttgacatcctgggctcaagcaatcctcccacctcagcctcccgagtagctgggactacaggcatgcaccccactgtcagctatttttttaaaaaaatttttgtagagacaggtgttcctatgttacccaggctggtctcgaactcctgggcccaaacaatcctcttaccttagccttccaaagtgttgggattgcaggtaggagccaccgcatctggcctagatttttattttacttatttttgatttggctttaagaatttataattttctggaaaaatcattcatttaagttgtcttatgttgttactgacagtagaagaaatataatgaagaatgtgagtgatttaggaatcacataaagttttgtttatacccttcatttgtgtgaaaataattatagtacattaaaaaagaaattcttgttgaaagcataaatatggtctacttttatcactctttttatagaagggaactatatgatatacaagaagtataaatatggaactccttttaatatacaagaagtttgaatatggaacttatataagatggacaaataaggttgaataggacctgttatattaaaaaggctggccgggcttggtggctcatgcctgtaatcccagcactttgggaggcctaggcaggcagatcacctgaggtcaggagttcagaccaacctggccaacacggtgaaaccctgtctttactaaaaatacaaaaattagctgggcatggtggcatgcccttgtacagaagaaagacttaattgaaatctttgaaaatcctaaaccagcataacaagactgaatactaacatgttgtatcttgataatgcacatatttttcactttatacttgctttaaggatcttgtataattctactccaggtgtggatgctgaaactgatgggcatgcaatgaaagctggtatgcagaaaaaattcagaggtggttttactatcttggtattcagttacatggttttattcccagtcttaatctaagatcaaggacaaggttttgtaggcgattgtgtgaaatagaagtatgtagatgaaaatatttgaaattaaagtataagggaggacaacaatcttaagtgcattttggaaatatttcaaaagcatcttaaagcagtatagttaacttgtgagactattttaataaaattggttcatttttgaccaaatcttcgagtccaggagtttaagtcaatataatcttttccttagctaccattagagagaaaggagaacctaataacttggtggcgacattaccacaatagtactttgtgtcagcagagttagctaaaatatagcttgcttctccattgacttcacctgaaaatgagcctcgggcctttcatatgggaactgtagtggctagaggagcaatttagtagctaattgcaaaattatattgagaaattcttcatgcatgttaaattttttttaaagattactaaaacctttaataaaattgtaatagcttttacttttgaaagataaaatttcaacttaatcttgtagctcagaagtttattctatgatagtgacatttgattttggctggatgttgattctaatactttgccctttgtcatacagctaaagtacatattcagtaatggatatgaagtaatatgtagttcaataatagaatgtgtttttttcacagttttgaagacatacaatttgtcttccaggtgttgctactgagaaattcaataccactgggatccctcatcttatgcataagaactattacctctggataaatttaggaacttctgtgtgtctctgtcagcataaaatttcataactatttgctttggtgtgggtccggttatattcattttttttagagactcagtaatttcttcccactgtgaactagtgctctttagctttgagaatttcttttgtattttttctttgataatcttttcaccattttttttttctgttctttattctgtaaactattatttggtcatctcctggagctcctgagctgatcctctaatttttctcttctttttctcctgtttttcagctttttgtctttttaaaaaatgatttaattatctgttgctgctaaacagattaaatgactcttcatcttttagtttacttcctagggacttcttcaagtttatcttctaacccttccactgagttttcatttatcctaccatacttttaatccctaagaactttgtttttatattttgtttttgctcatggatgtagtatcttatggaagatattaattatatttctgagattttattctgcttttagaatggattcctttcctccaagtttctccttctgcctcttggtttgcttctgtttttttctctttaatgttagagtctttccttacatgtctgctgctcttggtagtcccagcacactttagagctaagaggttttgtgtttgtgtgtaggttttaaatggtgtgcttcatgtttggttatagaaatgggccatttctttgggagacttcctacctttggaagtctcccaaagaaatacacacacacacacacacacacacacacacacacacacacacacacacaatcttcagtggtttaattttcccagagcaatattcgttcagtcccctgcctgagagttaaaatctttgctaccagtattctgggaatcaagttggaaatggaggctcccaaatatcaccattcacgatatactttccaacattttcccagtttttttttttttcttttagtagcacaccttatctcaattctctataagcctggtgctactaagtctggttcagtatgcaagagaagaaagccttcaaccttcttccaaggtgggggaagagtattcacccagatgtggagtgaactggagagctaggaatcctattgtttcttattcagacttgccatcagttcacccattttcagcttcaccttcatagtcactttctgggatacctgaggtttccaattcctcaggccctcttggagtttgcagtccaaatcagcttagttctgctcttccttcatggccagtttgttttcacctttctctggtttgctagggagttttacttgtccatctgctttcttgtttctaaatttgaatttctttatctcttctgctattctctttttacctgtgggtttatatcttaaaatcctttagtgccattttggtgaggtttcaggaggaatgagtcaagattaagttctatcttttatgttttactataagtcaactagtttaaattttattcttatgtaggcatactttttgtttctctctctctggatgatttcagagccactttaaccttaaacatatgtctttttcagcacagaaaatatttctaccaatgtatcattgagtatagtgtatgttgtgttttcttcaagcctctttctttaagagctagctctgggaataccttccctgtgaaccaaatctaacctcccctggcagagccaaactctccattctgtatctccatagcactttgtatgtgtgctaccaaagtgagtactctccagttttaccttggtatctgtgggggattggttccaggaaacctctcaaatacccaaatccatagatacccaagtaccttgcataaaatggtgcagtgtttgcatataacctatgtacatcctcctgtacactttaaatcatctctagattacttgtaatagctaatcctatgcaaatgctatatgaatcgttgttatacagtattacttagagaataatgacaggaaagaagtccatatatattcaatacagatgtaaccatccacttaaaaatatatttgtatttatattttttctgaccaacggattcttgccacatcaactatccacttttcccccagctgtggttggttgaatccatggatgcggaacccacaaatatggaaggctgactatagctagttacaattaatttgatttattaaagactcaccactttcaatgatggatcaataattatagataggagatactggaaagcagcatggatctgggtcccccatgtgagaggtgggagatgtggtggctaagtgactatggagtacagagttcctcaatagttggttacccacgttacactgagcatctatagcaagaagactataagcacatgcaattttagcaacagattagctactactataattttgaaatagagataaatgtaaatgttattttttagatatacattgcaactatagggtggtatgaaaatatttgtgatttctgttggtgactaagtcatagatgctgctaatattatggtggtttattaactttatttagaattaagaaaaatgtcaagttagagtttggtaaaaaatgtatcttttcctccctcccatgaccatgaatctctcaaattttactctgggaccccaggttaagcacattagccttagattctttattttagtttcacttatgatcttctgccatattagtcatggagtcttagacagtaatattggagacaatctcaattccaacattaccatagtactttagtttaattgttattgaatctagaaaaaggtgtttttgataaagatgttaaattctagatggtgaaatctgagaagagtggactatgccagaagccatggagtctggttgttttcacgtcctaaaaggtgactagctccatgaacaaactccccctgtttttcctcaggacttgagaaagattgagccatctttctttctacgttgaacctttccctgggtcatccacagggaagtatatgaatcagagacacatgctgtgatgtctggccctcagaggtatggttagcccagcagaactatcctgcaaggcatactctgaatatatggttttaatcaaagcaacttgcctagatttatttatttatttgtctctgttaatggagatagtgtgtgggggaaaaatctatatctgctgtaggcttagatccagtcagaaagctatagtgagtgctaatcttataatctgtgttttccatacatataaatttaaagtatggatatttgagctatatacagtagcaaccaacttaatggtaagtagctttatgatgttatatctaatgtttcttccaaatattatggcttcaaggccattcttataatttaagactgtaaaattgaacccatttttcaaaagttgaacgcatggtaccttattatgcatactgttgtctgaggtttggaaagataatgaagactctcatttcgtgtgggattctcaactgagaacaaggaatagaacttaacatttgagtttgaaagtccttgggttctgcttttgttatgcaataagtcccaatgataagcacaaaataggcactagaaaaagcctacttttaataggcatccattttaaatggggataaaaattttacggtatatagttaataaaaggtttcattacggcattagcaaataaagcaaaaatcattaaaacaagtttattttatttctctttataaaatttagcttgtaactatgcattgatttaaaacaaggaataaatcagatgttgactttggcatacattttctgacaaatggtatgacagtagaatatgacattcttctctttatgtttttgatttttcttgatgtgatcatgtagagtcagtttttgaaaaaaatttcattggcttcatagattttcctgagggcctcatttcatatttttatattcaaattatcctttttgaggtgtctatcttgtctttttcatattgcaagacttaaatttcactcttcagtctgtgtgctttgtgttgttaaatgttataaagattgactttccgtgagggtagatgtcagtgtattacatgagggatattgagaggaaaataatttcacaggtatttagttcatcagtgaacattttcaggttgtaacaattgcttccatatacattctcctaactgggagggttggggaggaattcatctcccaataattattcatgaaattattattatctcctctttatttatgaaaacatgagaagaaatatgaagttgtagtagcattaaaacataggcatattgagccgggcgcagtggctcacgcctgtaatcccaacagtttggaaggctaaggcgggtggatcacctggggtcaggagttccagaccagcctggccaacatagtgaaaccccatctctactaaaaatacaaaaaattagccaggcactgtggctggtgcctgtaatcccagctacttgggaggctgaggcaggagaattgcttgcacctgggaggtagaggttgcagtgagccgagatcatgccattgcactctagcctgggcaacaagaataaaactccatctcaaaaaaaaaaaaaaattaaaaaattaaaaaataattaaaaaaaggcatgtttgacaaaattctagaggagtttctaatagtgaaatatggaaagggccctgaggaggaatgtggggttgagctggtaagtggtatgacatttctacccattcttactatgccatctaccttggacacaggaagctttcactgagtaggagtaagagacaagagtctcttctgcgttctgcagtctgtcttctacatctgttctctgaaaccacccagagcattagcctttatcttcaactctaacacctctctctcaaatagttctttgtaagcccatatggggatgaaaatttgctataatacactacagcaggggcaatgaacaaccagtgatgttttagaatagagatgtaaaaacttaacataatgattatacaaaatggtgctgctattatgactaaaaacaatagtggctaacatttatggagcccatactacctagtaggcactcacttatgaactcatcaagtctttatgacaatgctatgagaaaggtactgttattatttccatcttattaatgaggaaactgatacatagaaacattcagcaacttgcccgagatcacatagccaataaatggaaggtcagaatttgggaacctaagtatctaactctaagatcctaccactttaaatgtcttctattgtatttgaggcagatcaatatttaatactgaacactaacttatgttcttatttgtttagaatctctgctttcaagaggagagttggccctgagatccatttcaaaggtaaatgatataatgtggtagaaaaaagcaggtgttcaaaaagtctaagctttagctgaagttagaagattgagaatatagataaaatgtttctgagaaacattgagaaataatatggcttttacttactttaccagaaaagaaaaagattccctggggctgagaggaatgaggttatatagaggagaattaatgaaaatggggagtctaggaggtcccagagagagggtccttgtctcttgcctccaggctgacagacaaggcatggtgccagactttagagaagcttgggtatgggtgggtgatatgacttgggcatcctgcccctggatgataatgccgtgtcagcctcaaagaaagtcatattctattattattattattattattattattattgagatggagtctcgttctgacacccaggcaggatttcagtggtgcgatctcaactcactgcaacttccgcctcccaggttcaagcaattctgcctcagcctcctgaatagctgggactacaggcacgtgccaccacacccagctaattttgtatttttagaggagatggggtttcacaatgttggccaggcttgtctcggactcctgacccacaagtgatctgccagcctcgacctcccaaaagagagtcatattctttagtgtgacatgaaaacaggagcaaaaagaatcctgttccactcttagtgtggtgctgaagaagcagaggaaatggagatcctgaaatgcccattcggacaggaataagaacaacttcttgctaagctgtgtgggctgatgatggaagaccaattgggattgtagatttctcagtgtatgtctgtgtagagaagtgattccaacactacatctgctctattccctcctccctgccaatatctcaatactttgtcagctccctggaacttagacacaactgcacacaagagaaaggtagctgagattcagatttataaaattctattgctctcttgacatagtttacttacccagatgtgcactctgagatctatggctactatgtttagtctcaagtttttcaggctgttctttaatcttcctagaaaattatgttgtacacaaattgtgaagttgatcaagcatctgcatgtatttacaaattctcccccacccaattttagttaattttcaaagtaggtaatatatgcacttggtacaaaaaaaattcaaaaggcggtcgggcgcggcagctcacgcctgtaatcccagcactttgggaggccgaggcgggcggatcacgaggtcaggagatcgagcccatcctggctaacacggggaaaccccatctctactaaaaacacaaaaaattagccgggcgtggtggtgagcgctggtagtcccagctactcgggaggctgaggcaggagaatggtgtgaatccaggaggcggagcttgccgtgagccaagaacgagccactgtactccaccctgggtgacagagcgagactccgtctcaaaaaaaaaaaaaaaaaaaaaattcaaaaggcgtcaacaaatagacaatgaaaataaatgttgcccctcagtcctaacacagctatcagttatttgtgtttcctgagatattatgtatacatattatcatatatatatacagtctaaaaacagacctgcaatgatagcatattttacactctgctctgtatcttgccttttccttgtaacaagatgtcttggatactattctatagttgtatttagcattccattctagggatgcaccatgatttatttaagcaatctctattgatgggaatttagattatttccagtttttttgctattacaagttgtgctatagtgaattgtttttagctccctctttgtgcatttgtttgaatatatgtgaatgataactttaaaagtagaatacagggatgatacttacatgtattgaaaatattaacaggtattgcccagtgactctccatagggactgtaccaagtgaaattctcacctgaaagtatgagtgcccatttcctcatattattaaactcttaaaatttgttctcatctgataaatgaaaatcagcatcttcttgtttttcctttcgttttaaaaaatgaatttgtatttttgtctgtactccttttttttcttatctgtctatgacctttgcccatttttctatattgattttcctgagcttacacattttatgaaattagccttttataatttgtattgcagatgctttcttccaatttattggctgtgctttgactttgcttgcttgtttctttaggtacttagactttttatttatatatagttgaattcatccatcttttaaaaaatggttttagtcaaaccattctcactcaagagattattgtcttatacctcatgctttctttagtatcttttcctaattttatttttatgttgaaatctttctcaatggagaatttgtttaaagggaaaagcagactattaattgctacatccatgatgttccatttataacttttactttaattttttgatgaatcatgggcaatggaataagattccattttttaccttcaaaataatatgtttgaatcacttatttaatttacttgcaaaaataagttctgcaagaaaagagtcttcattagatttttttcccactccaagaaaagccatatagtctggttgagttaattgtaacaagattagggtgggaagaaggtcagagagtgtgtttagctattgtaaactttgtgagcaaatgcaaactatggcgaatacagtttacagttttatggaaacaaagacaattctctagggccaatgttctaaaaaatgtagtttcctataacaaaaatttatattctcaacattacaagtcaacaattcttgaaattattaaaacaaacctttgaatattataagaaaactgtcttattctgtaaacttaggcagaaattcaatgttaagataacatgatacagaataagtatagatttaatttaaattttatggtaactggtatataaatattctctgaacttcttcaatatttagctaaaacaaagggcaatatctagtccaatgctttgtgttttaaaagcacttgtgtcaacaactcaaagtttctcattaaataacattgaaacatattgctatcattataactattattttaaccaaagcttagtcaaagaccttggccacagaatgatacactttaacagataatgaacctaagctatatgacattgcaaaacatggcactttgaatttaaatttaacaaatttgatgaaaactctcattattgatagagtactttctgttgccacacttactaattttgattactgccaaactttttaaaaattaattttaattacgcaacaaaacatggatacgttcacatttgaaaaagacaagagaagataaacctaaagatccctttgtttctactctcttgcctgattttctcttcaccaaaacctcaacctcagactgaagtttggggcttatacttccagagattgtttcacttcttcactcaacactatatttttcatatctatttgtattgagacatttagatcttgttcatttgttttaactgttgcacagaattttattaaatacatatacacataatcacattcctctgttgatggacatgtagtttgcttttggtttttcattattataaataacaatgcttataactgtctaccagtgcagactttttcctaaagaaagagtcctggaattgaaattattggtttataggatatgagcattttgagttttaatagatactgtcaaactattcttcaaaatggctgtacttatttattcttccatcagcagtatataataatggtgatttctctacatcttttcaacacttaattttgtcaaacttctaaaattagtgctaatttggtgaatgtgaacaagtatctcattatttaatttgcattttcttgattactactgagttgattatctcttcatatgtatactggccactcaagtttctttccctgtgaattatcctttgcccagttttcttttgggctgcttttcaatttcttgtaggcctgtacgagttctttattttgtcccaaatattaatcctttttatattatttgtgttacagttattttatccaagcctagtgattatttttaaactctatttcttgtgtcttaagtagagcaggatattgcatagtggttaagagtatgggctttaaaagcaaatgacttgggtttgaatccccactctgaaactatttgtgtgatctttggtaagttacctaacctctcttattctcaagtttctcacctgtaaacttaagattataatagaaatcacctcacagggttgatgtgaatgttaaatggcttaaataatgaatagtctctggcatataataagtactcaataattattattactatatagtcaaatttaacaataatttgtttataataattgttaaataattgttagataaaaagccttgtttgagaatgcttttcctaatgtgaagtttaaaaatgttttatattttgtattagtaattttattgattttatgtttattttaaaaatttgtctagatattttccatgtggcataggtaggaatgttaattttaatttttttcatctgtatatgaagctaattataccagttccatttacgtaaaggcctattatttcctgattgatttaaagtgtaacttctataatatattaaattcccataagatcactttcatattatcttcttttttagtgatttgtctattattgtgtcattgttacatttttaaaatttaattattgaagatttataatattccctgaattttttttgcatgcttctaaatttcagttgtgcttttaatatttgatggtcacttaagttggatacaaaatcattgactcatttttttcttggccttgagtaagaaatatatctctccattgtcttccatatctaaaagagttatgcctaaatgataactttccttcttgtatgtaatttacttttttggcttaaataacaagaaaatattttttaaggtacaatagttttattacattttggtggtaatcattctgggaaaattttcctatgtacatggtattccctttaatatgtaaagtattttgttattttaacaaagttttctttaatgacatatttaaaattttgttttctggcactgatttgcttttttcctttgagaatcttatacatacatgctgtgtatatatatccttttgttttttcatttctacttgattttttctaaaatttctgctttccattctctattgtctaagtgtcatctgtatactgctgtgtttcttctagtatagtcctctcttctgcaatttacgaagtgtgttttgatgacaaactccaaatttatagttgtatgttaaatctttattatactctcatttttaatatttatatttttaggtatagaattctattttagcagttagtaccattgacacaaagatattcctttgtcttctagttttcattgttgttattgagaagtcagctgtcttttctaactgttgtttctctcaaggtaattattttaaaatataggttttattataattcaggtatattgaggccatcagatcaggagactactgccattaaaaagatagtttgttcttcacagctctcaacaggaggggacatgcatgctatgtaatatcacatggagaaacaccaggttggtcaggaagcagaaagaatggaaacaaaacatggtcaaaaggcattattgtggcttctgtataaaggaatgtgtattagtcaaggttcttcagagaaacagaatgaataatgtgataggtagagagattgatagctagatagatttatcataagaaattggctctggtaattatagagactgagaagtttcaagatctgaagtcaagaagctggagatccaggagagctgatttcagtccagtagttccagtccaagtctgaaagcctatgagaagatctgatggtgtaagttccagttcaaaagttgtcagactgggaagccaagaagagccaatttttcatttcaagggtaagagaaagaaaagaccaatgtcccagttcaagaattcaggcaggaggagtttcctcttactcagccttttcattctaatcaggtcttccactatttggatgaggcccacccacattagagaaggcagtctgctttactcagcctacctatttaaatgttaatctcatccagaaacactttcctatacacatccagagtaatgtctggccaaatgtctgggcaccctgtagcccagtcaagttgacatgtaaaatgaactataaaagaataggtgaggcagggcgaatggtttcaggattggctagtttgaataatttcagcaggctctgggctgtaggagatgtcttgagttgtctgatatttgatcctgggttgattgaggcagttgaatattggcctaaagagtaagagccacatagaggagataggggattgtgccctggattggttagattgcatgtgaaagttgtgagttgtttgctatctttaggaattatgtaaccctggcaggggcagtcctttcctggtcagtgaggcctcagatgccagaacatcaagaataaagaaaataaagtataattaatacagtaatctattcttctctctggttgcttttaagactttgtctttatttttctatacttttgactctgaaatatctaatttgggtacattttaatttatctggcttgtgattcttccagcttttcgaatatgtgggttggtatcttccatcatttgtagaaaactaccagtcatttatctcttcaaatattgtgttacacatctcttcccttcttctccaagcaaagcaatctttgcatgtctttgtcttctattgtctcttgtttttcatattttctgtattggtctttctttctatgctacagtgagttttttaatggcctattttctagctcagcaattttatcttttgttttgttcagtatgttgctaaacacatccaattcagtttttaaaattagatattgtatttttatttcttaaggctcttatttgttctttttcgtatcttgtaggtcatatttctacttccctttgggtattttcaatcttgacttatttcttcaaacattacaagcctattcactttataatctgtgtctgactattccaatatctgacatctttgtgactctcttttcactggccgttcatgtttctggtctcccttatggtatcatttttccttgtgggcttggttatttttgactatgtaccaccacgtttccttaaaaattatttatggggattccctaggccttaaagttcctcctctagttagaatttgtatttactcctgttggatccctaggcgcataaccatcccagaattactttaaactaaatttacagcttgaggattcctggaccactccactaatgtgagacagggctgaaaatccatgcaagagttcacttgtggttaccagttttaagggacaactttttaaagattcgatttcccccttctctgctcagcatgaaatctcacccttagaaagttccctacatgtggattgtgattaggaaagtgcatttacttagttcagagttttagtttaatgtgcttgtctcctatttggattctcatggatctggaccttgacttatataccccatgccccttgaggccctctaaacttcagctcaattttatctaggtcagaaaatttcctcaggggaaaaagaaagcagcttaatgaggtgttcatttttctgaatatttgctctcttctagagtttggcttggtatctcatcctcacaatctttcgaaattttttattcttttttttttttctttttttttttgagacagggtctcactctgtcaccctagctggggtgcagtggtgggatcttggctcactgcaatcttttcctcccaggttcaagtgatccttccacctcaccctcctgaatggctgtgagtacaggcactcaccaccacttctggctttatttttatttttggtaacaacggggtttcaccatgttgcccaggctggtctcaaattcctgagctcaagcaatctgcccaccttggcctcccaaaatgctgggattacaggtgagccatcgctcctagccttctttgattcttttaagaaaatgagtttagcaattagaattgttatgaatagactaattcgttactggaaatgctgttactggaattggaagttgtaggaaatcttttacatttacctgaatgcttatagaattgcttcagtttccttgaaatttaaaaatagcaccaggatattttaaggtgatgactttttaaaattaattttgcctagttcataagaagcctttttgatttactgatttcatgagttttcccacagataaataagatagttattttattatatctttatcacctgtgttccatttcttctgatcatttctttagaaacaaagtctttttatatctatcattttcctcctttggattcatttacttcatattgttggataatttctcaagcatttctaaccttacaagtgattttttttgtctacagtggtgttgctattttaatttctacttgtagtaatgtagaagatatttatatgacattatttccttcattatagctttaaaatttttctagttctcttttgtctcagtatttcattgtttttgattcaggtttctttctgtacttccagaatccataatttttgtaattttattgaatattaattcatgatatagtattttatgaaaataattgtatttattttcataaatacactcatatctttccttgttttcagaattgttatcaagcaaatgggttcactacctgatgtacacagaaaccaataactatagcactagcttttgagaaaagaaagactttattgcaaaatgagtcaacaaggagtcaggagtgagctcaaatctgtttcctcaatctggggtctggagcaagtgtatgggcttggagagcaagagaaaagatttaggaatgtagatttgtagaatctgattgcaggggttcaaatttgaccagttatggtaaggtatattgaagtgaattttagctctagatcttctgggtcaacagaccccttgcttcagaaagagttctggtattatggttccagtcatgttccagtcttgttggctttgaggagagaaatcatttgttttgggtattgttagaggtcaaagcttttcctgttgtgcatgcctgggcttcatgacttgcagtttttggctctgttactacaaggtaactcaacattttgttattaacaacatgggcccagtttgggctggtcccagagttacaggatctttatattggtccattgtgattttatttatttttcaaattttttataatcacttttaaagtcttagataataaataaaatttaaatgatagattccactgaaaataattagccaaaacataaagcaggtaaattgcaccattcaaacacataattctttttaaacctaaaaataaggaagaaatacttaaatcttagttctttatttgtacatagaactttttaacactatatataaatgtgagaaatcattttggccaaaaaagaagtcagaagtcaaaattcataaaacaaaccttaggaatgtggaggttaagatattttctgccctaccaattaattattatttattaaaagaagtagagagatctgtatacatgaacaaaattgagacaacatgcaggtatatctgttgacaccacttaaaaaaacccacatttattttgaaaggacttgtgaacatccagtcaatagaaaaatacattcagaaaacacttactgaacatttatgatgtgtcagacactgtgttagaaacttgggaggcaaagcttctacgtctaagaagctcagagtcaagttgggggcaggtaagcacaaactttaaatatttacagtattctctctctctctctttctctctctctctttctcctccccaacctgttttatctaaacatgagttatacatgatatgtacaagcttatacattcagttatgtgtcccttaacagggatatgttcagagaaatgcatcattaggccatttcatcattgcgtgaacatcacagagtgtaccatatgtacataaacccagatggtgtagtgtggtgtggtgtacataaacctactccacacttaggctatatggtatagcctattgctcctaggctacatacctgtgcagcatgttactgtactgaatactttaggtgtctgtaacacaatggtatttgggtatctacacatatctaaacatagaagaagtgcagtaaaaatatggtataaaagattcaaaaatggtgcacctgtatagggtacttacaataaatggaacttgcaggactcaaagtttctctgggtgagtcagtaagtgagtagtgagtgaatgtgaaggcctgggacattactgtacactactgtagacattataaacactgtgcacttaggctacactaaatttattaaaaatacttttctttattcagtaagttaaccatagcttactattaaatttttactttacaagctttaaaattttttaactttttgattcttttgtaataacatttagcataaaacataacatatacacattgtacagctatacaaaaatattttctttctttatatctttatttcataagcttttttctatttttaattttttactttttaaagtttttggtaaaaactatggtacaaacacacacattagtttaggccttgtattagtcaggttctgtagagggacagaactaataggagagagatatataaagggaattttattaagtattaactcacatgatcacaaggttctacaataggtcacaaggtttcacaatacgccgtctgcaggctgaggagcaagaagagccagtctgagtcccaaaactgaagaacttgggagtccaatgttcaagggcaggaagcatccagcacgggagagagatacaggctgggaggctaggccagtctagtcttttcacgttattctgcctgctttatattcagtggtagctgattagatggtgtccacccagattatgagtgggtttgccttccccagcccactgacttaaatgttaatctcctttgacaacaccctcacagacacactcaggatcaatactttgcatccttcaacccaatcaagttgacactcagtattaaccatcacagacctatacaagataaggatcatcaatattgctgtcttccacctccacatcttgtcccgttggaaggccttcaggggtattagcagctctgttataatcttatgggaccactaatgtatatgcagtttgtcattgaccaaaatgtcattatgtggcacatgactgtacttatatatatcacttatttgtgtataccatatgtctttgaatgtatatatggaagttggtcatgaaggtaacgtttgtgtgaaatatttgcccttttagtttcctgtggaacctggaaggatcaggattcctgaaaatttaaaccagaactcagatattccagtaattgctcatcaagtgcccactagtagctaagcatctgctacacaacagcatacaaagtctggaaggtaatgaaaatagtgcaaatgggttccccatttcttttccaagaaaaacctcctaatgggttgctgatgagctaatcaggtcaagtgttctctgagttgccctctttctacagtcagcaagcataacattttgttaacctattgacacagaggaaatttgttttccatctgaccttttacagtaactactcaaaattactttctcttcagctaacaaagctaatgaataaattattcaagtttgacactcatagaaaataacattttacatttttcatttttattcctgattattttgctttctttttcagccattacttctttccctatgaagagttttaatctttacggaaattttgcagtgttggtttagagagtcatactcggactctctggaactaatcacattcacaaaataagtttcttattttgcaaatataacatttatatatgttgaaatggtcacatgataattttgtaaatgcagataaattccattaagaatttataaccatttgtataagaataaaattttaactttgggctacatgtaaacaaaaggtttcctaaggaaatagttattagaacaaaaatatttgggacattttaaacctgagaataaactcttctccaagatggaaaagtgaattataggtctttgttattattctttatgaaatcttaattctaagcatctctactcactaacattttgttaaatttattcctttaataaaaatttcttcaaaattatcttaatgtccagccttttatctgtctcaaactgtcctttcactaaacaggtccaaattggatgtttacttgcagtgaatatgtttttaatggtttgttatattcagaggatcataacttcaaagatggtcatcaattaattcacaaaggtaagcttttcttcactctttgtggttaggccaatttaaataatacatgttagagaatgagcatctacatatttcctctgcagactgactattctaacattcactatgctaagagtattgttatttgagcatcactaaatgcattcaccttcccaattttcagagacaaagtcaaactcactcatatttatcatgaatgtgcatacaattctattaatttaacattttccatcaatgtaataaaatagcaatattattttatacttgttagaaagattctaccaagagtatttttgatcatcatcagcaagtggtcactgtttcttttggaagatgctcctggtcactaaaaactgtatcactttaaccacaacctcgttaaactgggttcagagactcacaaattatatcaacagtagcatttctttcagttgaatttgcaaagtaggcttttattctctatgtgttccaatatctaccttgaacagtcttagaactagttaaagcatttattaagtactcttgtaatgaaggaagtaatgattaattgataactacttttgttatgcttataaaacattttccctaaactttaccttaattttgggggattgtgagggaagtctcctttactttaattacttatcgacccaggtatcagacagtcataatatcttttttttttaagcaggtaaaactagactttgtatgggaattcttaagaaatgtcagagagctggtcctgttgaaaagtttagcagttatagaaaaatatttcaaaacataaatgtagcagtttaaacatgatttggtgtccagaataacttgttggtcttatttttcattttcaacataaatatcaactgccactgtataattgaatcacaaacatatttgaattcaggaatttttatactgaaatatttctctgtgagcaaatcccacctcaccaaacagaaagattttgttactgtttgtgtgttctaaaatcgagaaagccttatattatataattctctgttgggtattttatgtatctgtatacttttttattccacttcccctgtcatttttgtattcctcaaaatatctaggacagcatttttgcatgctcgtgtacatttaagaatatagcatagtggttaaaaacttggcttctgcaaccagactgcttaggttcaaatcttggctccataaccttcagtgctatgacctttgtaattcactcaaacctcctatgccttggatttctcatctataaaccagaaggtggattaactgtcggtggattaaatgagtcagcacatgtagaacacttcaagtagtagctggtacatatcaggctcttagtaaacattagctattattatttttaacaagtattaagcacctgttacactgaaactgtgctgtgggtgctggggatgccacgatgaacaagtactcatctttacttctatcataaaatgtaaagtttggtgaaatattcaggcaaacacatgggtcattgtaatacagtatgataactgctatcatagggtagtgtagggtgccacaattgcctaatggaggaccccttaccagactaagggtatcaggaaagtttttctggtctaagcagtgtctaagctgagatctgaagaatggtgatatagcttgtaccctccaaatctcatgttgaaatttgatccccagtgttgaaagtggggtccagtgggaggtgtttgggttatggaggtggatccctcatgaatggctttgtcattcttgtgagactgagtgagttcacactcttattcccgtgagatctggttgttaaaaagagtgccaccttcctcccaccccgtctcttccttctgctcttgctgtgtgatgcctcctccctttgccttctgccatgagtggaagcttcctgatgtccttcccagacatagctgctcttgccatgcttcttgtacagcctgcagaaccatgaaccaaataaacctcttttatttataaattacctagtctcaggtgttcctttatagcaatgcaaacagattagacagatgggtaggggcttgccatgtgatagtgaatggtgtggaggaatgcagtttcaagaagacagggtagccagaggatccatgatacaggggaaagagagtatgacacatttaaggacttaacaaggctcagttaaatgcactatatagttcatgacaggggatggtgcacaaacctctctattctgagaagaataggcaatcactgaaggtgtagaagagaagggtgtcatgttcatattttagttttcagatctctccaactccagtgtaggtaatatactaaagtgagtttaaaagttgatataggaagatcagttaaaatgccagtgcaccatccaagagaaagatgttggaggcttggaactagagtggtaggggtgaatagaaaaagaacttgagaaatctaagagacgtttatgggaaaagagtcagaaggacttggtaataatacagtgctagatatggagtgagagtgagaaagaagacctaaagatggattcccaggtttctagattgagcatgtgattgatgccatctactgagacaggaaacattgtctgtaatgaatggacagtggttgtggctagtcagtatatatccttggtaattatgtctcaattgtcaactaggagcaactcctgctcaatctcaattcatgtgctcttagatggagttgattccacctccagctccaagggtggagcacatgaaccagattggaccaattagtgcatcacattctcccagccacatgtcagggttggtcacagcaactaagctgacacagttagagtgagtctgatagctttggtgggacttgttgaaaaaggcatgggagtgtgaattgttggagctgaagcagttatcttgaacccactagaggaatgtctgcgagaaaggagccaacgcagtggaaagcagagctgagagagagaagaaaattctgagaatgccctttaagtactgaatctagctatgcctatgtcatcctctcccttgcgctttttcttttctttttttaaatttaatttaattttaagttccaatatacatgtgcaggacgtgcaggtttgttacacaggtaaatgtgcgccatgatgatttgctgcacctaccaagccatcacctaggtattaagccccgcatgcattagctgtttatcctgatactctccctctcccgatcccccaccccgacaggccccagtgtgtgttgttcccctccctgtgtccatgtgttctcattgttctgctctcacttataagtgagaacacgcggtgtttggttttctgttcctgtgttagtttgctgaggataattgcatgtctaattttttaagaaactaccacattctttcccaaagtagtggaaccatttagctctcccactggtagtctgtgagagttccagtttcagaagaaatggtaccaactcctctttgtacctctggtagaattcagctgtaaatccgtctggctctgggtatttttttggttagtaggctatttattattgcctcagtttcagaacttgttattggtctattcagggattcaacttcttcctggttcagtcttgggagggtgtttgtgtccaggaatttatcaatttcttctagattttctagtttatttgcatataggtgtttatagtattcgctgatggttgttcgtatttctgtggggtcagtggtggtatccctcttatcattttttattgtgtctgtttaattcttctatcttttcttctttattagtctagctagcagtctatcttattaatttttttcaaaaaaaccagctcttggatccattgaattttttgaagggtttttcatgtttctctccccttctgtaccaccctgatcttggttatttattttattctgctagctttggggtttgtttgctcttggttctctagttcttttgcttgtgatgttagtgtcaatttgagatctttgtagtttttttaatgtgggcatttagtgctctaaatttccctcttaatactcctttagctgaatcccagagattctggtacagtgtctctttgttctcattggtttcaaataacttcttgatttctgccttaatttcattatttacccaggagtcattcaggaacaagttgttcaatttccatgtagttgggtggttttcagtgagtttcttaatcttgagatctaatttgattctgctgtagtctgagagactgtttattattatgtcagttcttttgcatttgttgaggagtgttttacttccagttatgtgatcagttttagagtaagtgccatgtggcactaagaagaatgtatatttgttgtttttgggtggagatttctgtagatatctatcagttccatttgatccagagctgagttcaagtcctcaatatccttggtaattttctgtctcaataatctgtctaatattaacagtggggtattaaagtctcccactattattgtgtgggagtctaagtctctctgtaggtctctaagaacttgtgttatgaatctgggtgctcctgtattgggtgcatatatatttaggatagttaactcttcttgttgaatcgaaccctttaccattatgtaatgctctctttgtcctttttgatattttttggtttaaagtctgttttgtcagaaactaggattgcaacccctgcttttttctgctttccatttgcttggtaaattttcctccatctctttattttgagcctatgtgtgtctttgcacatgagatgggtcttttcaatacagcacactgatgggtcttgactctttatccagcttgctattctgtgtattttaattggggaatttaatccatttacatttaaggctaatattgttatgtataaatttgatcctgccatcattatgctagctgattattttgtaggcttgttgatatagttgcttcacagtgtcattggcctttgtacttcagtgtatttttgcagtggcaggtaccattttttcctttccacatttagtgcttcctttaggagctcttacaaggccagcctggtggtgacagactccatcagcatttgcctgtctgaaagagattttatttctccttcacttatgaagcttagtttgcccagatttgaaattctgggtaggaaattacttcctttaagaatgttgaatattgccccctatctcctctggcttatagggtttctgctgagagggccactgttagtctgatggggttctctttgtaggtgacctgacctttctctcttgctgcccttaacattttttccttcattttgaccttggagattctgatgattatgtgttttggggttgatcttctcatggagtatcttactggagttctctggatttcctgaatttgaatgttgacctgtcttgctaggttggggaagttctcctggatgagatcctgaagtatgttttccaacttggttccattctccctgtctctttcatgtaccccaatcagttgtaggtttggtcttcttacataaccccatagttctcggaggttttgtttgttccttttcattcttttttctccaaacttgtccgcctgtcttatttcagcaaaattgtcttcaagctttgaaattctttcctccacttggtccatttggctattgatacttgtggttgcattgtgaagttcttgtgttgtgttcttcagcttcatcaggtcatttatgttcctctctagactggttattctggataacagctcctgtaatgttttatcatggttctcagcttcttgcattgggttagaacacactgctttggatcagaaaagttcattattacccacctttttttttattattatactttaagttttagggtacatgtgcacaacatgcagttttgttacatatgtatacatgtgccatgttggtgtgctgcacccattaactcgtcatttaatattaggtatatctcctaatgctatccctccccgcttccccaaccccacaacaggccctggtgtgcgatgttccccttactgtgtccatgtgttctgattgttcagttcccacctatgagtgagaacatgtggtgtttagttttttggccttgcgatagtttgctgagaatgacggtttccagcttcatccatgtccctacaaaggacatgaactcatcatttttatggctgcatagtattccatggtgtatatgtgccacattttcttaatccagtctatcattgttggacatttgggttggttccaagtctttgctattgtgaatagtgtcgcaatagacatatgtgtgcgtgtgtctttatagcagtatgatttataatcctttgggtatatacccagtaatgggatggctgggtcaaatggtatttctagttctagatccctgaggaatcgccacactgatttccacaatggttgaactagtttacagtcccaccaacagtgtaaaagtgttcctatttctccacatcctctccagcaccttttgtttcctgactttttaatgattgccattctaactggtgtgagatggtatctcatcgtggttttgatttgcatttctctgatggccagtgatgatgagcattttctcttgtgtcttttggctgcataaatgtcttcttttgagtattacccaccgtttgaagcctttttctgtcaattcatccatctcagcctccgcccagttctgtgtccttgctggagaggtgttccaatcatttggaggagaagaggcactctggcttttttgagttttcagcatattttttcattgattctcatctttgtgagtttatccagcttgatctttgaggctgctgacctttgggtggggttttggtggggactgttttgttaatgctgttgttgttgttgctttctgtttttcttttgagagccaggcccctcttttgtagggctgctgcaatttgctggggatcctctccagaccctatttacctgggtccctcccacacctggaggtatcaccagtggaagctgcagaacagcaaagatggctgcctgctccttcctctaggagatcagtcccagaggggcaccaacatgatgccattgggaacacactcctgtataaggtgtctggagacccccgttggggggtctcacccagtcaggaggcatgggttcagggacccacttaataaagcactctggctgccccttggcagagggggtgcgctgtgctggggggaatcccagtcaccggactgcccagattcctcagagccggcgggggaaagactaagttggctgatctgtggagaccatggtttccccttccctcagggactctgacatggtttggctgtgtcttcacccaaatcttatcttgaattcccatgtgttgtgggatgaacccagtgggaggtaattgaatcatggggggcaagtctttccccgtgctgtgaataagtctttctcatgatagtgaataagtctcatgagatctgatggttttaaaaatgggagtttctctgaacaagctctctttctttgccttctgccatccatgtaaaatgtgacttgctcctccttgccttctgccatgactgtgaggcctccccaggcatgtggaaatgtaagtcccttaaacttttgtttgtaaattgctcagtcttgggtgtgtctttatcagcagtatgagaacagactaatacagtaaattgggaccagtagagtggggcactactgaaaagatacctgaaactgtggaagcgactttggaactatataacaggcagaggttggaacagtttggagggttcagaagaacacaagacaatgtgggaaagtttggaactccttagagatatgttgaatggctttgacaaaaatgctgataatgatatggacaatgagatctaggctgaggtggtctcagatggagataaggaacttgttgggactggagcaaagtgactcttgttatgttttagcaaagagactggcggcattttgtccctgccctagagatttgtggaactttgaactgagagagatgatttggggtatctggtggaagaaatttataagcagcaaagcattcaagaggtgacttgggtgtgttaaagtcattcagtttaataagggaagcagaacataacagttcagaaaatttgcagcctgacaatgtgattgaaaagaaaatcccatttcctaagaagaaattcaagctggctgcagaaatttgcataagtaacgaggagccaagtgttaatccccaagactgtggggaaaatacctccagggcatgtcagaggtcttcacagcagccccttgcatcataggcccagaggcctaggaggaacaagtgatttcatgggccgggccaagggttccaatgctgcgtgcagcctagagactggttgccctgtgttccagatgctccagccatggctgaaaggggccaatgtagagtttgggccatagctttagagggtgcaagccccaagccttggcagcttctatgtagtgttgagcctgtgagtgcacagatgtcaagaattagggtttgggaacctctgcctagatttcagaagttgtatgaaaatgcctggatgcccaggcagaagtttgctgcaggggtggggtcctcatggagaacctctgctagggcagtgtggaaggaaaacgtatggattggagcccccatacagagtccctgctgagacactgcctagtggagctgtgagaagagggccacaatcctccagaccccagaatggcagatccactgacagcttgcaccatgtgcctggaaaagctgcagaccctcaatgccagcccgtgaacgcagctgggagggaggctgtacccttcaaaaccacaggggtgaagccacccaagaccataggaacccacctcttgcatcagcgtgacctggatgtgagacatggagtcaaaggagatcattttggagctttacaatttgactgctccactgggttttggacttgcatggggcttgtagcccctttgttctggccaatttctcctatttggaatggccatattaacccaatgcctgtacccccattgtatctaggaagtaactaacttgtttttgattttacaggctcataggtggaaggcatttgccttgtctcagatgagactttggactgtggacttttaagttaatgctgaaatgagttaagactttgagggactgttgggaaggcatgattgtttttgaaatgggaggacatgtgatttgggagggtccaggggcagaatgatatggtttggttgtgtacccacccacatatcatcttgaattcccgtatgatctgggagggacccagtgggaggtaattgaatcatggagatgagtctttccccatgctgttctcatgacagtgaatacgtctcatgagatctgatggttttaaaaatgggaatttccctgaacaagctctctttctttgcctgttgccatccatgttaagacgtgagttggtcctccttgccttctgccatgattctgaagcctccccagccatgtggaactgtaagtccattaaacctctttcttttgtaaattgcccagtcttgggtatgtctttatcagcagcatgagaacagactaatacaggctccattccagggagattagagttctgtctgtaaaccgctggctggagttgctaaaattcctttagggaggccctgcccagtgaggagggatgggtcagggtccagcctaaagaggcagtctggccacaatctgccacagccactgtgctgtgctgtgctgtggggaattttccctaggttcgaacctcccagtcttcctgagtccagcaggggaaacaggcagactagagctgcagtgatggctgccgcctctcttgcctggagctccattgtcttagtcatcttaggcagcagacaattgcagtgatggtgtccacccttcccctcaggagttcagtagtcttaggcagtctctagcagagtggctgctgagaatctttacagctctctgcttgggacccaagagcctggtggcatgggctcacgagggggtctcttgatcagtgggttgaacggatctgtggaaaaagcatagtttcctgggcaggttagcacactcagtcaccgcttcccttggctgggggtgggagctctccttgccctgggtggctcccaggtggcccatcgtaccaccctgctttttcttgctctctttgggtcacaccaatcacctagtcagtcccagtgagagaacctggatacgtcagttgtcagtgcaggattcactcgctgttttcattcttctcagtgggagcctctgaccacagctgtttctagtcagtcatcttggccccaccccctgcaccttttcttttatgtgcactaataagttgttttttggcttaagccagataggtttttaaatatatacactttcaaaaatatataagacaccacatatgaaggaactagttgtggaggtagaggttgaattcagccttggctatgttgagcttgaggtgtttgtgagacatctttatagaaaagagatatccggtaggaaattagatatgtggatagaaagttaacaataccttatacagtctttggtaaaaatttttagagagtccttttgtaatgcatgcagaaaagatcttcacaaaatgctgacctctcctgtagaaccacctagacccaaaggatttgaaggaagcaattctttattttcagttttttcaaggattattagtctattcagagtttctactcctagatgcaacatttacaatgaatgtccatttcatttccaatttaccttctagttgtgatgaactgtgtaatggcccctcaaagatatctaattcctggaacctgtgaatgttaatttgtttgttaaaagggacttttcaaggtgcgattaaggtaaggattttgagatggggtgattatccttggttatccaggcaagcccagtgtaatcacaagggttctcataagagagaaggtgatgtgctgaccgaagcagagattggagtgatgcattttgcagatggagaaatgggccaaaagcaaagagtactggtggcctctagaaactggaaaagacaagggaacaaattctgtcctaaggcttccaggaagaacgtggccctgccagcacctttattttataccagtgaaactgatccagactcctctcctccaaaactgtaagaaattaattttgtggtgttttaatacaccaagatctctgaaacttttttacagcagccccactgaggctgttagggtgagccctagtccaatctgactagtatcctttcagggaactaacaccccactgtaatatgatatttatatatttctttctatgtatatatctcaaatttaacagctttcttgagtataattcacataccataaaatttatccaagtataaaattcaattattttttattatatacagaggtatgcataaccatatctgcagtcaattttagaacctttcaatcaccacaaaaagataacccatgtactttagctatcttctgcctgtccaccagtttccatatccctaagcagctactaatctactttctgtctctatagattttccagttttagacaattcatatagatggaatcatatataacacgaggcccttgtgatcagcttatttcacttagtgtaatgttttcaaagttcatccacattgtagcatttatcagtactttattcctgtttttggttttgagacagagtctggctctgtttcccaggctagagtgcagtggcacgatttcagctcactgcagcctccacctcctgggctcaagccatcctcctacctcagcctcctgagtaactgggactataggcgtgcaccactccatccagctaattgtttttgtagaaatggggtttccccatgttgcccaggatgatctgcaactccttggccttccgaagtgctgagattatttccttttatagatgaatattatcccactatatagacacaacacatttttatgtatccattaattagctgatggaaaagtttttatgtagacatatgatttcattcctcttgggtatatatcgataagtagaactactgggtcatatggtaaccctaagtttaactgtttgaagaactttcagattgttttccaaaggctacatcattttgcatccctaccagcagtatatgagcattccgattcctccatatcttctccaacattgttattatatgactttttgattctaggcatcctactgggtataaagtgatatctcattaaggttttgatatgcattcccattataatggttatgacctgaattatcttccccaaacttcctgggttcatatgttgaatcccttatctcctgtatttcagaatgtgactgtgtttggagatagggccttttaaataggtaattaagttaaaatgaggctgttagggtgagccctagcccaatctgactgatatccttataagaagagaagattaggacaaatagagagacaccagggatctatgtgcacaaaagaaagaccatgtgaagacagagcaagaagacaaacatatgcaagccaaagagaagggcctcagaagaaagaaaacctgctgacaccttgatcttgttcttctagattccagaactgtgaaaaaatttttttctgccacctgctctatggtattttgttatggcagccccaggaaactcatgactaatgatgtcaagcatttttttcttgtgtttattggccatttgtatattttctgtggataaatgttttctgagattgctcattttaaaattgtcttcttattgttgaattgttgagttgtaagagttcttatatattctgcatactatgcccttagcagacatatgatttgcaaatatttcctctaattctgtgggttttcttttaccttgttgatagttcctttgatgcacaaaagtttttaattttaattaaagccaacttatctaatttttcatttcttgctcatgcttttggtgtcatatccatttcaaaatccaaggcatgaagatatttcctttatattttcttctgagagttttatagttttagctgttacgtgtatattcttaatccatcttggattaattattacctatggtgtgaggtaagggcccatttttttttttttttttggcatgtggctatgtagttgttttagcaatgatttgttgaaagagctattctttcactattgaattgtcttgacacctttgtaaaaaataagttgactaaagacacatggttttattctggactcccagttctttttatttattttattttatccacagggtgtatatgtgcttgtttgttacatcggtatattgtgtactggtggggactgggcttctagtttacccattacccaaatggtgaacactgtacctgatagatagttttttatcccttgctcccctccacaacctcctctcatttggagtctctagtgtctattatttccatctttaggtccatgtgtatccattgtttagctccctattgtaagtgagaacatgtggtatttgattttctgtttctgagttagttcacttagtataatggcctccagctccatccatgttgctgcaaaggacataatttcattctttatggctacgtagtatcccatcgtgtatgtatgccacattttctttatctggtcaactgttgatggacacttaggttgcttccatgacttggctattgtgaataatgctgcaatgaacatacaaatacggatgcctttttgatatgattgtttccttttctttgggtggatagccagtagtgggattgctgggtccagtggtagttctatttttagttatttgagaaatctccatactgttttccatggaggttgaactagttcaaattctcaccaataatgtacaaatgttcccttttctccacatccatgccatttattgttttttcaccttttaatagtagccattctgactggtataagatgatattctgattttaatttgcaattctctgatgattgctgatgttaagcactttttcatgtgtttgttggctgcttgtattttttcttttgagaaatgtctattcatattcttctcccaagttttaatggggttgttattttcttgttgagttatttatattccttatagattctggatattagtcctttgtcagaggcataatttgcaaatattttctctcatttggtgggtggtctgtttactctgttgattatttcttttgctttttagtttaattaagtccaatttgtctattttcattcctgttacatttgcctttgggatcttcatcataaaattatttgcctatgccaatgtccagaatagttttttctatgttttcttctaggatttttatagtttcaggtcttacatttaaatctttaatccatcttgggttaattgttgtatatggtgagagatagaggtccagtttcattcttctgcatatggctagccaattttcccagcactatttattgaatagggtgtcctttcaccattgtttatctttgttgactttgtcaaaaatcagttgattgttagtttgtggctttatatccaggttttctattccgttccattgatatttgtgccatttttgtactagtatcatgctgttttagtcaatgtagccttgtattataatttgaagtcaggcaatgtgatgcctccagatttgttcattttgcttaggatttctttggctattcaggctcttttttgattccatgtgaactttagaatttttttctaattctgtggaatatgacattggtaatttgataggagttgaatgtgtagattaatttaagcagtatggtaattttaacaatactgattcttccaatccatgagtgtgggatgtttccccatttgtgttatctatgatttatttcaacagtattttgtagttttccttgtagagatctttcaccttcttgattaaattaattgctaggtattttgtgtgtgtgtgtgtggctattgccaatgagattgagttcttgatttggcgctcagcttaaatgttattggtgtatagaaatgctgtcgatttatgtatgtttattttgtatattgaaatttgtttatcaagtctaggggtttttggaggagtctttagggttttctaggtatatggtcatgtgatcagtgggcagagataatttgacttcctcttttccaatttggatgctttttttcttttacctgattgctctgagtagtgctcctagtactatgtgcaataggaatgctgagattggatatgcttgtcttgttccagttcttaaaggtaatgcaatcaacttttttccatttagtataatgttgactgtgggtttgttgtaggtgggtcttatatttttaggtacttttttatttttatttttattttttttagaggaataaaatagtggctactccataggcagagcagccaggtatggtcttttgatgcctagtttgttgagggtttttattatgaagggactttggattttattgaatgccttttttcatgtattgagataatcatatggtttttctttttagttttgtatgtgtgatgaatcacccttttcaatttgcagatgttaaaccgtacttgcatcccagaaataaaacccacttgatcataattaattatttttctgatgtgctgttggattcagtttgctggttttttcttgagaatttttgcctctatactcatcagagatattagtctgtagtttgcttttctgtgtgcgtgtactggcctgattttggtgtcatgatgatactggtttcattgaatgagtcacagaggaatccctcctccttgagtttttggaatattttcagtaagattggtagcagctcttctctgtgtatctggtgaaatttggctatgaatctctccggtcctgggcttttatttgttgaaagatttttttattactcactcaatttcattacttattattggtctgttcaggatctctatttattcctggttcaatcttggagggttgtaggtttccaggaatttatcaatttcctctaggttttctagtttgtgtgcatagaggtgtttatagtagtctctgaggatcttttgtatttctgtggcatcatttttaatgtcccttttctcatttctgattataattatttgaatctctctttcttggttaatctagctagcaatctatcaattttgtttatccttttaaaaaactaactttttgtcgcattgattcattatgtctttaaaaataatctcaatctcatttagttctgctttgatctttgttatttcttttctgctactagttttgggtttggattattattatttttctagttccttgaggttcaatgttaggttgttaatttgagatttttctatctttttttataagggcatttaatgctacagaatttcctcttagcactgcttttgctgtatactagagattttagtatgttgtgtctctatttttatttgtttcaagaagtctttcaatttctgccttaatttattatttacccaaaggtcatttgggagcaagtagttttgctttcatgtacttgtgtagttttgagagttcctcttggtattgatttataattttattctactgtgatctgagaagatacttgttattattttgattttctgagtttattgatacttgctttatgggcaaatatatagtcaattttggaatatattccatgtggaggtgagaagaatgtatattctgttagataaaatgttctgtgaatctctattagattcatttggtctacatcccagttgaagtccagagtttctttgttgattttctgccttgatgatctgtctagtgatgtcagtggggtgctgaagtcccccactcttattatattgctatcaatatgttttcttaggtctagtagtatttattttatgaatctgggtgctccagtgttgggtgcagatatatttaggatagttaaatcttcctgttgtattgacttctttatcattttataatgaccttttttgcccccttttttttttaactgttgttggtttaaagtctgttttatttgattgaggatgactactctctcttgcttttgttttccatttgcgtgatatatctttttcaacccatttactttgattctatagctgtctttagccagtatgtatgtctcttgtaggcagtacatgtttgggttttccttttttatacagtttgccactctgtatcttttaagtggagcatttaggccacatacattcaaggttaatattgatatgtgaggttttgtttctatcatgttgttgttagctgattgccttgggatttcaattgtgtaattgctttataaggtctgtgagctttttacttatgtgatcttttatgatggtgaatgttgttgtttaatttccatgtttagaactcctttgaggttgggcagtggctcatgcctgtcattccagcactttgggaagctaagtgggaggattgcttgaggccaagagttttagaccagcctggtcaacatagtgagacaccatctctactaaaacaacaacaacaaaaacaaaactccttcgagcatttcttggaggaccagtctagtgttgatgaattccctatttctccttgatttatgaagcttaatctgacaggatataaaattattgggtggcatttttttttctttaaagatgctaaaaatagacccccaatctcttctggattgtaagttttctgctgagaagacagctactagtccgatatgattatatatatataaatgcaattagacacttctctcttgccattcaggattattttgtttacattgactttggatagtcttggtgaagttcttgcaatgtattatccagaaattctctgagcttcttgtatctggatgtcaaaatctctcctaaaaccagggaagttttcttgaagtatttctgcaaataggtttttcacactttttgctttttcttcttctccctctggaatacctataacttacaggtttgtacacttttatatttcacaaaggctttgttcattaaaaaaaattttttaaatattatgtctgactgagttaatttgaaagacctgtcttccagctctgaaattctttcttccacttggcctattgttaacactttcaatgtattttgtaactccttgactgaatcttttatttctagaagttttgtgtgtgtgtatttttttaaatgacatttatctcttctttcatgtcctaaattgcttttctatttgtatgggttttctgctttttcttggatctcactgagcttctttaaaatcagtattttgaattatttatctgatatttcaaagacttcattttggttaggatttgttctgaggagttagtattcccctttgggggtgttgttacattctgttttttccatactttcagagttgtttccctggttgtttcttatctggataagctgtctctccttcttattttttaattttgcttccctttggacaggattattttgcccccttgaggaggtgtctgtactgtatgatgtggtgtagtgtcctttgggtttggttctgggtattttcagtggcaaagagtctgtataaattctttggtaatagcctttgtatggtgactttctcaaatgctggttgttgtagtgatgtgctaagcatgtgagcagcctcactcactgcctcctgtgggctcagggtgatggaagtctcaggaagcttatttcattctccagtactctgcacttgagtcagcagatttcctgttgtgttgcaccattcaacttccaggccagtaggtggtgcttatgtctgtttttatctcctacacccttgtggttcttatgcttagtgttctacccatgagtgaaaattgggtattgaagtacccaattattgatgaattgtctatttctctcttcatttaaatcaatttatgcttcatatgtattggtgctctgttgttaggtgcatatatatttttgattgatgtatctttctggttaattgaccttttaaaaaacatcttcttttatctatagtaatatcttttgttttaaggtatattttgtcaggtaattgtataaccattccaactttcttgtggttgctgtttgcatgatatttctctttcatctttttactttaagtctatttgtattttgaatctaaagtgtgtttcccatagatagcatgtattgactcttgttttttgatctagtctgagaatctctgccttttgactggattatttagtccattcacctttaatgctattattgatatagttggaattatgtttgccatttttgttttttatatatctcatgtttctcttgttcctctgtttctgctttactgctttcttttgcatgaagtgaatattttataatgtagcattttaattttttaaattattttttcactatatttttgagttattagtggttactctagggtttttctatatacactgtgacttataataatcagtttgagatttatactaaattaattctagtgagatacagaaatgttacttctatatacctttgttcccttccccccatttttgtgatactattcttattcatattacatctattacatctaatatctgaatattacaaacccaacaatgcattgttgtaatgataaatttacacgcttttatgttttttaaggatattgaggagagcaaatacagacacacacaaacacacacacacatttatagcttttgttgtgttagccttttaatttatcatttctggttctcttcatttgttcctgtgcatacaagttgccatctgaagtcatttccttaatccaatacagctttgcccccacccacctcttttgttctattattgaccaatattacatttttatgttataggctcaacatcacattatatacttctttatacaattacttttaaaatcttttagaagaagaaaggaaaagaaatgccttgacttttacaattagataattacctttcctggttctttttgcttttttcatatatatattccaattactctcagggttcacttgtttgtagcatgaatttcttttagtacttcttataaggtaggtctgctagcaacacattccctctgtttttattaggacatgtcattattttaccttattttggtggatatagaattcttggttaataattgctttttttggttcattctgaatatgttgtccttctggcctcaattaattctgctgagacatcagctgttaatcttcctggagtttcagtctaagtgatgagtcatttttatcttgatgtagtcaaaattttcttattgtctttagctttagctttttcacttttaggtgtcttttgatgtgacattgtaatcatactttttaaatcatggcccattttatttgaaaatattatttgaaattatttataatctctactttgaaaactttttctgttcaatctgacatctgatgtctgttaaatctgacatctggtaagtcttccaggcagtttctgttgtctacaattttttttcagtgtattgcttattctttcctgcttctttatatgtctcataattttttgttgaaaaattttaggtagtatattgtaataatactgggtactggtcttctggggcttgttgttatttgcttatttacttgtttgttgattgactagattattttggtgtaatttatttcttcctctgaagcataaagtctataaagttgtttctcaggggatgcagtttgatatgctcacagtcagctggcaacacagtggatttgggagagctctcttttgtctttttctctggtcatacccaggtattatgctccactacttacttgctggctgatggctctgttgctttcaacaatgccctggaatatagattgttttacaaactgacccaaaaatttgggctcttcttaaaaaattgttcctgaggtcagtttttgagatttgttttgaccctaagagggttcctcccagatgtcttgctttctatttctctatagcaaatcatccagcttacaacttaggctatatctctaacaaatctatcaattttttcccaattgcttttcacaaactttcactgtttttgagagtgactttaggcttgaaattgtccatggtttgttggaaatgaagtcaatttctttggggagagattttaagtattctgttatacagcgtgcttctctacgtttgggcaaaatctctgagccacagctctggtcctggaacagggacaatgacagacttccctctaaatgatatacccactttaagtgctagtaacttttggtgtgtgtgtgaagtggtcccagttcaactcggcttgactctgctagtatggcactgatatggtttggctgtgtccccacccaaatctcaccttgaattgtaataatccccacctgtcaaggacagagccacgtggagattgaatcatgggggcagtttaccccattctgttcttgtggtagtgaatacatctcatgaaatctgatggctttataaatgggagttcccctgcacaagctctctcttagctgctgccatgtaagatgtgaccttgctcctcattcactttccttcatgattgtgaggcagccttgtgggactgtgagtccgttaaacctctttgctttacaaattacccagtcttgagtatgtctttattagcagtgtggaacagattaatacaggcatctgttaaagcagactaaatatggcctgagaaggactctgtatttctatatttgagtccttgtagatgaactgtaacctagcttaatagccagacaaaattgaaaacctaacttaatagtatgcaccgtaacaatagttgagtgttggccattccagtggtcatacttcaaccactcatagactgctgagtgttcaaacaaggcaaacgcagagctgtgaccaacctcactgtttctgtacttcacttttgattcccatacatcactttaactttttgtctataaatttgttctgaccacaaggcacccctggagtctctgtgtatctgctgtgattctggggatgcccaattcgtgaatcgttcattgctcaattaaactcctttaaatttaactcagctgaagtttttcttttatcagataatgtcagaagcaggatccaaagtggagcttctagtgacccccaggagtgctgagtaaacacgcaaggtacctgcaggacccacttgtgtccattgatctctcagagcagctgggcatcgtgggtaagttccctcttggattttggagctccacggatttgtgttttgagctctctgagtttctttgggcaaatttctgatccaaactgggtttggagttgtgacagaaactggactgggtccaggaacagatttgatccgggaattaactggcttggatccagttagaggcctcttacatctgactgggtcagaaaggaactggtagtaagcagtaatatttcaggggttatagagtttggcttttgaaaattcacaaggatttttgtgctctacccttttgttcatttttcttgcctgcatcggtaggaaaaaaaatcattggataagttaatcaagagagcctgagagtaaagccaatattttaggtaaaaatggaatccttaatttctggaaaactgagttccttctggcttatactttaggcctgggaggcagtgaagtcttacagaaatggcaaaatcttactaaaggtaacttacagtggaacgttccgaatgaacaacaatgcactgaagtacatttacaaatgagggctcttggtaaagtcccttttggctaagaacagggttggcactacgggatgtcaactgctgttttctttggaataatctgccttgcactctttgctgacaactatgggtgacagaattaggatcgtgggacacggagagctttttcctcccccaaaagggaaaacttgaaagctgatgggactgctggaaaaaaaatccttttacaacagcagctgcagccgcctgaacttctcagtatcactgcaatgggttggtttttctctggtcttcctgagcattttgccttccccaccctgccataggcaaaccttttctctctctcctttctgtttttcatcttttctgttactcagggcaaccatcatgcccagagaccatgtgttgaaactcctagtcagaggttggattaaagatgatggggcccagctgagggcaaatttaagccttgtcagtttgatattgggtgctaagcagagtggctaatgtctgtttatcacatgtgttttactctggccagaatgaaaaaagataattttcctttatgatgcagcttgtcccccaatgggatggtgtggcaagctgggttaccggggccacttagggaaaggaaacacagaaacctggcatgcaggccaaagggtaagaatttcttaccagtcagatttctggcttctccctctctgtgcagacagttgattaaatggtaaaaattgctgtttaagccaggcacggtggctcacacctgtaatcctagcactttgggaggttgaggtgggcggatcacttgaggtcaggagttcaagaccagcctggccaacatggcaaaaccccatctttactaaaaatacaaaaaattagctgggtgtggtggcaggtgcctgtaatcccacctactcgggaggctgaggcaggagaatcacttgaacccaggaggcggaggttgcagtgagccaagatcacgccattgcactccagcctgggcaacaagagtgaaattccatctcaaaaaaaaaaaaaaagaaagaaaaagaaaaaagtcactgtttatctcttctgtaaagttttgattaatgcaaaaaagaattccgaggctagtcttaaactgatatatttgtgctatgaatttgtttttctgtgtcaaggggtgccttaagataaaacatgggcttaggaccccataagctcgctgctcaagatggcccagcaggctggtcaataacaaactttcctgcaggtccctgaaacaaacaaatgaaaaactggatggggtctccatcttgtttcatgtccttgggagcttgaccttgtaaccacgtggcagtactttctcttggtctccaccttccagggaacacgaattttaggttttatgtcatagttagctctaaaaattatcttaagtagttaaaagcctctacaagctcaaaattaactactctagactccttctgggaagaacagtggaactttccctgtggtatagcttggtacataaggttttggcctttcacactagaagtccaggttcaattccctgcttagaaagcaagccttttctggtttaatatctacataaccttgtctagtctcttctccaccatggactatcctaagttttcctttcgctgagcacctgggaggttacctttggtaaagttcaaaaccagaaatattggccaaactgggtaataagaaattttaaaaggatattattaaagggtgctatggttaaaagtcagcttaattaaaagcagatattcaagctctaagagcctggattccttgggaaaaacaggaggcaccagaaacccatttcctggccctgttcttcctagggctccaccctaaagccaataaccaattaagaaacttaaaaactggcaaatgaaaaatcttataactactgtagtaatcttcttatgtctgtctatttgtgtaattatatatgtgttgtgtgtaatgtttatataaaagagctccaattaattggcttaaacaaaaacaagtgcttaaataaaatattttgaaagcaaaataaaaactgtaaggccttttagttcatgtaactttagtaattactgggaaataaaaacagctttaaagattattgataaaataaacacattttgtctaaattatgccggtcagatattaggtttgctaaatgctttaaggtcataaactgctttgacttttgaaaattgttcaatttattttgaagacattaaattctaaataaggcctggggatatatggaattatccatgtcccctagctatgcaaagaaggttataaagagattttacataagaaaggatgttttttggtaaattattgtcctaaagtaaaatgactggttgtttaaaaagagggatgtttagggcaggtcagaaagtctaaacatgtcatacatggtatgtgtaagtcgtgacaatttatgaaaagaaattaatgccagaaatgctttacaatttatttttttattattattattttttattatactttaagttttagggtacatgtgcacattgtgcaggttagttacatatgtatacatgtgccatgctggtgtgctgcacccactaactcatcatctagcattaggtatatctcccaatgctatccctccctactcccccgaccccataacagtcctcagagtgtgatattccccttcctgtgtccatgtgatctcattgttcaattcccacctatgagtgagaatatgcggtgtttggttttttgttcttggcgatagtttactgagaatgatgatttccaatttcatccatgtccctacaaaggacatgaactcatccttttttatggctgcatagtattccatggtgtatatgtgccacattttcttaatccagtctatcattgttggacatttgggttggttccaagtctttcctattgtgaataatgccgcaataaacatacgtgtgcatgtgtctttatagcagcatgatttatagtcctttgggtatatacccagtaatgggatggctgggtcaaatggtatttctagttctagatccctgaggaatcgccacactgacttccacaatggttgaactagtttacagtcccaccaacagtgtaaaagtgttcctatttctccacatcctctccagcacctgttgtttcctgactttttaatgattgccattctaactggtgtgagatggtatctcatcgtggttttgatttgcatttctctgatggccagtgatgatgagcattttttcatgtgttttttggctgcataaatgtcttcttttgagaagtgtctgttcatgtccttcgcccactttttgatggggttgtttgtttttttcttgtaaatttgtttgagttcattgtagattctggatattagccctttgtcagatgagtaggttgcaaaaattttctcccattctgtaggttgcctattcactctgatggtagtttcttttgctgtgcagaagctctttattttaattggatcccatttgtcaattttgtcttttgttgccattgcttttggtattttagacatgaagtccttgcccgtgcctatgccctgaatggtaatgcctaggttttcttctagggtttttatggttttaggtctagcatttaagtctttaatccatcttgaattgatttttgtataaggtgtaaggaagggatccagtttcagctttctacatatggctagccagttttcccagcaccatttattaaatagggaatcctttccccattgcttgtttttctgaggtttgtcaaagatcagatagttgtagatatgcggcgttatttctgagggctctgttctgttccattgatctatatctctgttttggtaccagtaccatgctgttttggttactgtagccttgtagtatagtttgaagtcaggtagtgtgatgcctccagctttgttcttttggcttaggattgacttggcaatgtgggcttttttttggttccatatgaactttaaagtagttttttccaattctgtgaagaaagtcattggtagcttgatggggatggcattgaatctgtaaattacctagggcagtatggccattttcaccatattgattcttcctacccatgagcatggaatgttcttccatttgtttgtatcctcagtggtttgtagttctccttgaagaggtccttcacatcccttgtaagttgggttcctaggtattttattctctttgaagcaattgtgaatgggagttaactcatgatttggctctctgtttgtctgttgttggtgtataagaatgcttgtgatttttgtacattgattttgtatcctgagactttgctgaaattgcttatcagcttaaggagattttgggctgagacagtggggttttctagatatacaatcatgtcgtctgccaacagggacaatttgacttcctcttttcttaattgaataccctttatttccttctcctgcctaattgccctggccagaacttccaacactatgttgaataggagtggtgagagagggcatccctgtcttgtgccagttttcaaagggaatgcttccagtttttgcccattcagtatgatattggctgtgggtttgtcatagatagctcttattattttgaaataggtcccatcaatacctaatttattgagagtttttagcatgaagcgttgttgaattttgtcaatggctttttctgcatctattgagataatcatgtggtttttgtctttggctctgtttatatgctggattacatttattgatttgcgtatattgaactagccttgcatcccagggatgaagcccacttgatcatggtggataagctttttgatgtgctgctggattcgttttgccagtattttattgaggatttttgcatcaatgttcatcgaggatattggtctaaaattctcttttttggttgtgtctctgcccagctttggtatcagaatgatgctggccccataaaatgagttagggaggactccctctttttctattgattggaatagtttcagaaggaatggtaccagctcctccttgtacctctagtagaattcagctgtgaatccatctggtcttggactctttttggttggtaagctattgattattgccacaatttcagctcctgttattggtctattcagagattcaacttcttcctggtttagtcttgggagagtgtatgtgtcgaggaatttatccatttcttctagattttctagtttatttgcgtagaggtgtttgtagtattctctgatggtaatttgtatttctgtgggatcggtggtgatatcccctttatcattttttattgcgtctatttgattcttctctctttttttctttattagtcttgctagcggtctatcaattttcttgatcctttcaaaaaaccagctcctggattcattaatttttttgaagggttttttgtgtctctatttccttcagttctgctctgattttagttatttcttgccttctgctagcttttgaatatgtttgctcttgcttttctagttcttttaattgtgatgttagggtgtcaattttggatctttcctgctttctcttgtgggcatttagtgctataaatttccctctacacactgctttgaatgcgtcccagagattctggtatgttgtgtctttgttctcgttggcctcaaagaacatctttatttctgccttcatttcgttatgtacccagtagtcattcaggagcaggttgttcagtttccatgtagttgagcggttttgagtgagattcttaatcctgagttctagtttgattgcactgtggtctgagagatagtttgttataatctctgttcttttacatttgctggggagagctttacttccaactgtgtggtcaattttggaataggtgtggtgtggtgctgaaaaaaatgtatattctgttgatttggggtggagagttctgtagatgtctattaggtccgcttggtgcagagccgagttcaattcctgggtatccttgttgactttctgtcgttgatctgtctaatgttgacagtggggtgttaaagtctcccattattaatgtgtggagtctaagtctctttgtaggtcactcaggacttgctttatgaatctgggtgctcctgtattgggtgcatatatatttaggatagttagctcttcttgttgaattgatccctttaccattatgtaatggccttctttgtctcttttgatctttgttggtttaaagtctgttttatcagagactaggattgcaacccctgcctttttttgttttccatttgcttggtagatcttcctccatccttttattttgagcctatgtgtgtctctgcacgtgagatgggtttcctgaatatagcacactgatgggtcttgactctttatccaatttgcctgtctgtgtcttttaattggagcatttagtccatttacatttaaagttaatattgttatgtgtgaatttgatcctgtcattatgatgttagctggttattttgctcgttagttgatgcagtttcttcctagtctcgatggtctttacattttggcattattttgcagcgggtggtaccagttgttcctttccatgtttagtgcttccttcaggagctcttttagggcaggcctggtggtgacaaaatctctcagcatttgcttgtctgtaaagtattttatttctccttcgcttatgaagcttattttggctggatatgaaattctgggttgaaaattcttttctttaagaatgttgaatattggcccccactctcttctggcttgtagggtttctgccgagatatccactgttagtctgatgggcttccctttgagggtaaccagacctttctctctggccgcccttaacattttttccttcatttcaactttggtgaatctgacaattatgtgtcttggagttgctcttcttgaggagtatctttgtggcgttctctgtatttcctgaatctgaacgttggcctgccttgctagattggggaagttctcttggataatatcctgcagagtgttttccaacttggttccattctccccatcactttcaggtacaccaatcagacgtagatttggtcttttcacatagtcccatatttcttggaggctttgctcttttcttttcttttttctctaaacttcccttattgcttcatttcattcatttcatcttccattactgataccctttcttccagttgattgcatcagctcctgaggcttctgcattcttcacgtagttctcgagccttggttttcagctccatcagctcctttaagcacttctctgtattggttattctagttatacattcttctaaatttttttcaaagttttcaacttctttgcctttggtttgaatgtcctcccgtagctcagagtaatttgatcgtctgaagacttcttctctcagctcgtcaaagtcattctccatccagctttgttctgttgctggtgaggaactgcgtttctttggaggaggagaggcgctctgctttttagagtttccagtttttcttttctgttttttccccatctttgtggttttatctacttttggtctttgatgatggtgatgtacagatggatttttggtgtggatgtcctttctgtttgttagttttccttctaacagacaggaccctcagctgcaggtctgttggaataccctgccctgtgaggtgtcagtgtgcccctgctggggggtgcctcccagttaggctgcttgggggtcaggggtcagggacccacttgaggaggcagtctgcccgttctcagatctccagctgcgtgctgggagaaccactgctctcttcaaagctgtcagacagggacatttaagtctgcagaggttactgctgtctttttgtttgtctgtgccctgcccccagaggtggagcctacagaggcaggcaggcctccttgagctgtggtgggctccacccagttggagcttcctaagcaagcctgggcaatggcgggcgcccctcccccagcctcgctgccgccttgcagtttgatctcagactgctgtgctatcaatcagtgagactccgtgggcgtaggaccctccaagccaggtgccggatataatctcgtggtgcgccgttttttaagcccgtcggaaaagcgcagtattcgggtggaagtggcccgattttccaggtgcgtccgtcacccctttctttgactcggaaagggaactccctgaccccttgcgcttcccaagtgaggcaatgcgtcaccctgcttcggctcgcgcacggtgcgtgcacccactgacctgcgaccactgtctggcactccctagtgagatgaaccctgtacctcagatggaaatgcagaaatcacccgtcttctgcgtcgctcatgctgggagctgtagactggagctgttcctattcggccatcttggctcttcccccgttttacaatttaaaggtgattaggcttcctaaatgcttcataaaatgccactatgactcttaactgtacagcttgcctactctacagctgggtaaggcctgggacacatggagttagacactggaaaggctcagatcttatctgcatttctgtttgggtcgtaggctccacacctagtacataattaaaatcccttaccaaggttttcaccaaaagtaaaagatgctaagagttaacattttaatatgtaattgagactactgaaaaaataagtttacatacaaggtttgtaaagggaataaaatgtgtttttgtgagagattataagaaagtatgggaatgtaaatttttgtctaggttagagggttaaagatttattttgaattaaaaagctaaaggttagaacaagttgtgaatggtttataaaaattaattacaagagattctatgtgtgaatgtattggctaaagttaaaatggcattattcattttttttctataaattggacattggaatagaagaacaacagagttttcttagaacattgttctgctctgagaaaaaaagttgtaaagggttataaaaggtttatgaaaatcttaccttatggtcaaactaattaaaacaatagatttataaaatgtcattaaaaactagctttaacataaaaaatacactaatgggaacataaaatttgtttttctcttttaaaaaggatttttatgtaatattaaaagataaaaggttttagtttaccttttaagtaagctacaaaagggaaaagtggagggaaggaaagaaaggagacagagtcaattgtcctaatgctatcttcattgggtcttgcttggaaagctgagtctcctctttatcagaatgttttgtccttttaaaaatttttgagttatcattttggctaaatgaatgacttatggtaacctaagattctatttggtaatatccaatgttttaaacatttggtatttaacaaacctttcaaaatcaagctctagattatcatgctaaatcagccaatactaaaattgtttaaatatacaatttaaatgaactccctggtctaagtcaaattacctatgataacccattagttatcagtgctatgcatctaaattggagaaacaactggtattcaagaggacatgagtctgatgttaagcatggactcatgaagaaccaggacagcctcctagtccttcccgagtccttaaagctcttgttactaaaggttctgcattccatgactcatcacggaaaagataaaataatccaaatagaatatactgatgtggtgacttatagatagtggaaatattttaaaaccaatgtttggtttcatattcctgggaaggcaatcaaagcttcaggtacatttggctacctaatgtgtcatttaaacatttataaagagatttcattcaattgtcattttcactgcatgttttctggttgtataaaagctttcccatgcaagagggctgatgtaacagtagattattgtgctaccatgtattttcaccaggtaaagaccttcacaatcgggaacccgtagattggatcttctgaaaacatcagagaaagactatctttgccatccacactacagtaaaactttggagccttgaaccttggatttataatctcacaactgagaagggtccctccatactcctggaactgtacacccattggaactcttaaggtaaaactaaccaggaaagtttctccccagaaaaagatggcatccttgatgtgaacagcttttcccaagatcacaggtcaaaacttctactatcatgagactcttacctttgaatatttttaccttgtttatgcctctatgagcaacagaaatgaaaagtgggtctataatgtgcacttatagggtataattttatttgtgaaggattttgcgggaagccagccttatacataaataaacttatactttaatagataaaagatgaaggcccaaggtgggtgagaaactttagtggtacatatgttgactcataatcagtcaaaactcctcttaacccacatcatggattaaagagaacattgccaggaggccttcactcttctagaaggacataatttgttaggtcctttttccatggtttagaatacaagaggcaataattagaaatgtctccctcttaataggcatgggttcaaataaggcaaacgtggagctgtagccaatctcgctgtttgtgtacctcacttctgattcctgtgtgtcactttaacatttttgtctatacattttttctgaccaggagacacccctggagtctgtgaatctgctgtgattctgggggctgcccgaatcatgaatcattcattgctcaattaaactcctttaagtttaatttggctgaagtttttcttttatcacacccttgccccatgagccagggaaagggcaactgaggccgcagtattttcagtggcaccaaggtacaccctgtattccacgagtagggtctggagagaagggagtccccgcctctcaaccagatttcagaaactatagtagatcttctatcctcaaggaaatgcatcttatttctggtatcagaatcaaggagaagcaggcaagactgttctataagatgagttagcatcctggagggtttttagactcaggaatggggatctctagggaaccgatagtaaaggttcctactaatctgggcaaatagagcttagtgttgcattacagctgttttctaagatggtcaatattgttctactctcttcctccattcagtaccttttttaaaacaattactcagaggtcattgcttatatcccaaactacttattaggacaatatcagttataaaaggttgctggattctctttgatttgtgccagcttcccatcacttgctgctaggaacctcatatcataagctgggagactggttgatatgcatagctccttacctattttatagtgttttccagtcttttatttcatgtgaattctgattgcctaacaagaaattttcttatcctactaaatttctcactaagaggaaatgtcaagcctctaaagctcttcccagctatctgtactcacagttaaattgaactgcagagactggtatgagtagctgattgaggaggtaatgaaatatcccaggctgcttttggcagcaactctgaatcaaccaaggccagccaaggcaaactttaaacgcaaaaacccggactaaatggatgaatttattctaatgtatttttgtccacatgcctctgcaaattgtttacaggttttctgccttttgactagtagaattttttattgcattcagatagatcattgatgaacactgctagtttcctgggctattgaaaatttgcctttcttattgggttttcatgaatgtttctctggtagagaaaggaggttaaaaaaatgagagattgctaactttctaccatcataaagtctggatttggatactgttttatggcaaagacagtaatgttcccccaaatttcctagaattcttgcagttgggttgagtcatgtggttagttgtggtcaatgggctcgaaatgacatatattgcctctgatatgaatcttagaagagtccacacaaacgtctccatctatcttttacttttctctattgaccaagaaggccatatggtagagccttcatcatcctgaataattggggaagagatctttttgacccgacaattgataagagccctggcaagtagtgtgagccgcagtaaactatttttggtacaagccagtgaggtttttaggggtggtttgttattgcagttgcctatcctgactaatgtatttttctacatacctaaaccatcaggtttcatcaaaacattggtggaaaataagaatatttctagatgatttgttggcttttcattcaagttgaatatgtacctatctattggttgaaaaaattaatagggattgtagacatgttattcttagtaggacaggacaggataatggtttttgaacattctccctgctgtatattagctttgcttttaaataaatacagtagtgaggtgtgtttatcagtgtttattctcccactattggataacaggggctccttgatctaaaatgataggtaagtgatcccctctactgtcctaaggtcattacttattgacacctccctattatgcctagtcaatgtgtgataaaagattgcatggaaatgacaggcatgaaccaggatcttttctcctctgtcctccttttcatttgccttttgatgtttctgctgctatttggcacctccactagaagattagaaggggaaaagagaggaaattaagctcttttcctgcagactagcagttctgatttttaaagggtacctcggggtattgtttcatctacttatgagtttcaggagtgtgtgtttgtgtgcgtggtggtgggggagaagagaaagagagaaagacacagagagagagacagatataattaaacatggagtttgagtttccatgttatctgattctaggaatttagtgttgcctccatatttatcaagaattatagtcctttaccgtaatttactataatgtattatgtttctgtgtgtgtgtgtgtgtgtgtgagagagagagagagagagagagagagaagagagagaagagagaaacagagagcgagacagagatggagagagagagagagaattaaacggattttcagagtttccacattatctgattctaggaatttagtgttgcttctatatttaccaagaattatagtcctttaattattatggaggataactaaaaatatcctgcataataattaaaagttccttattttcaagtggcataatgactttctgtgctaagatcacttgaaaatgttaattaaagaaatctatttgctcaaaaaaactaaatgtgcatactttacacctgtggtaaataatataaaattataatttgcctttgagcttaatcaaaatcagctttaaatttattaggcacctgacttttttatttttaattaaagaccattttgttcagtatgtagtttaaatcatggaagcgtagttacttctcaagcaattcctttaagacttggggcttctgtgtttgaagggatccaggggttacagtgtgggcagtacccctataccaatttaaggtttttcttactcagtaagatgttttctaagatgaaagagatgggtatattctatgtaacagagataaatgtaaaattttattcaccctatgggaaaaatttggatagattcctcttggcagtgaaaggtataaaatgaacttaaaggatgactctccataacataatattgagtgaaacaagaataaacacattatgactccatttataaaatatttttaaggtaaaattaagcaatttattgtttaaggacacatgtttggtaaaaccataatgaaaaacacatggaaatgaacacaaaataccatctaatgcttactttggggaacgggaagagagcctcaaacagagagatgtatgtggaggtttctaccactttagtgttatatttctaaagttgagttgtgaatacacagatgttgatttctattctagttcttcacactgtacatatgttttctgtactcttttggaactatactgtattttatgtatagttcaataagtgatagttcaatatgaattgttgatgtgatatgactcactcaaaagagttagtgtctcttgtacataatattgttaagaaacttggagttaaggaaattgaaggtattgtcatatccagccttgatcagaccatgctttagtactttgttcagttatatgcagcccactttaagagtgatgcagacaaactagattatgtttaggggacagtgatgaggctcgtaatgattcttgaaactatatatgatatatgattcttcatatatttgaagggaagacatgagaatgagagcttagatttatactacatactcaaaagaatagaatcaaaattaatagatgatgcaacaagaaaatattttattgtaacaaaaatagattttatcataacagaatcaagaacttactaataactacatttgttcaatgagtcgtcttgatacatagtgagtttcttactggtggagatgttctagcacaggttgaatgatctcttggtgggttattatcaggagatatgcctaaaagtcattctgggtcccgaaattcttcgaagatttccagaaatctctagtcaacctgaaatttctattcaagatctcttagttaagtggcagcggagtgagtaaaatcacagagtctaggaccagattcctgggttgaatcctggcgtttttcaattactacctgtataaccttgagaaaattacttctctgtgtttcctttttgcaatccataaaatgggtctatcagcctcacagagtggttgtaagacttagaagaatgccagatagtaagtgccactaaatgtttatttttttaagaaataatttttttctaaagatcagtcattcaatttactttgaatcaattacatttttgcttttgttttaaataaaaaaactttatttctctctcttcctatgagcaaatatatttaattatcctctgacatacaagggtattggagttttttttttttttaattttgtgggccctaaattctaacaattccagtaagtatagaattttaaactaaaaaatctcttaacctgacttaagtggctttagaatagctttgttgcattatcacagaaccacagaacccaaaaagccaagaagaacctgaaagaatgatttagtttctcttactcttggaattaggtaccttgtctgcaaagtctccttgcccttgagggattgctgcaaagcctgtctcattgttcaatctttgcatggctccttcaatcgttgctaatacgaggtggattgtctgttaaaagttaatgatggtgagccagggagtagtgtactgttttcggtttatttgcaacagtggaaagggcaaacctattcatctcaatgaaaatgtaactgtttacattggaagcttaaattttaggacacaccatgtcctgcttttgaaaagacaatttgtagggtaagagatgttacagtgatattatggaggccacaagaagtatattttctggtcattggtagaaaacaatgattaaaatcaggcttcttttgtaggagatactggtcatgttttctaaaatgttgactgtgagagaagaaaacaagaattattaaatctagatctctgatgggaagtaagaacagaaatgaggacaggtgaaaggaaggctagacatggtttacacaggtacatttcctgctgatgattggtagtggttgggaggggacagaaggcagggagatgtgaattgatgaggcacggagtatacctgggaatggtgagacttgaacctcaagttataacctaagattcacataaatcttgaaaaccatactcttgttttcttccaaacatggagccatacctattctaacttcttatgagtgatttgagcattatgacacctctacaggagatagagaaaaggcagagcaagagattgtcagcttggaatgcctctaggtgatgctggagatagcatcaatctgcttatcagggctttctgggtgtggtgtaacccagaatagcagtcaggataggctaggtactgctgctgtgacaaagtattttccaatcttgatggcttacaaccccagaggtttattttttcttatactacatgcttcccctgtttctctctccttcacaattctctagaataggggtgtccaatcttttggcttccctaagccacactggaagaagaagaattgtcttgggccacacataaagtacacgaacactagcaatagctgatgagctttaaaaaaaattgcaaaaaactctcataatgttttaagaaagtttacaaatttgtgttgggcctcattcaaagctgtcctgggctacatgtggctggtaggccatggactggacaagcttgccatagaggctagacaagtaagctttttgtgttttcctgtcttgttggcacttcctctttgtcataatcctctccttgccataggggtaattctctggggctataatagttaaagaacaacaaaaaagaacattggtttaatattttcaaaatgttaacccctttaaatatttgatgaagtggagatgttataagaataaatgtgaaagctattagaaaaattctggttaattggatatatatagagaaatataggctgactgctaaatatatgcagcctttctagcctcattggtggatggtaatgccatttggtgagatgagaattggttgggaggtgagggaaggtttcgagggagaaatctgtctagacttttattaatcttttgctagcttaaaaagtataattataggtgatttttttcttccctattttttacccctaaatttttcgtaaaagaggctttgatagtgaaataacctaatactgaagaacatatgtaggttacattctgaggtctgtgtctgggatatcccaggctgggttgggcctgatctgagactgaggaatgttgctgaaggaggctgggatgagcttcctgtggtttcttagatggtccttgctgggtggacagggtagggcatatggctcaggttgccaagatggtgctaaatgccttaatttggttcagaatggtttgatggatgcttttgatttttttttttaatgcttctcagcttgaaaacatttccagtttttgtccttttcatgggaatttattgaacataagtaagttggatgtttttcttgttaactagaagacttaatcatgtaacatgacaaaggaaagaaagaaaaaggatttatgattctaaagaatgggcaattcccttgaaggagtgggtcattcagtgaagctgtttgtttggcctgggttttctttaagtttatttttctcactcagttgagattttgactgtttctgactaccttcctcaactctatcactctttctatggcttgtggttggaaaacagggccatccaagtagcttgttgggtcccaggcgaatgccctttgactctcaacacctttttagaaaggtacattctctttcaaggaaaaatgaagccatgtaagggaagcttatgtacaaaataggataatccagttaactcaggttatggtgatttgtcctttttgtgtgtttgtttcagctgttgctattgaaaactcttatagaagaatttagttatttcttaattttatttagttaataattttagtaaatagatttactttttctatggcaaatgagaacctagcaatactacagaatcataggacatatacatgtacaagacacttattgatcttcccacaacatctaacatttctacatgttttgaaatgtttcttcagtagacgtgttctgaaatgttttgaaatgtttcttctaaaaactgttcactcctttctccctaaatgtgtattatatgttggtattatactgggtgctcagaattatctttaagaatgatggggtgtgccgggcatgtggctcatgcctgtaatcccagtactttgggaggctgaggtgggtggatcacctgagcccaggagttccagaccaccttgagtaacatggaaaccctgtctctactaaaaacacaaaaactagccaggtgcctgtagtcccagctactggggagacaggcatgagaatcactagaacccaggaagcagaggttgcagtgagccgcgattgtgccattgcacgcctgggtgacagagtgagattctgtctcaaaataaaaataaaacaaaataaataatgatgaggcccaattggtttctcaagaagtgcacttggtttctcaagttgcccacttggccctcccgcaagttgtactttactttacttttccttcctttccttactgttctaaagcttttaaataaactttcactcctgctctgaaaaaaaaaagaatgatgggaaacacaggggctgctaaaatcaagatcaagtactgtacctggtcttgggctgcttataagctagttggaaagaaaagacacacacttggaaagatagctaaaatatgacaaatagctaaaatatgacaagtgtcatgtgagcaaaacatagaaaaaaaggccatggaagttcagcaagggtatattctctgtgcacagaacaatctgataagccttctcagaagaaatggaattggagctgggatctgaggtttagattagcagagacggcagtgggaaggacatttcagggaggaaagaagcaaaggcacagaaatgaaaaagtagaatacatgtttgggtggggcaggatgatgaaagcaatgagaagattaatttgtttggagcagaaaccctcccatccccatcaccaatcctattaactcaaaggttcatttagttaaaatacagtaaagcttcagtcccttacttgcccttttgagtcccagtttccttatttgtaaaacgaggttaatcatacctaccagccatagattaaattattaaatgattaaatggattaaatgagataggatactaaaaggaaggtgttgagcagggttcctcacactttatcatccctcttcactcaattcattgcattcaatttaattccagtgctgtctgtcatactatcaagacatctcctatgctactcccccttgaggataatttaaatttgactgttattgcatttctctaaactagtttctattcaccttctggtttaggagaattttcttggcataagccatctgtatatgcaaaggagaccaatgtcacatttgagggctttaaataattcctcactaaccagttcagggtggctagagtataacaagctaaaagggagtagttggcaataagaaaggtgtctcagtttgttttctcttgctataacagaatacttgaaactggctaatttataaagaaaaggaatttatttcctacagttatgggagatgagaggtccagagttcagcagctgcatctggtaagagcctttttttttttttttaagttttgattcttttttttttgtttttttgtttttttattttattttattttattattattatactttaagttttagggtacatgtgcacaatatgcaggttagttacatatgtatacatgtgccatgctggtgtgctgcacccattaactcgtcatttagcattaggtatatcttctaatgctatccctccccccttccccctaccccacaacagtccccagagtgtgatgttccccttcctgtgtccatgtgttctcattgttcaattcccacctatgagtgagaacatgcggtgtttggttttttgtccttgtgatagtttactgagaatgatgatttccaatttcatccatgtccctacaaaggatatgaactcatcattttttatggctgcatagtattccgtggtgtatatatgccacattttcttgctaatggggatgctgcagagtcctgaggcagtgcagagcatcacgtggcaagggggctgagtgcgctaacatgctagcttaggtttttcttccttttcctatatagccacagttcccttccaatgataactcactatttcattaatctgtgaatagactaagtcattcatgagggcagagccctcatgacccaatcacctcttaaatgcttcacttctcaatactgcctgatatggttttggctgtgtccgcacctaaatctcatactgaattgtagctcccataatccctgcatgtcatggaaaaaaccccatgggaggtaattgaatcatggcagcggttacctccatatcatgttcttatgatattgagtgagttcttatgagatctgatgagatctcatgagatctgatggttttagaaggggctttcccccacttctctctgcacatctcctgctgccatgtgaagaaggacgtgtttgcttccccttccaccatgattgtaagtttcttgaggcctcccccgccctgtggaactgtgagtcaattaaacctccttcctttataaattacccagtctcagatatgtccttatagaggtgggagaagggactaatacagtaaattggtaccacagagagtggggcgctgctgtaaaggtacctgaaaatgtggaagtaactttggaactgggtaacaggcagaggttgaaaccatttggagggctcagaagacaggaaaatgtgggaaagtttggaaactcttagagacttggagggctaagaaggcaggaagaagtgggaaagtttggaacttcctagagacttgtcgaatggctttgactaaaatgctgatagtgatatgggcaataaagtccaggctgaggtggtctcagatggagatgaggaacttgttggaaactggagtaaatgtcactcttgctatgcaaagagactggcggcattttgcccctgccctagagatctgtgaaactttaaacttgagagagatgatttagggaatctgacagaagcaatttctaagtggcaaggtgttcaagaggaagcagagcataaaagtttggaaaatttgcagcctgattatgtgacagaaaagaaaaacccattttcttgggagaaattcaagccggctgctgaaatttgcatatgtgatgaggagccgaatgttaatcactgaggcaatgtggcagctgttttcagggcatgtcagaaacatgtcaaagttctcaggtatcctataatccccatgggtcatgggaaggacttagtgggaggtaattgaatcatgggggcggttacctccatgctgttctgatgatagtgagtgagttctcatgagagttgatgattttataaggggctttcccctccttttctctgcacttgtctctcttgccaccatgtgaaggaggacgtgtttggttccccttccaccatgattgtaagttttctgaggcctccccaaccatgctgaactgtgagtcaattaaacatctttcctttatcaattaccgagtcttgggtatgtccttattagcagcatgagaatggactaattctctgccacatttgggataaaatttcaacacaaattttggtttgctattcaaaccatagcaaaaggatactttccttcttgtagttttatcaacatcttccaggacataaatttaatggtaaacaacaggtaaaataaatgacattgctcaaaggaatgcaattaaaacctaactgctattgcatttaatccatagaggaatgtgacccaggtctggggagagggagcactgcattatgtttcattctcatgccatgtgagaatgtttacaccagcttgagttgttgtgatggggtcgtccatatcatttggttcttgtccttgtgactcactgcttctgctgtagagttagcttcctgcagtggaaaagggaggagttattttccagaccatatggagtagaaaacaacagattgacataggttttgtggaagctaaaggcacatgaactgaagcctcccagagtgtaaccttgcaaaactctttaaaatagcattttcatagaggtgtttagtatttaggatctatcttaaaaccttaagattccaaagttagcttacagaaaataggcaagagaggataaattgtattaggtatggaatttcactgcctctgcttgtgtttccaggttggagaagctggagaaaagaatgcttccctttgatttacctgggctggggagtatgacaatgtccatgtgtgtgtataggagattcttgtacttaaactctgtaaatgtgtgtttctgtggtcctatgctgggtggagggttcaactaaggtattgttaaggaatatggatgagccaaaaagactggaaagtttcaaatgcatgtgtgtttccaactaatattggagaaaacttttttggcatcgaacactggcaatttatagacttgttgattgatagtggatttacctttagagtgtacctggattatagaggaatctagcttccctgtctaactcatttatcataagcttactgaataactgctatggactatgcatgtgttagatgctggggtagaaagataaataggacacagtcccacaggaattatagtctagtggagagaggtgtatataaacagtcacagaacaatgtgataagtattatgatgaaggaatatgtaataactgctagcaaagagaaggaaacatttaaacctgcttgggagtggagggaaaagtcagagaaagctctataaaaaagctaactatataatatgtttggtaggatgagttacttggcaaatgggctggagttacacacccagttggggaatatgttgcctccaaaatccaaagagccccattaggcgttgtgcttttcttttcttttcttttttttttttttttttttttaactgtaggaagcaccagatgcaatagcttattccttgccttttaattcttttaattcctgcaagataaataatccaagccaaaatgaagcagaaatatcattagactgtcaccagttaaggctccagattaattgtctgagaggtagagaagagaaacaggaaagcagaaatagactttaatttaaaacacaagcaagtaagagtggatcagtcaaggggttctggcaagaaacacagaagaaacacagcatattctgaagagtagaactgatttgtgaagagactatgtcagagccatgataagaaaaccaacaaaggatagtgaggcacccagggactagcaacatcagggagctattagtactcttggggctgcaggggccagggaaggaaatggtgttaatgagcccagtgaaagctggcgtcatggaggaggggaaatagtttatcatgaaaacagaactatggctcctcactcacaatcacttccagacatgaaccactttacagactcagaataccctgaatgaagggaaggctggatccccttgaggaaggacccctgtacgtggacaaatatttacactgttaatattcctcccagaattccacaaagagctttatgcctttttaatggtactgtgcattgggaaaaaaaacaaaacaaataatttgaactttcagagattactggacactggctctgaactgacagtaattccaggagactcaacacatcactgtggtctaccagtcagagtaggggcttatagaggtcaggtgattagtgaagctttggctccagtttatctcacagtgggcccgatgggtacctgaacacatcctgtgattatttctccagttctagaatgcataattgcaatagatacattcagcagctgttggaatcccctcattggttcccttacctgcacagtaaggactactgtagtgggaaagacctagtgggagcagccactagaactgcctctacagaggaaaatagcaaaccaaaaggaatgctgcatttttggaggaattgcagagattagtgctgccatcaaggacttgaaagatgcaggggtgatgattactactccccactcaactctcttatttggcctgtgcatagaacagatggatcttggagaatagcagttaagtaagcttaaccaggaggtgactccaattgctgcatttcattgcttgagcaaactaacacatcccttggtacctggtatgcagctattgatctggcaaatgcttttccttcatacctgtcaataaaaaccatcagaagcagtttgccttcagctggaaaggccagtaatataccttcactattctacctcagaagtagatcaactctccagccttacaccataatttagttcacatggatcttgatcatctttctcttcaaaaggatattatactggtttgtcatattagtgacattatgctgtttggaagtagtgagcaagaagtagcaactactctagacttaagtcatttgcatttcagaaggtgggaaataaatgagacaaaaaatggaaagactttctatctcagtaaaatgcctaagggtgacaaccccctcaccccccaccactgccaaaaaaataagaacaatgcttaatggacctctttggattttggagtcaacatattcctcatttgggtatgttactccagaccatttgctaagtaacctgaaaagctgctaattttaagtggaacctagaacaggggaaggctctacaacaggtccaggctgctgtgcaagctgctttggctcttgcatcatatcatccaacagacccaatggtgcttaaaatgttagtggcaggtagggaagctatttggagcctctgccaggctcctataagtaaatttaggcatagtcctttaggattttggaataaagctctgccatcctctgcacataactattttttttttttttaaggaacagctgatggcctactacaaggccttaatagagactgactgcttaatcatgggctacaaagttacggtgcaacctgagctgcccatcatggtgttttgactcaccaagccataagtttgggcatataccacttcaaatggaagtggtatatatgtgataggacctaagaaagccccaaaggcacaagtaagttacacaaagaagtggtctaaatgccaatggtttcaactcctgttacactgccttctctccctcagtctgcacttatggcctcatgaggagctccctatcatcttagtacattttctgttgctataccggaatcaagcagactgggtaatttataaagagtagaagcttatttggcttacagccttagaggctggaaggttcaaaagcatggtggcagcttccagtgagggcttttcatactgcattataacatgatggagaagtggaaggagaagtgggtgtgtgtgaaatgatcaaaacatgaggagtggcctcagtttataatacccccagcccaatcttgtggtaatgaatcaagttccatgacagtgagaactcattccccagagaattaactgagtccttcaagagtgacattaatcccatttaaggacccaatgatgtcttcttcttctttcttctttcttcttcttcttctttcttctttcttcttctttctgagacagggtctcactctatcacccaggctggagtgcagtggtgtgatcttggctcactgtgacctcaacttcttgggctcaaacaattctcccacctcagcctcctgagtagctggaactacaggcgtgcaccaccatgcctggctaattttttatttcttgtagagatggggttttgccacatagcccaggctgatctcaaactcctgcactcaagcaatctttcctccttgacctcccaaagtgctgggattataggcatgaggcactgcacccagccacaatgactttttaaagtccctacctcccaacactgttgcaccaagaaccaaatttctaacacattaattctgagggtacactcaaactatagcacctatgatcaattgataggagaaaagattactcagacctagtttatagatagttctgtatgatatacaggaatcaatgggtgaaaagtgagagttgcaccattcacaattacattccattcacattcacaatttgctaatgacccactagcaaaacttttttttccttgttcctatgaccctgttctctgctggcctagaagtcttagttccaaatggagaaatggttccaccaagagacacaacaatgattccattgaactgcaagataagagtgccacctggacactttgaacatgcctctgaatcagcagaaaaagaagggagttattgtgtagactgagtgaagtagattgccttccccagtatggttgggcttcgtgcaatccattgaaggcctgcatagaacaaaaagaagaaaaaaatagaagtcactctttgcttgactgtcttccagctgggacattgattgttccctggctttgccctagaacttgtgctagaacttacatctttggatctacaggttctcagatctttgaactcagactgaaacttataccattggctctcctggtccttacccactggactcagagaagaagtatctcactggctttcttggtcctcctgctagatgactgtagatcctgaaaatttctagcttccataaccatgtgagtcaatttcttctaataaatatatatctatatttacatcttcatctatatctttatcttctattctgtttctctggataattcataccaatacatattttggtactgaaaagtgtttgtagttctgtcataacaaatacctaaacatgtggaagtggctctggaattgggtaatgaatagaggctggaagtattttgaggtgcatgctagaaatatggatgttaagagcaattctgatgagctctcagatgaaatgagaaacatatttttggaaactggaagaaaggcgatctttgttataatatggaaaagaatttggctgaattatgtttgggttctagtgtttgtggaaggtagatcttgcaaatgatgatattggatatttagttgaggatatgtctaagcaaatgtttaagaagtggcttgcttccacctgactgcttatactaaaacctgataagagacagttgaagaagggattgttaaaggataagttgaagaaggaattgttaagcaaaaaggaacctgaatttgaagatttggaacagtttcagcctacgtatattgcaaaaaaatgaaaaagtattcagaagagaacaccaagggtgtgcctggactgtcattcaatgaagagcttatgggactatataagcagcaacattgccagtttaaactgaaggagatgcagaaaggactaaaggaaggaaggttattagactcatcaggatttgtgggggaaaagatgaaagagtcttttggctgtgaacatgtgctatccttcaataagaggaaaaatgaccctaaaggtaattcagaaattaacagagccaccatcttgttttcaataagtcagatgccctctttcttgaagctgtgaggccaggaccactttgttgtgctgaaggatcaggacaccttgaagaacgctggggacagggtgcctggaagggccatgaatacaggatctctgcccccatgggttttgaagataggaccccagtgggtctggaagatagagaatcaagtcaaagagaatgattcttgagccttaagatctgatggaatgtatcttactaggttttagatttgtttgggactaatcatccttttctttcctatttttctctcttgtaatagaaaggtctttcctatggctggctcgccattttagaagtacatgacttgtttggtttcacagattcagagctgaatctgaagaggaattttgcttcaggatgaattgtaccttgagtctcactcatacttgattcaaatgatatttcgataagactatggactttagactttagagttgatgctggcataaattcagacttttgaggctgttgggatgaaataaatgtactttgcatacaataagaacataaattttggggggccaggggtggaatattatggactgaatgtttctgtcatcactgaatgtcatgtgttaaaaccctaactaccaatgtaatgtggtttgaagatggggcatttgcacagtaattatagctaggtgaagtcatgaggatgggaatcctcatgatgggattgttgtacttctaaggggaagatcctctctctctctctcggctccccactccccaactctaccctaggtgagagcacagagagaaagtggccatctaaaagctggaaagataaccctcaccagaactcaaacatgctggcacctgatctcacacttacaacctccacaaacgtgataaaaaaaaattctgtaatttaagacctgtagcctatggctggcattttgttatagcagcccaagcacactaaaacagtcaattaagtttataatattattcagatcttctatcactcatcaactaattttttgtgtctacttgtcctgttaattagtaatagaggtgtgtccgaagtctccaactgtaattgtatatttgtctatttctcctttcagttctatagattttgctttattttggagttttattgggtgcatatacatgtagcaatattatgtctttttaatgaattgacccttttataattacataatgttgatgttaatataccttattctgaatactactttagctaatattaatataagcactgcagcttcccttaattaatagtataatttttccatccttttactttttcctttgtctttataagtagatttattgtagacaacatataattgcattttacttgtttgtccaacctgacaatgttaggctttaattggagtgctaattccagatgtatttaatgtaagtattgatatgtttgggtttaaatataccatcttgctaaatgttttctacttgtcccattggttccttgtttttcctttcctcttttagtgcctacttttgaactaaatatttttcattattatatttattttcaaaattggcttattagtggtttctctaggatttaaacatctttaacttatcacagtttacttccaaatgtatcactttacatagagtgtagtagctttaccacatatacttctatttcctttcttccaaccttagtgctattgttgttacagtttttacttctgtgtgtattatcaaccccataatatattgttactattatagttttagacaattatattttaaaggaattcaaaatttaaaacatcttttatacttaaccatatttttaccatttctatgctcttcattctttcacacagatgtaattttctatctggtatcatatttcttgtgcctaaagaactttcaataggttagttgcaggtctgctggcaatgaattccctaagcttttgttggtctgagaaagtttttattttatctttattctgaaagctatttttgctggatatatcattatcagtttattgttgtgcttgttttattactttgaagatgttacatcatctgctgaactgcatagtttctaaaaagaagtctggtgtgattcttatcttcctccctatgtaatgtttcctttttcctcttctacatcaagatttttctctttaaacttgaatttcagcagtttgactacaattttcatagctgtgtttttaaaatttttgtttatattgcttagagttttctgagattctttggtctggttttttttttttgctttttgtttctgtttttgccttcaatttacttcagacaattcttgatcattacctcttcaaatatttctttggttcttgctgtcttcttattctggagatacaagtccatgtatattagactgtttggttttattccctaatttttggatgatctgttcttttttcccatgcatttaattatttaattttcagtagttcctgtcatcaagttcatcaattatttcctcattgtgtctagtctacagataaagttgtcaaaggaataataataataaaaaaactctagaatttccattggtattggtttcctattgctgctgtaacaaattaccacaatgctactagcttaaaactacacaactttattatactaaagttctggaattcagaagtctgaaatgggtctcagacttgtctaaaatcaaggtgtcagtaaggctgcattcctttaggagactctacaggaggatctatttccttaccttttccatcttctagagaccaactgaattccttatctcaggacctctttctccatctttaaagccatgttctctttctccatctttctccatctttaaagccaaactgcaaatcatctccaaattactctgtctctcctggttccctctttcacagtccttgtgattacattgagcctatcaggataatcctggataatattctcatatcatgatccttaacttagtaacatttgtaaagtcccttttgccatgtaaggtaatatagtcacaggttcagagaagtaggacatggacatctttggtaataatggggtgtcccattattgtgctgatgacaccatctgattctcaggatttccacctttagtaggtagaatggtggcctctcaaaagatatatctatgtccaaatccctggaacctgtgaatgttatcttacttggaaaacgggtatttgcagatgaatgaagttcaggttcttgagagtagatcatcctggattacttgtgtgattcctaaattcaatgataagtgtgtttgtaatatacagaagaagttaagacacagacagacagaggagatggcaatgtgaagatagaggctgagattggagtgctgtggccacaagtcaagaaagccaaggaatgctgactgcccccagaagctgcaaaaagcaaggattttccctttgcacctccaggagtgtggctctgctgacaccttgatttcagacttgaggcttctagaactgagagaataattttctcttattttaagccacccagtttgtggtaatttgttatggtacccctaggaaaagaatacatctttctgttgaaatctttatctctttaagtatgtattatagtttttccattagatcctttaacgtattaattataattattttaaagttcctgtctgttagtttcaacatctggaccaaattctgagtttgtttaatctcttgacaatgggttgttatgttcttgctttttgtgtatatggcaattttgtttacataccagataatgtgtacaaagtaacactagaaactgagctaaataatatttatgcccagcagtaggcatgcttcttcttctgttagatcatgagtctttgggcagttgaggctctctgatatgtacatgagctgagtttaagtttgctgttgtcgtgttgatatattgttatattcagtgaaccctaggcttcaaattcctcctgcggtagacaagtgctaccttatccttagtgtgaggtctgaagtgctagaggaattttctaaatgtttcttcactctcagctttcagcaatccatgtatgactttgccactggggggatttatctccatgttcttgtatttaccctagcctagagacttcagttgtttgttattctgtgcaagactcatgctggagttggaagctttcacttctcctgttccagccttagtttcaggcaggtcctgtgctcctgagcctgatgtcagttgttttgaatacccccatgtctctcccatgacaagcctttgcctccttttcagtccatgttttagagtgcaggtaggtttcctgtacttccctccccgctgaacaggtgaactctgcctccgcccccagcaatagcagtcctcttctttgtattagtgcaggatcctgcgcatgagaaagttttctaccactttcccagtagcagcctacctttgcctggaaatagggacatgacagggtttcatgtccctccctcagtggcagattcattttacttcatataaaagcattgtcatgtctgggatgtgaacatgttctttctatcatctcaacagcgacagattttacttcctatctgagaacattctgggctgtgggaagtagcagctgctcaccatactgtactcatgcagagcccattgagagatgaaattccatagacactcctgtggccgggcacggtggctcacgcctgtaatcccagcactttgggaggccgaggagggcggatcacgaggtcaggagatcgagaccatcctggctaacttggtgaaaccccgtctctactaaaaatacaaaaaaacaaattagctgggcgtggtggcgggcgcctgtagtcccagctactcaggaggctgaggcaggagaatggcgtgaacccgggaggtggagcttgcagtgagccgagatggcgccactgcactccagcctgggcaacagagcaagactccgtctcaaaaaaaaaaaaaaaaaaaaaaaaaaaagaaattccctagacactcctgctcttctctcaaacctcagcagaccctgtacacctgtgccaccaagaggcgccttctccagcttcctacctgccctcaatcgttcttgtgaatattcagatgagacccatcaagaaccccatgagtgggtgcagacttgcctgtgcctgtggcacctgaagattctacactttcacactagtccacatttgtcctttaagaatgtgctaaatttcatctattttcatcttactgactccaataactgcctcccttccctcctattctccctaaaaggtgaaacatttgagtgtcctatgttacctatgaggagcctttcacccttaggaatttagttcaactgatcaacctcagcgcactgatgaacttgaaaactattttgtagattttcagctttttttttttttttttcctgaggcagtgtaaattatttaagagtttagattaccaacttttcctgttttggtgatagtgacattcttttgcagtttctgtatcctaagtgaaattagaactatattcattgatttaacagatattcaaatcaacaaatgcatacccagaggaccaagtgatgtctgaaacttaacatatatataatggaacttttggtttgccccaaccattgcctgttccaccctaagcctatctctgtaagttgtaccactgtccacctagttggttaagccagaaactcaagtgttttcctgattttctcttcttcacctcatacatccaatacaacagtaaccactataattattgattctatttccgaaataaatataaaacccatttacttttttccattattgctgtcactagtgtggtccaagctgtcatcatctgttgtctggacttctttgtcaaccagaggatctcacagcttttacttttgtcctcgtagactacatcatccacccagcagtcaaagttaaaacataaatcttatcacattctaaaaatataagtaaattttgagcatgtcaaatccctgctcaaaatcattcagtgtttccccattacctttctaaaggcaactcaatctcaactcctcaccatgacctgcaaggccgtgaatgatccagccctgcctatttccacaacaacttcatttggggccactttcttcctcactcacttattcatctgttgagaaaagagaggcacttttaacttatacatgtctgaagaatcagagcagctgtgaacataccccagaactctgaaatttcaaaagtataaaatgttaatccaaaaagaattctaaacttcaaataatcttctttttgcttattttttatggcatatgtgcattattatttcatcactttcaaaactgacacagtttccatagttaacttcgagttatttttgtgaactgactattgaacgaaagctctccatttactaacaacagtgtagtcttctgaatcttttagctcttattgaaaaaaacattcctttgttatagagtgcaatgtggtttgttttggagggagtaaaggaggcaggatgtctgtctttgcttggtttcctggccagtgcatctcatttgaaaatagtttgtttcaagtagttaagtctattcctgggaagcctctatttttatatatttttttaatttttagacaaggtcttgctctgttacccgggctggagtgtggtggcacaatcatagctcatagcagtctcaaactcttgggctcaaatgatcctcccatctcagcctcccaagtagcttggactacaggtgtgtaccaccatgcctaattgctttttttcaaaattttttagtagagatgaggtcttgctgtgttttctcaggctggtctcaaactcctgggctcaagtgatcctctaacctcagcctcctgaaatgctagattacagacatgagccactgtgagccttttatttgtttaagttttattttttcctttcttcccttctcccttcctttctttcttttgtttttagacaagtaatttgacattaggaggtcttgaaggtgatggtttcctctggcagtagtgccttttctgtcactgaaggtgttcagttggtcagaatgcatggccaatggaatcattctttcattaaagaacaaacatttgttaaacgcctccctttgccaaagcattgggacactcactaggagttcaaagataaaaaagcacgctttttaacaagtgtacgtttcagtgtcagacatacagttttaatacaactgctcattgttctaatgggaaataagagattcagccattaaactactgtgtggtgtagaagaccttttaaaatagactgatttctgagagtctgtgatttcacttataaggcttatgagggattcttagcaaggaaaaatgagaatcgtttctggttatactaattatgaactttgtgagccttgagcaagtctctaaactttctgaagctcagtttgttttcttatattttaaaagagaatattttgaagagagataaatggaataatacaaataaagttccagcacctattaagtgggggtaaggtggagcagtgtttactgaaaatgaaaattagattaaaggacagacacttcagggccatttttttttcctcctccatatgtgtgagtgtggatggggtagggagaggagggtgttttataataaagaagtaaacggaaagaaaaaatgtgaagatatagttcactgggggaaacactgtaaatatagactagtgacaggcaatgaactgcaggacctgagctggttctgaggcagtgagcctcagctagaacatcccatatacatcgcaggaggatgatgacgtttaatgtgtcaaagtgtacgtaactgatgacagttttgtgatcaggctttgtttgcaatcatagagaatccagaaaagttaattttaatactcttgattttgacagataaattctttttaaaatgtaaaattattatttctcattaaagaaagaagaataggacattcctagccttttttttttttttttttttttgagacgagttctcacctgtcactcaggctggagggcagtggtgcgatcatggctcactgcagcctcaactttcaggctcaagcgatcctcccacctcagcctcctgcattgctcggactacaggcacatgctatcatgcccatctaaatgttgtattttttgtagagatggggtctcggtctgttgcctgtgctggtcttgaactcctgggctcaagcaatcctactaacttggtctcccaaagtgctaggattacaaatgtgagccactatgcccagcccctgatctattaacattttagaaactagttctttgtgaggctctttcataataaattatcagtatgttacagcattatacaaattgcaagtgctttcacatggataatctcatttttatcacccccttttacacatgagaaaattgaagctcagaaatgactagtctgaggtcacacaggtaagatatgccaaagttgaaacttgaactctggtgtttcttatcatgctgcacataaaattatggactgtgcctcaggttaggagaaatcagaattttcaatgaaaatacaattaaaattggattagtatgtcattctatctttgatcagtcttaaccttaattggctaatcatataaaagctcttacactgtgatctaattcagtcctgctggacaaatgctattctattgtattcaatatgatgtcactgaaaacttcatggaatatattgagctggaaagattagacaaacaactcctcacttacggtgcacacacgcacacacacacacacatccccacacacttacacatccctactcatttaaatatagaactgtatacaataattaatataatcaattaatatttacatattacgttattagtaagttacttttgaatactccagtataaataatgtaaacaaattaactttaatcaatactttagggccagttagttacagtaatgtaataaaaaatgtttaacaaccagctctggggaggagtagagtcctgatttgtagcatttgctgatttctgtccatcaatactctcaccatggctggtttcaggctcccagtgtgaggtcacctaatgcaggaatacagatgctgctatttaaatctgcaccagagggttcattgatgagggtaagggatgttgagcataattttgggggataagtaaatggtgtccaatgtatgtctggctgaaaaaagattacacaggcatctttgtccttgaaggaacagtattgaaggacccatcaagcccagaagccttacatcttcagagtatcccctgggtctagaactttggttctacacctccctatttaatcaaggctctattacctgatccaattacaggctttgctgattcttctgttagattattattgtaaagcttgttggagtgcctaaaagatagatatcagggactgacttcctcaagccaggggaatagtttctatgactattttgaagcttgcttgctaatagatatttctatgtagcagaatattgtctaagatttcctttattacacttgccacctaatggtgaggtgaaggaagaagtcatagcttccatttctcttttatcgtattaccaaatattgaggtgataaatatttaccaaaaaatctgacagttgtatagggccaacttggtttattatatcaatttgcaatatcggtaagtacctactaagtttggggcactataacatgataaaatccttgtctacagagagcttttaggtggatttaaaaatgcagtgttaccatttctatttataaagtgtgaaaacaaagtggatgccagatcacacacaagccagcagagaatgtctcccagtcttgtttacagtactgggattgtggtcaaggtgaatacacacagtcctttactctcttatcagagagtgaaggtttaaagagaaaccaacaaaagtgtccaggtactttttttttttcttcagacagggtctcagctaggctggagtatagtggcacgatcacagctgactgcagccttgatctcctgggctcaagcaatcctcccacctcaggctcctgagtagctgggactacagacgtgccaccacacctggctattgttttaatttttttgtagagaccaggtctcactatgctgcccagtctggtcttgtactcctgggctcaagtgatcttcccaccttggcctcctaaagttcttggattacagacctcaaacaccatgtccagcctccaggtactttttaactgtagtgattatgtggcattttgatgtaatggctctaaaatattgcccctgaattcttggaaacttcttccttgtagaggttgggtgtggtctatgtccttttccttaaagctgggtttttgactacttgaccaatagtacatggcagaagtgttgctgtggcagtttcttaagatacaggtctggaaactggcacttgatctggtaaggtccgaactatataccaagaaactggctatttccacttcctatctctgggatatttgctgttagaacctagtctctattctgtgaggaagcctaggccacctcatggagaggaaccaataggcagcatcaacttaccattcatgaaagtaagccatcttggaggtgggtcatccaaccccagttaggccacatggagcagagataagctgtcctgctgagacctgccaaaatggcaaattcttaaataattattgctgtttaagtcatgaaattttggggtagcttaatatacagcaatagaaacctggacacctagtaatctgtttgtgagaagagactatcagatgcttctcagtactatttttcctgttagttggtgactcattcctttgtagacagtctatagatttcttttgtgtttactccctcttggggacttcccacttgtgcctgcctcctgtttagcaggaatctgtagcagacaaatcccaagctgaagcagggattaggggtgagcttctgtgagcagtggaagtttgcacaacctaacaaagaggtaatttctgcaggggtgcttttggcaagagagatgcccatatgttggattgcataattcttttttcttcccagttgggggtcatcaggtcatctgactgctaattcttcaggtatggacttttcttccagctctgtgaatctgttctaaagggtagagtctgagatgagaatctagagacacaaattgttgctgtgtcaccaactgtgtgagctcaatcaagccaattgacattactaggaacataatgggattaagatacttagaagccctacacattgaacatgttatgatattatgaccccagatgtaatgtaagcaaatacaacaaaattctgattttcaccaaggtgactacttgatgcattttttgaattaccaaatgttaaatttgttaatttttgttattttagtgttcctaattagtctacctagtgaataaccattgtctaggcctcaattgcttcatccataaaatagataagtagatggtttgatctgttcgatttcttttgtatctaaattttgattctgcaatcacttttattccctttcctttgtttggtatgtttttttttctctttgctatagctttattgaggtataattgacaagcaataaactgaaaaatctaaagtgtacaatttgagaatttttgacatacttttacaccgatgagcattacctaatcaaaacagtaaacatctccatcatctccacaaatttctttgtgttcttccctttcccttttcttaccccagcttctaggcaactattgagctgctgtgtatcactatagattagtttgcactttacagaattttagataaatggaattctagagtatgtattcttttttgtctgacttctttcactcagcataattgatttgagatacagacatgttgttgcatgtaccagtagttcatttttttaagttgctgagcagcattccattgtatggatatgccacaatctgtttttccatttacctgctgatggacatttgggttgtttccagtttggggctattagggataaagctgctgtgaacattcacatataaatacttacatagacacatgattttatttttcttgggtaaataaatacctatgagtggaatggttggatcatatggtaattacatgtttaatttttaaagaaatggccacacttttcaaaagtcgtggaacaattttactttcccactggtagtctgtgagagttctagtttctccatattctcaccaacattttgtatggtcagtttttaaagtttagccattctaataagcatgtagtggtatctcattgtgtcttaaatgtacattcttgtggtaactaatagtgttaaaaatcttttcatctgcttattggctgatatggtttggctctgtatccccacccaaatctcatcttgaattgtaatctctgtgtattgggggaggggcctggcatgaggtgactgaatcatggcagtagacttcccccttgctgttcttgtggtagtgagttctcgtgagatttgatggtttaaaagtgtgtggcagttcctccacactcactctctcctgcttcaccatgggaagaaggtatgccttgcttccccttcagcttgtgccatgattttaagtttcctgaggcctcccagtcatgcttcctattaagcccatggaactgtgagtcaattaaacttatgttcttaataaattacccagtgtccggtagttctttatagcagtgtgaaaatgaactaatacatttgccatctgtatatcttctttggtgaagtgtctgtcacaatattttttctagttcttaaaaattattactgatttttgagagtttaaaaaatatattgtgcataaaagttgttagatacataatttgcaaatattttcttgcagtctgacttatattttaattctattaatatttggtatgttcttaaagaggaaaaaatcttaacatgtgaaatattttacatactcttaagttcaaagagcagcataggtggatctgggaagaaaaagacattagcaaaccattcaatggtttggcattgaatgcctttgtgtaagattttctttagttagcttttattaagtgacttttgtgtataaagtattgcagtataagtaaacattgtagtaagtaatgttttagcttgaattctgggctttatgcatgtttttcagaacagccaccaatttagactcatggtttctctcagtattatgcctggtctacaaagagtctaagctaaaacacccatgtgtgatatctatatctcccacatcatcatacaccaatctatttctatttctatatatgtatgtataacttgcaaaaaatccaacttatattcatattcaacttacatctttggtcaaatataaccatcaggcaaactgttgtgacctcacaggtataataaactaaatgataatataaaatatgtatcacaaagcttgtgcactttacttcacagtagaaacatggatctgccttcaggtacttatgtagacaattatttataaagcaagatagattataaccagtgaggccacactgacagcatgtggaaaaacagttcacaacagtgggaagagagacagagaaaatacagaccccaaaactagaatgcaaagaagtctggatatattttgtatttgtatagaaagccttttaagtatgaatttcccagaggacatggagtcatgagatttgtaataatttatctcagaaatgcttggaataaattataagttcttaaagggaataaggttttgaagaatgtatagttaactccttgataatataatttatattatgatatgatcagaagctataaaaagtataaaacttgccaaagaagggagtgagactgctgaatgaagttaaagtagagggtttatcttgaaaattcttctgctttaaatattctgaatatgaaatagaaggatatggttaattgtcagtgggagagaaaggaacaggtattgaatggacctctgtattgtaagagtaaaagagaaattcccaaccaaccaattattaaacctcctaatattaagaatttatatctagcatttgaaaaatttgatctagaaatttaagaacaggtagaatttccttcatcatccctgttatttcctctcttagtgcttataagtacaaactccagaacagtctagtttgagtttgagtttcaacatcatcagtgggttggcttccacaaacccaagttttctaacctacagaatggaactaaaatccccacctgaagaggtggtggtgaggattataggagatgcaggtaaagggcttagtatagtacctggcccagggttttaaacacttagtaaatataaaatattacaattattgtttattctagggagaaatttgaaggacaagcagcactgaaaaattcaagcaaaaacattagcagtcaatatcccataatttgaaattaaggattaaaattaggtattattttcatctgtttttgtttctcttattttaataaaaaagctgtggaagcccccagaaataactgccagcttttggagggtgtctctggatgttttgtgtgttccatctgggctgcagccattattctacctacttgacagacgatgaggtcatggaggccaagtgttcttcacgacgacacccaggtcaaaggcagagttaaagtacatcccaggtcacataactcattctctgttcaagaatctttcctaatccctggtgccatttgggaactgtttcaaaggcattccaacctcagaatcatgccagtgcactggttatcaattattttgttgatcctttagcaaatcctcaaactgatttttctgccctcctgagacacaaatcacaaagctgaccttaagtgctttggcatccccctccagtcccgaggcacacaaaaaagcagtgcagggttggtgatttattgttttcccacgcaggtcacgctcaagcccagacagatagagaagatttgtctttaacgagagaaatgcaccattacttggtcataaattcaacttaatggtaattttagtagggcagcttgcccagggtttgtagaaacacaaatcaaaaatcccaaattccatgcatatcctcctagaaactcttttggcaactcccttccatttgctttttaaggaaatcaatttccttagttatggtccctagttgcttagggtggttttgcacagagtctagaatcactgtggcagcagagaggggagtgggtggcatgctgcttgaactatttttgccaagcattcggccttgacttcagttgtcaaggaggcacaagtgagctgacacacagattcggtagacagtcccaaaaaagtagtatgtggtgaaaatgttcagatgactctgtctaaggaaaaatttttttcaaatcctcctgtccttgactgattccaaactgacaaattctggtcattatgaatctcaggtcacataacaagctctgaatccttacagagttggtttagtccaagctggcatagaaatatctatggagtatattcaggcacaaggctaccagacacccctccagactcttagaagtagactcaaacataccatcttgtatgcatgccatatcctgtgctccctatgatcatagcaactagaagaccttattgtccttaattacttatgcgtgttcccttatagcacactgtgtgctcccaggtgtatggcaatgccatacctgaatttgtttctccagtttttaacccagtgcctgacatgtgacagatgcacagttagcattggttgaatgaacagaagtatgaatgaataacgttcatgcctttccagtaaggtctgacttttaagttggggaacctgggaaatggccattccttcttcttctttttttttttcaggatgatatacatggccaggtgaagacagtagagagaaaacagaactgaaagtaagtgtctcccataagtagggtaatttgtactttatttacttacaccaaaatttacagaatgccaatacagtcaaaatatagtgtcaggtactgaagaatatttaactaggaatcaaagaactcaagatctcttactctttagatctaagatccaatgtataatgctaccctaaattactttattcttaatagcatcactctatccagagaaaatacacgacattctagcttctctgatttggttttgcagatgggtctacctataaccttcccctcaggggtagagaggagtttagctggcagtttatttctgtttctactcacacgcctagcatatgagaaggctgggattagagccaaaggagaagcctggaacacccaggtgatggcatgtttggatccttataattctctatgaaagagtgaagagactcaaaggctatggctctccagcttgagtgggcatcagaatcacctggaaggcttcctaagacacattatttctgggcccccacccccagagttcctgagtcagtaggtttaagttcagattccagaagttgcattcctaggaagtccccaagcaatgcaaatgctactggtttaggaccagctgaactaaggtaagccctgacactttccaccaaatcaaattctctcattccctcatataatgccacaagatgattccatttgtatggttttgtccaggtagccttggactcaaataaaagaatcagttggaattacttatttcatagctgttttccactgatctggggcaaattttttgtgccagataccttcctttgtggtttaacctgtatttatgggctgcctctcttgtcattagttggaaataaaaacaatgatagtatcaatgaaagcaacctgcaaaagtattgttaacatagagatgcatacacataaactgtttattcatgccattgggcttgtgtggataactgtgtaaaataatgaatttaacattagcctttggattttttctcctttccttcatctgctctgactaggagaataattgtagcttcagtctaaatggagaaatattagccaggtctttctgtcttctagataggtcctgtagtccagccaagctatctggatttctgattagacagaaatccatttttataaagagaaaaaaatgtattttctcaagaattatttttagttattttctctcttgtgatgaaaggcttatctaaatagcccaagcttcattcaagattcttccccactctttgttgtcacccagccttccctgacctcactcaccctcagacagccagggatttaaaaatacgttggaagattttaatggtctctgcagagtagaattacattcttctgtgtaacatttggacaccaagcagagagatagcacagtctgtctagctcttttgtaattatttcatggtattgttttaattgtggcatggcttaatcactggctgtgcacagattatgccacatacttaaaataattacagggatttggtaagataatgctgtgaattcatttaatgcttcttttccaatagactccacactcttaaaaggagagagaagcaaagaaggacagtcaatcaatgccagcattggtcattttctgcaccttgtgaggactgaccaggatgatatatgcacatttttttatttcagtcatcttccacctgcccaaggaggcattttatctagtactcaaagatcctgaaactagtgtgacaccctgttaagatccctttaccagctaacacttaatataggttcacaactagtaacctagccaggcctgtgtgaacacattagttttaaatccaatggtttgtctatgtaactgtattagggttctctaaagggacagaactaataggataggttaatatatgaaagtttattaagagtttattaaggagtattgactcacatgatcataaggtgaagtcccacaataggctgtctgcaagctgaggagccaggaagcaattccaagtcccaaaactttaaaagtagggaagctgatagtgcagccttcagcctgtggccaaaggcctcagagcccctggcaaatcagtgatgtaagtccaagagtccaaaagctgaagaacttgggagtccgatgtttgagggcaggaagcatccagcacaggggaaagatggaggccagaagattctgccagtttagtccttccacattcctctgcctgcttttatcctagccatgttggcagccgattagatggtgcccacccagattgagagtgggtctgcctttcttagtccactaactcaaatgttaatctcttttggcagcaccctcactgacacacccagaaacaatacttcacatttttcaatccaatcaagttgacactcaacattaactatcacagtaactgatgactgctatctccattagcagttctttagcttcagaagagtgtaatctggttataaatctttgttagaattacttcgttggttaattttatgtgtcaacttgactggcctaagcaacgcccagatagctggtagaacatttgtcctgggtgtgcctgtgagagtatttctggaagacactaccatttgaatcatcagactgagaaaagaagatacactcttgccaatgtgggtgagcatcgtccaatccattgagagccaaatagaaaaaaaaaggtggggcaaggtgaatttaatctcttttcttgagctgggacgtccaactcctcctgcccttgggtcttagagttcttatttcttgggcttttggacttcaagacttaaaacaatgcccccactcaccacaaggttctcagttttatggccttggacttggagttataccatcatttcctctgatctcaggccttcatgcttggattgacttctgccactggatttcctgggtctcccacttgtagatggcatatcatgggacttcttagcctctgtaatttcatgagccaatgcctgcaataaatatcctcttatatctatctatctgtctatctatctatctatctatctatctatctatccatccatccatcttctgttggtgctatttctctggagaactctggctaatacaactatcatgcaatttgtatggtttattgaatactgatttaatcattcattcaacagatatttatcttgtgcctgctatgtgccaagtgtgttctaaactctagcagtgaacaagctaagcaaaattcctacttcgtggcactcgtgtttgagatgtaggggagacagacagtaaaccaacaacaaaataacaatttcagatatggttagtcatatgagtaacataaagcagggttggggaatagagagtggctagagtgtggagattttagatagaagatagcatttgaacagagtcctggtgatgagaaggaatcagacttgtgaaggtttgggggaagggaattttaggcagaaggaaggcaaagtgtaaggggctgaatccatggtaagcttagtggttctgcgaacagtgaacagtgcagaggggctggagcagagcaagtaagcagtagagttgttggaagaggaggaggctgaggccatgtcaaagggttctgcccccatggcaataaggttagatttttatgtaatgggatgtcttagagggtttagattgcctggttgatatttttgaaagatcagtctggttgatgagataagatttataggcaagaatgaaagtagaaagggccatttaggaagctattgtactggcccagttatcctcggcttggattaggatgggagtggtagagaggttagaaatattttggagctagaactcacaagattttctaatagatagtgtctggggattaaaggaatgaatagaatcaaaactgattcctagatttctggcttaagcaactggggaatggtggaaccattaactgagagggagaaaactagggcatgcaaaattttgtttagatttgttgagtttgagataagtattatacatccaagtgggagtttagtagacagttgaaaatataaatctagggttcaggggataggtcagaggtggagatatatgtgtaggattccttactgtatacatgtaatagttattacctaagctacatcttggctgagtgatgagatgaggtgatgcaaacaaagtatacatcattgtcctgccctactggagtatatacttgtaaaatcttatctttttaaaatgatgtacttaatgaataatagaaggaaacatagagtaggttttgaatacaatatgtttttgttcatttgttgtttaatagcaaataatccaaaatttaaatatttaaataagaattatctttcaaggtagcctcttgggagggctagccaatcagcccaacaatttcttagagctttcttggagtgattgggattcccttttagatttggtcatgccacaagaaagttagtctaccttttcataaaactatatctcattttttgttaaaaaataggacttgcttgaaagttcacctgttgttggacttgtgacaacaagaaaaataaaaaaaaaatacgtcaccgaggaatatgacttggtacccatattagtccattctcctgctgctataaggatatacatgagactgggtgattcataaaggacagatgcttaattgactcacaattgcagggctagggaggcctcaggaaacttacaatcatggcagaaggggaagcaaacatgtccttcttcacatggcagcaggaaagagaagaatgagagccaagcaaagggggaagctccttataaaaccattaaatctcatactcgtaagaactcactcactgtcatgagaatagcacaggggaaacctcccccatgattcagttacctcccactggatccctcccatggcatgtgggaattacgggaactacaattcaatgcccttccaacagtcccccaaagtcttacctcattccagcattaactcaaaagtccaagtccaaaggctcatctgagacaaggcaagtcccttctacctatgaggctgcaaaatcaaaagcaagttagttatttcctagatacaatggggctacagatgttggcaaataccccctttccaaatgggagaaattggccaagacaaaggggccactgtctccatacaagtctgaaatccaatagggcagtcattaaatcttaaagctccaaaatgatttcctttgactccatgtctcacatcgaggttacgctgatgcaagagatggactcccatggccttgaagagctctgcccctatggcttttcacggtacagcccccttcctggctgctttcatgggttggcattgagtgcctttggcttttccaggtgcacagtgcaagctgtcagtggatctaccattctagggtctggagaacagtgaccctcttttcacagctccactaggcagtgccccagtggggactgtgtgtgggggctccaaccctacatttcccttctacactgccctagcagaggttctccatgagggctccacccctgtagcaaacttctgcctggacattcaggcatttccatacaccctctgaaatgtaggcgtaggttcccaaacctcagttcttatctcctgcacatacacagggccaagaccatgtagaagctgctagggcttgggcttgcatcctctgaagcaatgactcaagctgtgcattggcccctcttagacatgactggagccgaagcagtgggaatgcaggccaccatgtcctgaacaggagggccctgggcctgatccactaaagcatttttccctcctaggcctccaggtctgtgatggaaggggctgccatgaaggtctctgacatgtcctggagatatttttcccattgtcttagtggttaacattctgctacttgttatttaggcaaatctctgcagcaggcttgaatttctccccagaaaatggggttttcttttctgtagcatcgtcagcctgcaaatttttcagacttttatgctctgcttcctcttgaatgctttgccacttagaaattttttccacctgataccctaagccattgctttcaagttcaaagttccacatatctctaaggcagtctctttgctaaagcatagcaagagtcacctttgttccagcacccaagaagtttctcatctctatctgagacaatctcatcctggacttcattgtccttatcactgtcagcattttggtcaaagccatttaacaagtctctaggaagttccaaactttcccacatctttctgtcttctgagccctttaagtctccaggaagttccaaactttcccacattttcctgtccttttctgacccttctcaatgattccaatttcttcctgttacccagttccaaaatcacttccacattttgggatatctttacagcagtgccacactctctgtggtaccaatttactatattagtctgtaataaggacatacccaggactcgataatttataatgaagaggttgaattgactcacagttccataggggtggggaggcctcaggaaacttataatcatggcagaaggggaagcaaacacgtccttcacatggcagcaggaaggagaagaatgagagtgacaaaaagggggaagctccttataaaactatcagatctcataagaacttaatcactatcatcagaatatcatgggagaaactgcccccataattcaatacctcccactggattcctcccatgacatgtggagattatgagaactataattcaagatgagttttgggtggggatacagccaaaccatgtcagtaccactgatgattttaaatggactttgtcgcttgccttggtggttcatagaagagtgtctggatatgttttgagcaataaagaaatgattggaaaaagtacacaatctcccatgtgataactttgaaggaaacactgtttatttgcttttagagctttagttttattcattcacttatccagtcatgaaaaaaatatttattatctgacatgtgcctggtggtattctaggcagtgaaaaggcagttacaagtagtgaaaagaaaaaaacaatactaattattaagtcttcatctttggcctaaaatgttagtatctcttagccttaaaaaatccagtgttttgcaaatggctcaatcaatcaatcaatcaatttattgaacaaacaaaaacattcaaatgaaggaataaaatttaactttacctttgccttcactatctgtcttcctctttgtattatatccccagaaacctcattcccacccctctgcttttgaagtctaaagtaatctgttcctgtatgctgtaacatctccttcaaacatgaaacactcttttatttttctttctcccccattttgctgctgggatatgtcaacaaatctctgggctaggacggtaatatactaattaattcatagtcaggtataaatgatttgacgctgatttactaagccctaaacttttattttaacaacaggacaggacttaaatatatctctattgatggaaatgatagcatttgcaagtagtaaaatgatatatttcttggctgagagccttctccatgtctctgaaatcacagcctatacaatctacttaaattgccaattataattcctaggaacaaaaacctttcagtttctccctgatgctactatttctttttctttttaagagatactttgcagcgctctcatgtcatgtaatatattagcaagtaatcctcatagttgtgctagaggaatgggccaaattttgccttggcctttgtttagctggatggtacctccacactgtactggggctctccatcaccatagctccttcagtcttgtgcaacatattattacaatcagcttcacttgttcccagttctttcagcatctgtagtggcagctggcgcatctcccacttcatcaggaagtgcattcaagggtatccggctagaaagttcccccagcaagcatttcttcatattgcaaaatgaagaagcaaggtttcacttgtaggtattcatatctggggtcaagtaaggtagaataaagttagggggatcttccatcatcaaagtgtcttcatcatgggtgaggccagtaaaaaatatcctcttttttttctagtagactggtattcctttgatcctggttttaatcagaaaaggaatgaacagaattatgcgattggcactgcccttgtttgttttctaaattctcaaagggaattgctctcataccatgggtttcccccaagatctacaattctggttaccaaggttcacttttgtgtggggtttcctgcattttgcctttggacacccaagtctatctttcctgcaattaacaggaaaattccattgtgccaattgtggttttgctttttcttcttgagaaaacaacctttattgcccttcacctgcctttgcgtccagtattctgtacaaatgtgtcatcgcatgacaaagagggtggcaatgaggaccagcatgtgtcaaaagtgtttgaaaactgttctagttaattagaaagagccatgctctagaaagttcaactcacgtgaaaattactggctcggagaactaacttatcttcaccattttctctctggggaagagctttgggacaaccccctccaaggtcattcatttttgtctttgtaatttcatagtatgccatgtgtctggtaatcagtattagagccagaagtgttgctagacttcaacaatctttggcagttattgagatagatgtgtctcttggagaaagattaattggagtctgaaatgtttaaggaagctaacaattattgagtgcttgttctgtgccaggcaatatgctaggaatttctgcatatgctatctcatgtcacagaatctcaatttttctgcttatgagttggaatatgggattttatttaagtcttccttttagcaattttgtctgaagtgttgcctatgtaattttacacttgaaggaaagtgtattcagtggttaaaaagagccacagaggtagcaaataatttggaattcggcttgttcattaagtacacaaataaatccaaagtacacaaacaaattcacattacagagttagagcttgtattaggccattcttacattgctataaagaaataatgagacagggtaatttacaaaaaaataagtttgattggctcacagttctgcaggctgtacaggaactgcaggctgcatagtggcatctgcttctcaggaggcttcaagaagcttccaatcatggcacatggtgaaagcaggaacaagagaaagagaggagaggtgttacacacttttaaatgacccagatatcatgagaactcacccactatcgtgaggacaataccaaggggatgttactaaaccattcataagaaatccacccctatgagccaatcacctcccagcaagccctacctccaatactggggattacatttgaatataaggtttgggtggggacaacatccaaactcttattagggctagtcaacaccactagagtcaagtgagctcacaggacaattttgtgaatttggtactaaagcagtcattagaactatttatcaatatttccagactttctcttcctgcagtgttctcaagccatataatgtattagcaagtgatcctcatattagaccacaattccccaaatccttgaaattaggtgtggccatgtaacttgctttggccaatgaaatgtgagcagaattgatgtacgtctcttcaggtagaagcctttaggttcagcggaggagacatcttcccttcctccagccatggtgaccaacaacattccagaggatgcaggtctgcaagcctgagtcctgagtgatgacaatgtgaagacaaactcactaccaacccaaagtaccatgagcgagaaataaataaacctctgttataagtcatagagatttggggattgtttgttaatgtagcacaaactagattgtgctaactcatacaggaaccatccagccagaaagccaaaaagtccttcctaaatgtatttgctttcattaccggagaggtttaaccagaggtttgaattgaccaaattcttgtgatgattatacagtttggtagttaagaggtctctgcagtcaggctgtcaccataggtacatcagccctgctgctttctacctgtgaaaacttgaatgtgttacttgatccatctgggtctcaatttcctcatctgaaaaataggtataatagtaatactgacctcctagagctattgtaaggtgaaataagataatgtacagaaagcacatgtcagtttgtaagttttctgtgattaatgttagctgtcattccattatccagtaccagcactcactttatacaagtctatctttttgcagtttaatggtttggataactgatctttcaagtccctcccagctctgaaactatgagtccatgaaatatcttgctttttggtacctaaatttccttagagtagctttaaattgtagtttgagttttgtggcgcatgtgggaactgatgttagcagagtttctctggcttaagaaatccatctacaaaaaatcagttttctctgcctcaattatctctcgcttgtcctactacatcattccttgaagtttttccagaattttttgactttgtagttgcttgcttctttttcattctgaaatacattttttccttttggcttttgacactgaacaacataaattttccttttaatggacttgcctatgtgtatggtaaataaaagcaggaatatgtgaggaacaatttcccaatagattatggaggtttttggtggcgttttaaggttttatgacactgaagagaggaaaggagaaaaacttgttcttagaaacatatcaactttaacattacaccgaaacatttcatacacacatatttgcaggaatattctgatttgctgtgtatgttttccagtgttctctctaggaaagaatgcactaagatctgaaaaaagtagttatgattggttaaaaatgttttgttaaaatagaaaaaagtgtagccttaagtattttgctggcatagtaggaaccaataactattgctttgaaatgcagctgtgcattgtgaagctgtgaacaagacttttcaaggaaaatagcattgtctaggatggaggaagaggccaggacctatagttgtgtcagatgtgagcaggtagtgccaaagttatttgtagaaaagatcatgatggttgagttcctgggacaataacctgagagatcagggaacacgaaaaggtagagtcaggaaaatcaagcttggggaatggggatggggtatgaaagggagaaaaactgaggcaggaagagggatgagatcaaagaggatacagaataaatgcagagctacagataaagccctcaggaccaaaagtcagagatcccagttgtttaatccagagacaggaaaaaggacatcctctaaaaagacctaggttatgggctgaagggagaagatagataacaggaaagaaccaggtttctcttgggacccagagagcaagaccagccctaacttccccccttcctttctctgttctaacacttctcataaaacaatagtttaacttgatgctagaatgtggagatgaaacaaactctctgaaaagagagagaacctcagagtccccaagccaggagactgacagagaagccctgacagaaagactagcataatgatgggaattgcagtgacaggccatggccggaagggattgtctcatgctttacaagtattgttttatagaataagtgagtgtgtgcaataggaagcattgaacttgagctgggcttaccagtagcatggccttccactccacttctggaaagctaacaccctaaaattccctcccaggtgggaaagtgccttgcctagagttcctgcccaacaaataatgtatgagagagaccactccagaggaaggtagtcagatgtgagctggggtagggagaaggggcaggagaggtatattgtgctggaaagcaagtgggaagaagagcaatttcctcttttccctcttccaaccctcagataaggtgaatcatagggaacactgattggtaaatccatcaacctaagtaggttcctttcaccatgtaatggcattgtgtaatttgctgcaatatttccattgtctaggctatactagagggtcactgataatccaaagcaaataaaagaagagtttgggaaataattgatgttagacaaggctccagaatcctatgacaatgcaatgtcttgaatgcctgcctatttttcccttgtaatctttatgaatcccaatggaatcagatctaattcagccttaggatactttaatttgtccaatttgggttattagaccctaagaattccttgacttacctcctttctccattctttggagggagggattcctaaatgttttctagaaggatagtcttggatgctgttacctcaaacttgggtccgctacttgtcttggttttgttttgtgctgcaataacagaatagcacagactagatcccttataatgaatagaaatttatttggcttacatttctggaggctgagaagtccaagactgagaggccacacctggtgagggccttcttgctgtgttataaaatggcaggaagcatcacacaggtgggagagagagagagaaagagagaggaagaagaaggaagaaggaagaagaagcagaaacagaagaagaaaagaagaagcagaagaagaagaagaagaggaggaggaggaggacggagcagaagaaaacgacgaaggaaggaaggagaagaaggagaagaaaggagaggagagggctaatttttttaaataaaaaattagcaacctctaatataacctctattctcatgaatggattaatgctgccatcgcagtagcattaatccattcatgagagtagagccctcaagacctaattacctcttaaaagtctcatctcttaacactgttgcattgggaattaagtttctaacatataaacttctggggacccattcaaactgtattaccactcattagctgtatgtccttaggaaattgccttaatcacctaaatttcagtttcttcatctgtaaatggggtaccacctccttcttatagagaagttgtataaactcatgacccagtagatttgagaagtactaaggttacatatggcacccttctctcaggatgctgagtgcctagtatgtcttctttgcccaaataatcctaggggatctttccccagaagaaagcaagccaattttgtgtgaaggtctcaaggacttggctccagagacaaagtttctcctaaataaccaaactagtatgtgcaatgaattgtccattgtttctttcatctcccagcttcaaatgttttcttgaaagtctggctgcctgacagcttaagctgctagcctcttcattagtccaacagaggactgggtatgagaattggtgaaaatgggcatgaccagtacacatgttttaggtgaatatgatggttaatactgagtgtcaacttgattggattgaaggatgcagagttttgttcctaggtgtgtctgtgagggtgctgccaaaggagattaacatttgatcagtggactgggaaaggcagacccacccttaatctgagtgggcacaatctaatcagctgccagtctggccagaataaaaagcaggcagaagaacgtgaaaagattagaatggcttagcctcccagcctacatctttctcccatgctggatgctgcctgccttcgaactttggtctcaaagttcttcagctttgggacttggactggcttccttgctcctcaacttgcacatggcctgttgtgggaccttgtgattgtgtaagttaatactacttaataaactcccctctgtatatatgtctatcctattacttctgtccctctagagaacgctgactaatatagcaagttataccttgctgaggtcaacttaaaggaaagaagtctcaccaaaggctagggatgatataaaataggagacattcactgagtgtagattcttaggacccacaagtacaaaaagatgacacagttaggttcttccatgaccttcaatctcatcacccctgaacctagtgtggtcatggtggcatcagtgttcattgctgctttagtcacaggttatgaaataatcactagatatcacacatgtgtgactccgcaatgatgacttgtgttccagccatgagacctgagacagagtacgtccagcctgaccatggcaaccccaggcttgcagtattcgtgctgaagcctgctctgaatcagatagttgagttcaatagtgtttatgggcaacatagagagactcctgtgccttctgctggaccctttggagagctaatgccatctctgttgcagggagctatgtttcccaggttccattaccaactggttttcaggtaggtttggctaatgagaggcactgcagagcagatgaaccagagcatttctcctcctttttgctttaaatgaggcttccagcagtggctacttttgtttgtttatgaaattttagctcttattggttaaccccattctttgtgtttccagctcctatggagtgatccctgccatggttttaactctcaccaaatggctttagtttctggttctggtaatgctgtattctctctttgtccttccagctctagaggtggtgaccacttttggctgtttagctctttcatcatttatgtaaccaattccctgtattaaattctttctgcttaaaatgcctcagttggtttctgtttttctgactagactttcactgttacatgtttctcagtcattgctacttcatcttcattttggattgaagtctcccatgcaagttttgcagtctcccaagccacaaactgggaaaccaggtaatgattccttcagtccttaggtttctctgaacataccctaggtttctttcactgaactctttgggcttttgaccctatgaaggagacagggtgctttttatttccaagtgacctaccttatatcaacaccagtcaagattcctgagattgttctcccatccaatggttaatttcttttagaatagaaaagctgctcttagtttatcactcattttctcctttcctttgttttatgttataaactctatgttatctctctagactttactgttggagaaaaaagccttccagtaatacaaataaacacaaacacaaagacaaaacagggatggatgcagaacttcaaggatcacatagatctattgaagtgatgagtggcagcaacagcattacttcaaatttcaagggacagcaatggctgcagggcaattagcaattcccagtcatgggagtgtggatcatcacacccacttagtagtggtaacagtggtgtctttatcaactagggttttgtagcatgattttgaacatgatcccttaatgtatagcatcgaagcctgatttgctgactttcctagagattttttgagctactcaatataattttttggtagatcattacaaatttgtttctgtaattaaaaatagttacaaaattgaaattctgaacaatgttttctgattacaaaaccatacattccgacgtgtccaggtgtactttaatctgatgtgccctcataatgaatctacaatatttgagttccatgtaacattgtggttccccacaattattaggtgattaatgtaatctaccctttgaagggctttgtcctcagctttgtcaatggtgctcagtggacttgttagtcaagtggccatggtggcagaaagtgacatcctagcttaactatgtgagcttcccttcaccaagggtttcttgacatcatcaatttgccagctctggtgacaaacactgacactgccatctgataccattccaaggatactggtcagtcacatggtggctggtgagccatatttaactccttcttttggggaggaggaagcactataccgtaactaaaataagcactatttggatttggatttactttcctttcctcccccaccttgcttctgccaaagctatgatttgtagataatctagattccttgttcactatcacagtatcccacccaatgttgcttctcaccaagaaacttttttgggagaggaagccaacaggctgacacacatgaaaattcatgttcttataaactctctgtcctggaagcaactggctttacaaaacagtggaatgactgaggtaagactcagttatgatgccaacttgaagttgaaatcttgaaaggttggggtaccattttggaggtgagacgtgttttcctgtgtttgatacatgatgaaggctcttgctgaaaagataaatccagggaccaaggtaaggaaatgggaatgccatttctcatgatcacattaatattacacctgtgactctggacaataaatgtataggattttagtagttggaggagaaatgctttaaccacaggaagcaacagatactgccatcctgctatttcaggctccttttactacttggcagggaaaatatgggtcatagtattggctggggtgactgatcctgttagcaaagatttctgatacatattttgatacacagtgggatcagagaggaatataaatgaatctaaaggaaccttttaggattcccctgtctggtggtaagttaagggaagatatagcaattctatataggcaggaaccactgaaaactcagatccctcaggagtcaagttttgggtcacttcacaatagaaacagtggccatttgaagagaaaataaaaggaacgtagatgagtagttgagggtggaaataataaattttcactatggtctttttaccagggaagccatgctttgagagaagacatgaaaagagcaggacatatttttatttaaccagttctgttactgagcacataaaatcataaagcaaaccctccaaagattttcttctgcaaccagaataaaatccaaacttatttgaatttattgaggcttacaaaatactatgtaaattggcacttgcctacctctctcactctatctcattccacttatccaattgcctgccatgtttaagcctatgggtaaagctcatttcagcctcaaggatttgctctagctgttccctccacctggaatgtttcccccaacatatccagatggcttaatccctcacttcatttggctctctgctcaaatgctcttgttagtgaaaccttcccttcgcaccctatataaacagcactaccccatgttctctctcttccccttatccatgatttagtttccatgttagaactggtaactgtattacatattagacatgtatgtgtttcttatctgtccctctccagtgggatataatctccacgaagagagagactttttgttggttgttgaatcctcagagcctagaactgtagagttgctcaagtatttgttgaatacatgatttaattaatttatgacagaggaaagatttgttaacagattctagaaagccttggaaatcagactgagatgtttggaaccttaacattttgaataaattagtaaggagtaaaatagaagctattttagagagtttttgaaattgctcagggacctttgctgtcttccaagttctttggtcattcagaattgtgccaatgacttccgctgttctggggatgcttttatgttgatccctattcttcaataagtgcccccaaccctccctgctggttacccttgtttccttttccagctagcaacagacctctctccctctttcccattttttgtttaacattttcttctctaagtggtatattttgattattcagcagctgcttcatgcagatggtgggaaggggccttgtatatttgttattgcccagtatcctgatgaatatgccatttgcttctgtgtatcagcttttgaaggctattctaaagcttctgcttcgtactttcattatcagaatgtacaggctgctgctcagatggctggttctagtgaaatagatatagtatggagttagctctttactatccagcagggcagttgaggtggccttctttttccacttgttctgtccaaatcattctgcttcaaatcattgctgcttcaaggtttgtctggaaactcctgcttttttttcaggccttgctggtcttctccttgagctcctttcacatgtatagcttatatctcacatctaagcccttaattatatgctgttacacattattccttcagggcttcagacactcttctgccttcatgtagttataagttcacacattcccatcatcaacacatttcttcatcagtaatcatcagtattagagagcttgacatgccccactccattctatttgaaaacctctgcctattatttcatttgtctgaattatcttcctcaattagattgtaaattcttgcatccttgattgtatctcatgtttctatagtattcttctagttatggtttgatgcctagaatagtactgggcacataatggatgcttttttctacaagaattaattgatattttttattgagtcctaattgattttttttcactgaaatatagtcaccatgtgtatatatatttgatgtttttacctccattccaaactttcaggacagctgtgctagttctaatctgttcttagattgatcctatgactatgcaatgtgactacaaggaaaatccagttttggttctgtaagaattaactccattcctaagatagcaaagaccaggcctaccttccctgccaccactcaggcctcttccagcctgacccccaacatccaagaaagcaggagtgcagctgaagacagggtacaaccatgtgagcaatcaattgattgataattaatgaatcaatcaatcatgcctatatcataaaaccccaataaaaactctggacactgagctgagttccccaagatggtaatactctgtattgttaaacatcaatgctggaaagataatttgtactgaggacaatagaagcttctcatttggaatcctaaactctattctgtgtgtcttttcttttcgctggtcctaatccttttctgtaataaatcgtagctgtgagtataatagttttcagtgagttctatgaatctttctaaataattatcaaatctgaggtagtttagggacttccccaaactcgcagttagtgtcaaaacttagggcagtctgggagattgttcccactttggctaactccaggtaatgaaacacctacaacccccccgcctttcctgggtaatgacaacttatccagttgactggaatgacaactttacactgttgtagcttgagagagacaggactggattttctttgtgttctagtttattttctcacccactccgttagtgctggcttcatttctcagcttccagaccctctctgcataatatgcctcatcttgtactcatccctgcctcagctccaggcttcatggaggtaggatagataggaagacctgcaatgcagctggtgcagctcactattaaggctctctaaaagtcagaagtggcctcctgggaaccaggaatgacccttggccactgtcccacaaacttacaacttccctcacttccaatcacacctgggacttagtaccaccaggacagatcattaggtgcctgaggatgctgggtttcctctgcattaagaaccttttctgcctcttcccagtacttcctgatgttggcttagccccatgtattagtccattctcatgctgttaataaagacatacccaggactgggtaatttataaaggaaaaatgtttaattgactcacagttcagcatgtctgggaaggtcttaggaaatgtacaatcatagtggaaggagaagcaaacacatcctttttcacatggtggtaacaagaagaagtgcccaacaaaaagggggaaaatccccttataaaattatcagatctcatgagaactcactcactatcacgagaacagcttgggggtaactgcccctatgattcaattacctcctactgggtccctcctatgacacatggggattatgggaactcaattcaagatgaggacattcaagatgaggatatgggaactcaattcaagatggggacacaaccaaaccctattattccaccctggcccctaccaaatctcatggcttcacatttcaaaacacaatcatgcccttccaacagtcccccaaagtcttacctcattccagcattaactcaaaagtccaagtccaaagtctcatctgagacaaggcaagttccttccacctgtgagcccgtaaaatcaaaaacaagttagttacttctcagatacagtgggggtacaggcattggctaaatacacccattccaaatgggagaaattggccagaaaaaaggggctacaggccccatgcaagtctgaaatccaatagggcagtcattaaatcttaaagttccaaaacgatatcctttgactccatgtctcacatccagggcatgctgttgcacaggtgggctcccacagccttgggcagctctgcctctgtggctttgcagggtatagcccccctccctgctgccttcacagctggcattgagtgtctgttgcttttctaggtgcatggtgcaagctgttggtggatctacaattttggggtctggaggatggtggctgtcttttcacagctccactaggcagtgccccattggggactctgtgttggggctctgacctcacatttcccttctgcctgccctagcagaggttctccctgagggctctgcccctgcagcaaacttctgcctggacatgcaggtatttccatacatcctcagaaatctaggcagagatttccaaacctcaattcttgacttctgtgcacctgcaggctcaacaccatatggaagctgccaaggcttggagcttgcactttatgaagccatgatccaagctgtaccttggtcccttttagccatggctggagctgaagctgctgtgacacaggacaccatgtcccaaggctgcacagaggaggggggccctgagcctggcccatgaaactatttttccctcctaggcttccaggcctgtgaagggaggggcctttgcaaaggtcttggacataccctggagacattttccccgttatcttggtgattaacgttctgcaccttgttacttaggcaaatttctccagcaggcttgaatttctccccagaaaatgggtttttcttttctatcgtattgtcagcctgcaaattttccaaacttttatgctgtgctttctctcgaatgttttgccacttagaaatttcttctgccagataccctaagccctctctttcaagttcaaagtttcacagatgtctagggcagtggcaaaatgctgccagtctctttgctaaagcataagaacagttacctttgctgtagttcccaagaattttctcatctccatctgagatcaccctggactttgttgtccatatcactatcagcattttggtcaaagccattcaacaagcctccaggaagtttcagactttcccacatcttcctgttttcttagccctccaagtttctaggaagttccaaactttcctacattttttctgtctttttctgagccttccgaatagtttcaatctttgcctgttacccagttctaaaatcacttccacatttttgggtatctttacagcagcactccactctctgtggtaccaatttactgtattagtttgttctcatgctgctaataaagacatacccagaactgggtaatttataaaggaaagaggtttaattgactcccaattcaacatggctgaggaggcctcaagaaatttataatcatggtggaagggaaagcaaacacatccttcttcacatggtggtggcaaggagaagttcccagcaaaaagggggaaaagcccctaataaaaccatcagatcttgtgagaactcacttactatcatgagaacagcatgagggtaactgctcccatgattcaattacctcctaccatagtccctcccacgacatgtggggattatgggagctacaattcaagatgagatttgggtggggaccatggagtccccacccaagtgggatcatgggatgatatggtttggctgtgtccccacccagatctcatcttgaattgtagctctcataaactccatgtgttatgggagggacccagtgggaggtaattgaatcatggggacgggtctttcccatactgttcttgtaataatgaataagtctcatgagatctggtggttttataaaggggaattcccctgcacacactctctcttgcctgccaccacataaggtgtgacttagctcctcattcatcttcagccatgatttgaggcctccctagccatgtggaaaggtaaatcaattaactttccatgataaattaccccatctcgtgtatgtctttattagcagcatgagaacagactaatacacaccatgttttacaaactggactgatgataagaatcacctggggctgttgttaaatgttcagattcgcagcatgtctaatggagattttgattgtaggtctgggttttggctcaggagtctgttttattttaatttaaatattaagtgccccagttattcttataatcatctactacatccctgtgccttaagttttgcttcatgtccattttgaactttaaattaccatcttacatatttcccctgtccttgctggtgttagaaaacaaacctgaatctgttctgcataccctctgtgttggaggagtcatgccctagtcctcatcctggggcgggcagttctcttaccctgcctcattatgaccaaccctcctttctggcactaggctctttcctgtgccccattccagtgtctgcagtcttgccacttgtagatggacatctgatatggtgatcaactccacaaacaacttcatttaattcaataaacatttactgacttgagttatgtcccaggcactgtgctaggtgctggcaagatgaaaaaaggaaagaacagtttaaagggtgtgacagacacataaagaaacagccataatattgtgtgataaatgctttagcagaagcatgtacaaagtgctatggaaactcagacgagagtgtgattaattcctcctgggaagggtcaggaaaagtcacagagaagagtttacatttggaaggtaatcaaaagttctctcagaggtcagggagaggggagggccttccaagcagagagcaaagccgaaacaaatccaaggagagtgagagtgcttgatttactccggcaacttggactgagtcacccagtgggccaagagcagtgttttttccaagtgtagtcctcatgccatcttcatccataattccttgggtagcctattagaaatacacatttcaagatcttaacctcatacttactgatttgtaatcttggggtgcagcctgacaacgtttattcataactaaccccctcagtgattctttaaactgaaaataaagcagttgttctctactttggtacattataatcatcagggagctttagaaaatactgaggcctgatcttatcctccaaggttcccatttaagaggtttgggatatagcctgggcatctccatttttaaagctcccccagtgattttaatgcatggaaccactgcacccaatttgaggaccacagaacgagagcatcagattcaagaaggcaaagcaggcacttggagacctgctacaaattataatggagatgtaaaaagttcatgcagagttttccatgccatgttggggagtttggtttcaattttgtagatggtgaagagacaatgcaagaggtggctcctacgggctcatatttctgtttaggcctcaataaatggtggtgttagaaaacaagattgaatctggtttgtacacccatggtgttgagggaagggatgctttactaccactccatgaagtgggctcaactatgccctcagagtaactgttcgtctttcagataaaggctctgaatactcctgttgctttcttaagagacacagtgggcacctatcctgtactcactgttgaaaaatcctcaactgtatcccacgtaaattctgagccgtgcaaagcttcatgaagggaagacctaagggagattggtggtgggcattatatattcacatggtctccattaggcccagcagttacaggtattgacttcaaccttgaagttcaggaatagaagaaaatgtgttgtgtggattattgtgcctacaaggcacagagaagttttgggatagattgcaatggcatagaagaaggagaggtgagaggtgagtggggaaagtatagttataagccaatcaccactccacagtgaggtgttgggacttttgtggaccaccttgattaagatagaaccagatatgttgtgggtacagttgtgaaggaaaatgaagggaggtcagaagtctaatgctggagccacctgaagaccctgactagcagctagtcatgcagacctcaatgaagtctctccctctcattgtctcttcaattttctcccctttccctcttctatcttctcagtcttttcccctcttctttaaccctctgcatcctcactgcccatagtgctcccagaaacaacaataaagcctaccagactccaacatttcttaatgggcccatgagttacagcctttgttgaaacttattgctaagaagaatgttggtgattctttggtacaacctcttcaatttgtgaatggagaaatggaggtccagaaaggagacatgattgtccaggggaaaaaaaaaaggtcatagagctagttagcggtagaattcaaacagatccatgtcttctgactttctctattagcctgcatctactgtgctatgctccggtcacaatggggaattctcatactttgcatgctttgaggggtaaattgtacactcttcacgtttggttcctacaaccactttgtaagaaggctatagccattagttcatcatgtgtgctaagttcaaagagaaggaatgtgctttgcttaagaatgcgagtttcaccagaaaggaagtagaaatttataaaataggaaagttcaggtttacataattttaggccatatgagtagaatttttatatagtagattctaaaattactgttttccattatcatgatgtagagtcccagaaccattaccctaggacaaggaaagactttgtctgatggttgtgtgtttgagtgcaggaaaagacaggatgtggttacataactttggtgttttgaccttggtcttgcttcattttgaaggcttctaaccttgtttgctggtgccctcatgagtatgtggaagatgagatcgttgcttctctcacacaacagtgcaatgagaacattatctgtgacattatggagtctgggaatccagtgtagcatctgagtcagtcctagcccaatagcaggcactcatgggttattttttgagttgagttgagatgaggcctgcaggtctgcagcaaattactattgatgccatcttgagcaagtcgttttctttctccaaactcactcttctctcttacaaaataacagacaagaacaagacaacttctgacattccttcccactcagagattggcatcccttttttaaaaaatcccagaaatttggacttaggagaccctttgaaggtcaattagcccaacccacagcttgttcaaggcagagccagattattcaaagaagtagagatttggcaacttcatggcttgtataatagtggaaatcagccaaaaagaataattgaggttaaaaagttatttgagggccagaattactctctttggtcaatatccatcacattaatgaggaatagtgaaatctctattttgctttggttttctcctttgctctctactgatatataacatatatacatcagtaaaatgcacaagtcttaagtgtacagtgtgaggaatttttacatatgtatccacccatgtaactatctcacaaatcaagatacagaacattttgacaactggagaaagcttcctcatgccttcactaccctctctcaagggatagatctaatttctatcactgtaggtttgttttgtctagttttgaactttatatgaatggaaccacagcgtatataacccattgtgtctgacttttcactcaaccttgtgtctaagattcatccatattgttgcatatgtcaggagtctttttgttgttgttgcaatgtgtgaattgtaagactaccacaacttaagaattcatcagtgcagattattagctacagacgaggagaaaaagttagaagatttgtctcctaatcttattattaagtagctacatgaacctctctctgggcccattttcctcaactgtgagtgaagaggtcaggctaaagaatcactagcaatttttctaattctaaaggccaaagaatgtatgtgaatcacagaccaaacaagcatctggaagatatgaaaaaaatcacatatctgacaaagaactcatcctagaatatgtaagtgactcctacaaatcaataagcaaagaagaaaagtcaattaaaaatgggaaacatgcgtgtgtgcatgtgtgtgtggtatttgctgctattgttgttatagtaaagaaaaaaattgttcagtgggaaaccttagggtcatcatgatgaccatgtaataaatattttcaaatatgcagaaatgttgggccatccacatgatgcagaagctgatttttgaaaaaggatccctttgtattattttctgtaagggaggcaccatgtttaattttagtgaatgcatgaaatgcatgcaaaagggcttcataaactgtaaagctctctgcaaatgaaaagcattattattattccagatacaatataagtgcagctgacatcaaccaccatttatcccagttgcaggtgtaacaaccaacaagggtattgtcctttgttcctttgccacagctgtgagagagcatctgaatccaatacataaataacagctgtgattttaattgagacttttgagtggataagcaaggtgtacactgaacgcatagcaacagataggttttcatttgggcagccacattattatttcctcagactttgaaaagggaaagttttaacagccctcttggaagtgacccttgtttttccccccacctgttcgcagttactgtcacagaatgcgtcatcactctcccacgcgcacagtgggaaaacaagtttgccatccagagcaaagggagtttttatgctgtgtcagggatacaagagtctgtgtatggttcattgtccatttcccaattaggctccctccctaggcgttggagcttcctgcccagagagcctgcctggactccttatcatttcagcagaaataagtcacatgagaagccactgcaaatcagatttttgccagaatgcttgtggtctctgccttgccctttttttcccccaagattttgcaactctgttcttgtcttaggagggtgagaaattatcccatcaatgtaatcaacccagattggtcaaccaaagggaatttgcttgttgaatcacatttgctgctagtatgttcttggacaagggtatctccatgactctgtcccttgactggggtgtctaactattgggtattctctttcttgtactgtgcatagatatgtttcagactttgtatttgccccttaaagctgcccttgtgatagatttagcagctctgtagtaatacacactgaaaactaatctaaacactatatagttgtagagtggaaagagtttcaaagcccagcaaatctgaattggaatcaaaatttatcactatacctgggtgataggcctcagctgccttatctgtaaaatggggataaaaatacctccctagctctgaagatcattgtaaggtcaagagaggcaatgcatgtacacttcccagagagggtctggcccatagtaattgcctcataattagtgagtgagatgattgttccataaactgtacagctggggaagatcccccaatgcagacacatggctagcccaagtttaacagcaacttaatggcagatgtaggagaaaagttaagatccagagcttctttctactacatctaagaattgtttcctcaggtttggggaggagacagcaaagctaaacacttcaaggtaaattatgatgctttgatgatttcttaagctgagtggtctatagttcactggcatagaaggaaggtttttgttttagaaatatcatctctgcttatgtttacagcatatctttcctgttcagccagaggcatccatattgctttgaggagagttagcattgttagattaggacagcaagaagaaagaaactaataaaatagattcttgcaccccacaatagaaacatggattcgaatgctaaagtgttgacttgcaagagccaggttcttaatgagagaggaagaagcttgagaatccaaagagaaggtctttaaggaagcaagttgtccatgacataaagttaggttacaaagagaacaggggaagaacgaggtcaccccaccccctctctgggctagtgggtagttgatagtgacctgattggaggagggagaaaagtggtgggctgagggttgggatgaagatgctagaggggaccatggggaggagagcctgcaagtataagtggacagtgtaccttgctttgccatttaggggagggccatgttagctgtctctctcagcctttgctgttgagaaccttctgtaaacatatgcttacataccaacccatagattttcagcagaagtgataccccacaatgtccccagattttgctaaggtccatatgagttatctatttggatatcctttttcagtgaccacggtcactaataaataccgtgaaacataggcatgatttccagaagatgcttggagatgtggagcataggccctcagcatttgtactggatgcagcaaccatcctcatgccctaggtttaattttaggagttaatacagcatggcaattaagaatgtggtctctggcatcagactgactgccttagatcctggttctctcctcttattagctgggaaattttgaggaagtttataaaacccttagattcttagcttccttgtctcctcaatcacagtatcataatttctgcaacatagtttgcagtgactaaataaattaatacacaggaaggacttagttagaacaatgcctgctacatagtatagtttaataattgcctgttgtagttgttcttactgcctgtgcccagccaaatttgtgtgtgtgtgtgtgtgtgtgtgtgtgtgtatgatacagagctaacaatctgacagcttttttttttttttgcaataacaaaaagagaagttatttatttactatttcacctttctggggttgttaatttgattttctactcattcatttgtatatgcttttaagaaatatttatggagccccttctatgtgcctatcaggcactgggctgactgctggggataaaatggcatgtaagataggcatatccctgccctcatgtagtttacaactacaactagtctattccaataactgttttccctttatctgattttggggcctgggccaatctcctgagcacatttcctagtgctggcaattggggtcctgcagcaggccataaaatgcatggtatatgggtttaataatgtcaggggaaattttcagttaatcccttggactgtgggtacacccaggattcaaaggccagaccaaaacggcacgaagagaaacagagaactggtaattatctggtgaatttgggtcatgtggaaagccaaactaaattactttcgccaaggaaaaaatgatttttttttttctcttcaaatgaattcgttttggtgagattttcctagggtcttcccttccttgctttgcattattcaaccaggtatttcctagaaaccagcacagcgtgggtaaaatataaagacaaggacttcgagggaaatgaaaactgcttgtccatggggtatttggggagccctggtcttattcccgatatataacatataaggaaaattgtactaagttgacagtgctaccataaatccagtcagctcgtgggtgctctaattttgaactaaatctaacagcttctgtttatttgtgaaacagatgttttaagttaaacgtttcttatgtctttttgttcagaattatatcatattataattttgcatttctaaggcaaaagcaaatgaagggaacatgcttaatttttaggatatgagtaatttattatacttttaatagaggatttcaatgtattccccatccaggaaatggtaatggaaattgcctacttcaacatgtaatctataagatcttgttaaatagtgtaatgagaatttgtcactttgtcacctagctgaccttttacaaccctgaaactcaaagtgaagtgacacctccctcaattcagatgaaatgcctgcatattttactgtgttttcaccaagaaatcccttcagccaaaatttcagctagtccaagtcaatttttaagcaaagtgcataaccagaaattggcacaaacatttgtgtatcatcctttccatattcaaaagctgtctgagactcatttgattaagcataaaaataactctgtgaatgtcattagaaaggcagcgaacattctatgtctggtcccttgaatttgtattctggggatgcattattaagtcactgctaagtcgtttctcttgtaagaacctgatcatgctctctagagtctgaaaaaattattttcattttgagtttagaaggcttagtttttctatttccgttcaacagaaaggaaacagctggtaagttagggaaggccagtgtatttggctactgtaatctccactgccttccctggttaacagaatatctttattccaaccagggctccctccctgccaaatctccttattaaactaaattgtgattagaaaagaataaatgacattttatttcatatgtggctcctttcaaacttccatactcctctttaagttttcctcttacaaaacttttccttggccttgggcatttctcctccttggcagaccttcaacattgcaaagttcctgacaagtcttgtagactactactgaatgaagcacctcctcattcgttcctgtgggatcaactgttatccatgcacttattcattccataaacattaattcttacacacaaaatggctatgtgtattctagactcaagtggtcgtctctgaggatcatgtattggttcaaaaatgggatgctctttctctttctcagatttgtttttctgttaggtgcagttgcttttttccaaagtcaaggaagtccaaaatgcaggttgcatattggtggaatgggttccaaatgtggacagatgttgacagaagaagtgtcagttggggagtttattacaaatggatatttagggtcccagtttctagaagttctgagccagttgggtggggctcagagttttcttatgtgcagctatatgttgtcccactgatgtgtagggctagagtgatagcagtggatgtggagaaagaggatggattgaaaaacgacctaggaggcagagtgtgcagggcttgatggccacagataggagtgaggccacaggtaggagtgagaacagaggagttgaagataacctgtgtatacatatttgttcttagttcatctgcaaaaacaaaaagaatactacttatttcagcaatggaaaattacccaggattgtttcaacaaggcaacactaaaaatattccccaaacaattctttggtatcaaaaaataaataccagatggagtatacactttttgattgactgcaaggaatttattgaaggttgaaagaaagtaaaacttaatgttgcatttagcaaagactttgacttttctcctttgtacattcaacctggggccatagtgaaagtcatattggggataaaatgtcactatatatttgtaattcagaacttcaaaaggaccttctctgttgatgtagttttctactaaagttgtcttgcctgccacaatgagcatttttttttttttttttttctgagacagggtcccactccattggccaggtgcagtggtgtcataatggctcactgcagccttgacttctagggctcaatagatcctcctacctcaacctcccaagaagcttggagcacaggtatgtgctgccacatcaggctaattttttgtaatttttttttttaagagacagagtttcaccatgttgcctgggctggtctcaaactcctgggctcaagcgatccacccacctctacctctcaaagtctggaattccaggcatgagccatcatgcctgccccacaatgaacattttataccttttacgctcacttcaaactttcaccctccagcccacttcttcaccattatcctcactttgagtgatggacttgaactctacctcatggagaagatagacattatcacataggcacaccctactttttctgctaagtctataaacctacttgcagctgcactttttttttcttcttctcgccgcaccattgtcatcaaggaagtaacatttctcctgcaagattttggattttatgccttctcatcttctcaaggacttcattcttcaagttttctcttttctctcttttttacctttagcctctaactttatactggatcatttttttaaatttccataggttttttggggaacaagtggcatttggttacatgagtaagttctttggtggtgatttgtgagattttggtgcacccatcacctgagcagtacacactgaacccaatttgtagtcttttatccctcacccccttcccaccctttccccctgagtccccaaagtccattgtgtcattcttatgcctttccatcctcatagcttagctcccacttatgagtgagaacatacaatgtttggttttccattcctgaattatttcacttagaataatagtctccaatcctatccaggttgttgtgaatgctattaatgcattccttatttatggctgagtagcattctatcatttacatttacatatatacacacatatatataatacatataatacacacacacatatatatatctcacagtttctttatctactcgattgatgagcatttgggttggttccacatgtttgcaattgcaaattgtgctgctataaacatacatgtgccagtatcttttttgtacaatgacttctttccctctggatagttacccagtagtgggattgctggatcaaatggtaagttctacttttcattcttcaaataatctccacagtgttttccatagtggttgtactagtttacattcccacaagcagtttagaagtgttcccttttcactgcatccaagacaacatctattattttttgatattttgattatggttattcttgaaggagtaaggtggtaacacattgtggttttgatttgcatttccctgatcattagtgatattgagcattttttcatgtttgttggccatttctataacttttttcgaagatttatagattgtgattttctcctactctgtgggttgtctgtttactctactgactgttccttttgccatgtgaaagctctttagtttaattaagtccaagctatttatctttgtttttattgcatttgcttttgggttcttggtcattaaatccttgcctaagccaatgtctagaggggtttttctgatgttatcttctaaaatttttatagtttcaggtcttacatttaagtctttgatccatcttgagttgatttttgtataaggtgagagatgaggatccagtttcattctcctacctgtggcttgccaattatctcaacaccatttgttgaataggatgtcttttccccactttatgtttttgtttgctttgtctaagatcagttcgctgtaagtatttgagtttattctgggttctctattctattccatcggtctaggtgcctatttttataccagtaccatgctgttttggtgactacagccttatagtatagtttgaaatcaggtaatttgatgcctccagatttgttctttttgcttagtcttgcattggctatgtgggctctttttgtttccatatgaattttaggatttttttttgtagttctgtgaagaatgatggtggtattttgatgggaattgcattgaatttgcagattcctcttggcagtatggtcattttcacaatattgatgctacccatccatgaacatgggatttgttcagtttgtttgtgtcttctatgatttctttcagcagtgttttatagttttccttgtagagatcttttacctccttggttaggtatattcttaagtattttattttatttttgcagctattgtagaaggggctgagttcttgatttgattctcagcttggtcactgttggtgtgtagaagagctactgatttgtgcatattaatttcacatccagaagctttgctgaattcttttatcagttctgggagctttctggcagagtctttagggttttctaggtaaacaatcatatcatcagcaaacagcaacagtttgacttcctctttaccaatttggatgcctttatttctttatcttgtctgattgctctagctaggacttccagtactatgttgaagaagagtggtgagagtgagcatccttgtcttgttccagttctcagagggaatgctttcaacttttccctattcattattatgttggttgtgggtttgtcattttactttgtcatttctgttagcatcaataccttttctagcaccttccattaaaaaaaatctcttaattccacagccctgtttctctgattcctcctggtcaacattctttttaaaagtcttctacacatttttttcttcatttccacacctctcactcattctttacttcagcctcaatgtgatgtttgttctgattcaccaaagctactcacgaaaagcacaaatatcctttacattataaaataccttacgaatattttattacctttcaatgcagtagaacactaactggctccttgcaacactttgtcgtcctgacattaatttggggaaattcccagccattattatttcaaatatttcttttgcttttttctcttctccttctggtgttcctattgtacatatgttacaccatttgtagttgtcctacagtccctggatattttgtactgtttttgtccccagtatttgttctctttgctttttagtttttaagtttctattgctgtatcctcatgctcagagattctttcctcaactgtgtccagtctactaagaagcccatcaaagtcattctttatttctgttatggtgtttttgatatctagcatttctatttcattctttcttaggatttccatctgtttgcttacattgtccatgtgttcttggatgctatctcctttatccattagagcccttggcatgttaatcacagttgttttaaattcctggtctgataattccaatatccctgccatatttggttctgatgcttgctctgtcttttcaaatgatgtttttgtcttttggtatggtttataattttttggcagttggatgtgatgtatcaggtaagtaagccccttgtagtgtggggtaagctgtggggagcaggaaagcaatctatagtcatatacttaggtctcagtcctttagtgagtctatgcctttgaactgtgaacttcagaagtctttctcagtttttttcttcccttttaggtggaacagaatggctagagtgggatggagttgggtatttccttccccccaggtcagttagtttctgatgataccctagggggttagactctgattaattagtttattccggggaagatcttgttaagaacagaattccccggcctatttcaaaatggttccctttaccctccccctgatggaaacatgaggggatttttctcttaggcttactgtgggaacttggttgagctcctgagacccctaaagtttttaattatctggcttgtcagcgctgagtccccagtaattagtcaattacagttcaggtgttcctccacagcactagttcccatggcagtttctgctcatgagcatgtcctgggaagccatgattccctgtatttgcctctgtctccagtcttgtggatagcagtttgccttgtgtcttcccctctattatggatccaaaaagagttgttgattgttcactctgttcagctttttacttgttttgagaatggagttttgacttctaagatccttacctgcaagaccggaaaccagaagttcctgtgttaagaacagactgtagaagatgaaaggatggagtattatttttctagagatgccacaacatactaccacaaacagagtggcttaagccaatagaaatgtattctctcacaattctggaggccagaagtaagacatcaaggtgtcagcagggccatgctctctctctgaaaactctagaggagaatccttccttgcatcttccagctctggtggcttctggcattccttggcttgtggaagcacaactccagtctctgcctccctcttcacatggcctttccccatgtatcagtgtctctgtccaaatcaccctctccttgctcttagaaagacaccatttattggatttaggatccaccctagatcaagaatgattcagtcatgggattcttaactaaccacatctgcaaagactccatttccaaacaaggtcacattaataagtgtgtgtgtgcgggtggtagggctcaaatatatctttttgagggatacagttcaacccactacagcattaagtaaccaaattaaattttaagtgagcagtggcagggcttatgatgacagtgtatatatgaagatttggtgtatgtttctatgagagagattatgagattcgctgatggatttcatttggagtgtgacaaagaacagcatcaaaaatgacttcgacttttaacttgacataggatgaataggacttttgatctgacataggatgaatttactgatctagaaagatgcaagttttggggggagaggactatgaagactttccccaattactttaataatatagcatagaatttaagagcaacacctctggaggcaaatagacctgggctcacaaataatgttaacataccttggggtattttacttaatctccctgggtcttgggattcccatttgcaaaatgggcataataaaaataatacctctctcataatattattggaatgatttcacatgattatgcatgtgagctattaatagtcagtggcaaacaggcagtacttcccctgtaaatcttatctattcatctcattttgaaaggagcctacagagatttggaaggccccttcaaatgcaccattcttttattctgacatcactttggtggattaggaagactgatgtggcagcagcatatagattagactggggtgggaagagaaggaggcagggaacctactaagttgtccattgagagatgtcagtggcatgagaatagtggggaaagagaaaacagagaggacgttattgagggaactgcacaggacctggcaaatgatgcactgtgagaaaagataaagatgtctgactttctaactctggaaagttggaacacagtaactgatgaaagtggcaaagtggaagtgtagagtaaccttgggatgagaaaggggaaggagcatattcagtttagactcaccagattgaagtactgacagtataagaaattaggcaccaagtagaatcatggcatgcagtaagtgctccatatctgaatggttggtagatctaggtcagtactgtccaatagacatatgagagccacaaatgtaagccatgggtcatttaaattttcctagtagccatattaaaaaaagtagaatgaaactaattttgataatatgttttatttaacctaatataaccaaaatactttcattccaatatgtaattgccataaaatattgattatgttatattctttttttcaggctaagtttttgaaatcccatatgtattttatacccacagcacatcccaatttgtactagccatatctcgagtgctcactagctgctgtattggatagtataattctaggtggaggtgattgtcaggcagtagattatgataactgcacttcgaaagacaggcatcaatctaaaatcacctgtatggaagaggaaaccaggtaataggatgaactttgtaagagagagaatactaaaagagaagggaacctaagatagaatgggggaacaattcattttgcaaaggtttggtttttccattagactgcccagcccctgaaaagaggtgaattagtaatagtgattcaatgcatgtttttaacatatggacctcttggttttttaattctactatttgcaagcatcttgttcatgtatttgtttattgtccatctcctcattaccataatgtaaatctgttttgctcacaattatatttccagaataacatctctcacacattagtgctcagtaaatgcctgtgagataaaagtctaatctctaccttcagaaaatttacaatatgatgggtaaaaaaccattacatagaggaaaaatatactaatgatagattcatagagaattagattcctgatgaatgatattgctaaggttgggtccaggagttcaacagagagaaagagtcattgattttggaggagcctagaaatacagaattgaaacatggtctatgccttaaatgatggctagcctttgaatgtatgggaagcaaggggaagctttccaagtagggtgaatgacttatgcaaaggtgtggtgcatgtgaatattttagttgcaatagctattaagaaaaagaaagatatcaaattgaaaatggtggccactgaagtttttcataaggtatgccaagcaaaactttaaaaatgctatatcaaatggattgagagaggagtactggtgagcagccattgcaattgtccagaaggcaataaaggttggactaataagagtgatgcctttgggggtaggaggaggaaagatataagagatgtttgaataatggccttggcatattttgatctctatttttaaaaagaggctgttatttagcataaatgaccttgaaggatgacctaatgagcactggatgtttgaatgtgttgctgaggaaaactccaaggttctgaacttggttgactgaattatggtgccatagacagaaagttccaaatagcaaattgcttttagaggtgaagactagagaggaaaatgggttgaagtcaaagtgttggaagatatccacgtggaaatttccagtaagccttcagatgactaagggattcagagaatgtaggctctttccaaatcttctgttctttttgcctatatagaaagtgtttactttatgtgtttccttgtggctctgttgattacatttttatgtgtggtttggagctcctctggcttcagacctgtatttgttttgggcatagttggagtagagtgctaacaagctcaaggtcataggtttgatccccaaaagggccagttagtttcatggagaggaaaattgcattccatggttcacagacttgacccctaatcctgtctgcttgtctcaaaactatctagcattggtcccaagagggcccagtgagaaagtgtgagcagttgtgtgcgcaatctatttaaactactggaagaataactccaagtgggtttatctagttgcttcttcaggaagttttgtctgccctccttcctcaactcttgggacagagatcaccttttcagagacaacaccatgaacaaatgcacatgaaactgtcatgctcatgtctgcctgcatctgcgttcctatgttcatttacttctcaagcaaagggcagtgtgagcacccaggagcgtatagttctttggtacaagtgtctacttgtaagtattggagtattatcagtttgactttgagaactggcttaccagtgttgtacaaaaaagccctagagagcatgaatgtgcccaaaagactctctaagcaaacctttccccaacagattttccttatcagactgcttttgcttgcttcgtacttttactgggaaatataagtcaacacagaattcttgtcaattggtcatacaaggatacagcatagaattctcagtgttcttgagaagaatgctggtatccataaaacaactcctaaacaaacccacagaaggcatcttccacacaagtacagagttaccagcacctgctgggatggcatctaaaatctgtttttttggatactgcattttcaaaaatcagtcttagaggttctcaaattgctttttcagttaacagatataccctgggtcctacaagagttaccctgaagaggacttggaataatgctatgcacacactgaaagattcaaaataaatcttcatggcttaaaaaggacttgaaaattattttcaagttcacttctctttcagggaattggagattgctacaccagggatatttctcttatttggcattatggaaaattttggaggctgagaagtaagagaccagaccatcaaatcttatttcattgatttctaagactaatagtgatgtcttaaaagaatatgttatggaataaatatgactaaaagtaaaaggcagaataaaattatatgctgatgaatccagcaaaactggttgaaaaattcttagtgtttggtttgtacacagacaagcaacatacttatttgcattgttccttcaaattgattacattgaagataaattattttaacattataaagggacagcctgaaaatatcaaataagtagttaaaaattattacatgaaaactttgcatgtctgctggctgggctgggctggagtgaagaaagataaagaattatgacacagtaagaaaatgttagacttgaaatttttacatctgcattgtggtgcaaggatctgcactagcactttttacctgatttttctggtcagagtcaaattagggggaaatgtggtcagtgtcagaaatgttgagaccatgagttaagagtatatatagaaaacggtgtgacacacaccgggacctgtcaagggctggggggctgggggagggacagcattaggagaaacacctaatgtagatgatgggttgataggtgcagtaaaccaccatggcacgtgtatacctatgtaacaaggctgcacgttctgcacatgtaccccagaacttaaagtataattaaaaataaaaaataaaaaaaagaaagaaaatgatgtgacaaagccaatggagagaattctactttggctatcttagatccttaattaatactctcattcttaataatagcagaagtaatgataataaaagtaatagtaaaaataccagaaaccacacaaaacaagagctgataagcagacaagtgctggactatgccagtggtttcatctagccacagaaaaattaaaaaagatgaaaaaaattaaattaatgatgagttttctataaagcttaatttacacaattaaagaatctgcccttttttcttagattatattcttgccatgtttttaaaaaattaattcattttcagtgatacaatggtgatgatagatgatttttttatttccttattttaggcaaataaagattttgacacctcaggttgatttttctcaatttctacttttattttttgaaatttcaatattttgagaaatctagaagtttaggaactgttgtatgataatgtttaatccttaaataataatttgaggcagatattgctgttattatcaaaataagaggaaactaaaccccacagaagtcattttaatttgtccaaagcacatattagaacatgacacaagcccacatctgcctgatttcagcacttgtttcttactactatgtaattcctgtttgtactagttagggcctagtaaggagagcagaaacccttctagaccaggcattttaaacagagaggattcttttttttttttttttttttaagacatctcgctctgttgcctagactgggctgctgggctggaaagcagtggcgtgatcacagctcattgcagccttgacctcctaggatcaagtgatcatcccacctcagcctcttgagtagctgggactacaggagcgcaccatcacacccagcttttttaaaatttatttatttatttttatttttaggagagataaggtctcactctgttacccatgctggtctccaactcctggaatcaagcgatcctcctgccttgacccccaaaggtgctgggattataggtgtgagccactgtgcacattcaacagagaggatttaatacagatgatggaagagatgagtagctaaataagggaggggagtcaacccagaaaaaacaacatcctaaaatcactaccatccctatggctagagatactcagagaggggaaaaaccatctgcatggatctaggtccactaggggaacagaatgctgcttgcactgggaggaaggggttatggagccaagagctgcaagtactgctgaagacgctgttggaggcaaagagaaaagggggataatacctggcttctcccttcttcttgtcttttgtcttttgctaatgcctcctattggccaaacttacccagaaaccagagctcataggtgctgagaaatgtggctcattgtgaaaacgagcaaatcaagggaatgttgggaaatggatatgagagcagacaagtaatcagccagcacattctagcacaaatctgtattaagttattccactgtaccttttactatagcagtgaggtctagagataccagaggacgcttttcaatattaactatctaagagaatctacttggtgatagttgacagatgaggatgtctctatttccaattcatctttaaagcagagtgaggcagaagaaataaaaagaaatttggctctggggtagccttatttttgagtattttagatcatataagggtggctgaatttgaagctctgaactaaataggatggagaagcacaatcctgggtcgtgtttctttcttactgttttctccttccctctctccaggaacaatcacctcccacctctgtttcccttttagagatttgggtttgggaaagacagttccatattcatggggtggagtgatagcttcagcgatagcacgtgtatagggacatttctatgatccctgttatcccctacatgtccatttgaagggagagaccctactcagggttctttctgaaggaggtttgcacctaagcaggaaccactgaattaaataagtgaggtggagttagaaaattatagcacagttactcaatttttaaatctcctcttaaaaggaaaacctccctaccaggccacatttcctactttacttgtagttcaaagtcaaattttacttttgatgtactgctgcaattgtctcaaatccaatttacatctgctcctgtttttagtgattgttttattcttttacaagccatctcattccatcacagggcgaagaaaagaacatttagaaaccagatgttgtattaactataaccattatcctttatgggatcccagaggtttaatctctatccataaacaggtgaggaagataccagctttcagctgagctttacagttaggatgcttcactgagaagggggcgaaggctctgccatccatctgtcattatgactcggggaggctcataatggatgggtatagcccagcagtttcaaccctatcagacccaaagctctcctttttataacatatattttatgatctaccctttaatgtccctaagtgaaattcacagataatatcaacatacacaattttaacaaaaagcaaaatgatgcctgaactgtacataaagtagaaataaaaggaaaaaagtttgtaataaaataacatgcattacaagatagaatgcttaggcacaactctcctagaaaacacacggaagtggtcagatgtttatactcgtggagaatcacgcatgggacagctgcatgtgcggactgatgcagatgtggagtggaaagattcaaacagcacaattagcattgccactgatgatgtgattttctaaaacagtgaaaaagacttggtaaagttctaccttttcttaatttgtatggtaattgcatccctgaagaagtcggtttatgttaaaattgtgcaaaaacactttgagtttataaaaattggagttatattccggacttaggtgattataaacaggattatctcctacttgaaatgtctggagacctggtccatacccaataaatgtcagaaatgctctccccagtcattgcaacagtgccaaatgtctcccaaattatctaggaccagcaccactccaccctttgggaatgcttgtgtgggctgtctaagaccactttggagggcagggatatgggaatgtttgtctcatggaactctaggctctaagtccacagtttttctccagaagccctgattcaaccatagcacttgagactacctcaacttcaataagctgtcaagagaaaaatagttggattgttgccagaggtcttggtaagattctttataatcagcttccagtttcacttaggtgggaatggtttattcctagactgtgtaagagccaatacataactttcttcatggaggtatcccgagattggctctatatccctgggtgttacctgcatagcatgaagtactatccagaactgacatgcacatgtggaagaacggcagtggggaatgacacattattagatacattggttaccgtgcagaaatgcttctttatcctgataatatcatactcaataataggtcatcactcaaaggtgccattagccatgtgtctgcctgtagcgtgtaaagccaattttgaacaagaaagtatcagtcagtattctgagctgtcctcatgcctggattgggtgtaagtggtggagtagtaaaagcaagtgtcttcagacccagatttgatgtcctcagacccagattcaagccttctctgctggtctgtgaccttcagtaaactaagtaatgtctttgagcctccatttccttatcagtcagtgtttacaatagtgcctgatgcataggcttgttggaaggatgaatgagataatataggtaaaccacttggcataatgactgactcacagtaagtgctcagtaaatattaaccacccttattgttggagtggtggtaattatctccaataaagatcttacagaagaaaaagatgttcttttaaaaaaagaggctgttatttgacgtagatgacctggaaggaagatagaattcctcttagggatagaattggtatttcctttaggaaagaacaccttttgtacatattcagtaacaaaaggtgagccagccctgcccccacccccaccactggcaaagctgggatggggaaagattgccctgcataagaatacaatataattttcttataagttctttccaaaggaggggataaagggtttgatagaaagtggttcctgggagagtttgcagaagagtggaaaagatcttgctaagatgacaggaggcacatgagccaccagaaattccttggattcatagtaatagtgatgtttgccattgaaatggaaggtattttctgtcctgtgcttaactcatccccttttcattgtttacaaaatctttagtgaaaggctgtggctagatcaccctagtgtgaatgaaaggagagagggattgtctggagtggagcgaggggagaagtagtacagaacaccatgactataggaggcaaaatgctaagagcatgaacaagacatttggaggaagaaggggcccgcataatgttagtcccagggagattcttggacattttgagggagcaaaggtaggaatgaacgtgagatgggacaccaatggcacgtgagaaaatattaaagaaaactttactataatttccttaaaactaagtacaaaacttgtgagactttttttatatttgggtaactttccaaatagttaatgaatttttaaaaaatgaaatgagatgcttttaaacgagggagattaccaatctttataccttgtacttctataaatgctgttgtgaatttgatattcacagtatctattcagtaaaaaattggaacgatttattgaaacaaaaactcaatgctgagagatcacattcttataaatctcttggtatgggaatgtattagatgccatttatatattatgtgccttatttgatacgtgtgaaccttctggcaatagaatattttcccaaccactttgtgtcagggattataagtcactgttgggtgacagtgaggggattttacgtacaactgctttattgttaatgcatatattgtacaattcatacatctcttacatagcttttgcaagtcctttgaaacatatttacttttaaatagaatctgtaaattctatgagatgtcttcatttttgtgtgtgattagttttgtttttctgggtatgttttcatgtttatttattgcaatgaccttaataaaaatggtatataacagtagaattcttaaggaatgacacattacaccaacattatccaaaagaactaattaatcaaacatgactaattttaatgtaattactaaagaaagatataccattttattatgacactctagccatacattttcaaaatatgcttattaaacagtaaatgtaagataatgattcaattagttacatttttagaagtcattaggattgatattcctctgccataagtgaattgaataataatttcaaatacaatcagaattaatttaataaaaaatatgcttttcaactaagacagatgtaacgaatggccagtcattattttctggtttcaaagtagcaggggaaattaattcagtgtctgtaagtttatttatcacacttggcctataagtgtgataaaaatacatgaggcaaaatacatgatgtaatcccaattctcatagttcattaactcttttaccaaaaagatctgacatggtatttggggcctttatgtaaactgaatataagctgcgtgatatttgaaaggttttgatattttgaatagacattttcatgatacacagacacagataaaagatgtaagtagacagcttgaggtttcagagtccctcctgcagtgtgtttagcagcgggtacaagataaatatccaaacaaaatcagattaagggattaacagaagtgactttgctatgagttggtgagtggggtcaatgggtggcttgaaagggattttagagctctgtttttatttttcctactttacatcagtgcattttgggcaaaataaaatgagtaatgtttacttttaggcctcagtaatataaaaaaaggcagattctaaggattgtggaaggtcatgtttttgaaagtgaaaggtaattcagctccggttattaggagaaactctgtctccatcttaactcatatttcagttgagcagtaacatttggttttgtgtcctctctttttttttttttactttaaaaaagcttggatttttttccccttgaaagaccccatcaaagatagttgaagaatgaggagagaaggatcatgtttaagatccatgtaatcatacattaagagggaacacatgggcagggtgtggtggctcatgcctgtaatcccagcaatttgggaggctgaggcgggcaaatcacaaggtcaggagtttgagaccaacctggccaacatggtaaaaccccgtctctattaaaaatccaaaaaattagccgggcatagtggtgggtgcctgtaatcccagctactcaggaggctgaggcaggagaatcgcttaaacccaggaggtggaggttgcagtgagccgagatcatgccactgcactccagcctgggggacagtgcgagaccccatctcacaaaaaggaaaaaaaaaaagagggaacacgtgaaatatatgttttcagtgaggttcctttaattctagagtttcagcttggtcagccctctataaaattctgaggcagatactaaaataataagggctgggttgggatgggggcagaataaagacagcttcaaaaatcccctgggcctctgtcttatctgtgagaggtttctttaaaaaacaaaagcattgttccagataggaattggttatttaaattgatatctttatcctgtaccatatgcacttaaagcttctgacagtcttctctcttttttaaatagaaattacacaaaaaagatatctatgtatcactttctaatacctaacaggaaggtcttataaaatattaaaatagcaataagcaaatatgtactacaggattaaacactagcattgaaaacaaaacaaaatccaaaaccaagaatcaacaacattttccttttgttgttgcccccctaccagatctggactttatggtctttgcaagggaggggcataaactttcacaattcttctgttttaaaataaatgatgccattgcataaatcagatttatcttttgaaaatattggtggaaagccatgtgatttgaatggaaagattctttcttctgaggagagccaaacaggttctgctctaataaattagcacaatcttttaagattaaaaatagcaaaacattttaaatagtctgattatagcttcaacaagtcaaacatacatttctatctagcctatagttttaaagagtctatgtgggtttaacttattattcctcattctgatataaaaaaagaagaaaagaaccaagtcattttgaacattaagaaattcataaagactgtataaagtaaaaaaaaaaaaaaaacaaaaacaagaaacaaaaaatcttcacagattgttagccatctctttcaacaatttctcataaattctttctttatcagtagataacccccatctcataaggaaatactttccaacatttcccaaatgagatcagtgattgcttttcatgagagctactgctctttgagatgtctgggtgaagggagaatgtcttctataaaccagtaaatgccaaagaatacccaagggggatttggcagaagctattttttgcaggtaaatctatgtattttttctctttgttcttattttctccacttgctgaatatctgttttagagcagagtgcacaaaaatcaataaggaacttacttatcttttaaattcttctatttgcctataagatcttttttcccgcgtttattctccatgctcttgatcaagttcagaagattggataatatattgctaattttgctaagtttgagagccaacaaaacaatggagccttctaactttaaaaaatttccaactcctgcccctgcacccccaaattcacaatttggtgaacagtacactacttgtgagtgataaaaagttgaaaggtggtggtggctagatagacctaatgctattttattaagccatctatctatagaattgttgtttttatactttaaaaaaatatgtctatgctttcttttttttctttttttcttttttttttagtcaagtactttcttaaagaaacaatagcaccacattggcatagctggccaaacaataaatgggaaagcaaaatgtgctacatcttttattctaagccttctcccaagtgcataaaatagtaacagaaaccctggagccacagagcatgagatggtttcatctacacaaacattgacgttccaaggagaggaaggattctcaagggtggacaggctttttgtttgtttgtttgttttttaataaaattttcaaggaagtgatttcttttcagtattccattggatccttagggtgaatgtgtgtgtgtgtgtgtgtgtgtgtgtgtgtgtgtgtgtctgtgtatgtagggtgggtgttaagagattttcatatccctagaagagtggattctgatggagagctgcattaactttttcaggggaactgcctcatcttaaaaagttcaaataatactttaatattatttggggaagagagaacagaaatttgacctaagtatccagtatggtcaattaaattggaaataagcctatgagttgaaagctcattcttaccaatgtttactgttcttttacaaatatcttgaaattgcctcattcaagaattataaagcaatctaattctgaagcaaagcttgtaaagttttgggttgtgacattttggttgctcctttctatgaaatctgagtcattctgctgtagtatatagtaatcaactgacttccagggtttgcatcaatttgttttctagttttaattcattaaaaaataaaatagtgaattggtataatgagttattttcaatttatttataatccagttggagaggattatgtgttggaaaaagttaagaaagataatatggcagtgcatctttcagctttcctccttgggggatttttgactgtggatagaattaagtgaaggaaataagtcatagacactcttagaattatcacatctaactatgacagaaaacacgttaagtctgcagaagactgcctataaagttttgttgagagggaataattttaaaaggtacacactggggacaagaaataaaaagaagtgccatcttgggaagaggagtccagtatcttattccacagaacctgtatgtctggaaaacaggcagagggcaaaaatgatgtatagtttcttttacatctgtccatagtgattagaacattgctaagcatgcttgaggtgctcaattcaaataatgttggactgagagttaaaatacttgttgactgaacaggattgctggctccactaaatggggccttctttttgcatatattcagagatccagggagtcttttttttttttttcctggcctctgatccttgaggtgacccagtgggagaaaaactgaagatgttatttttgtttttcatatagactttccaagaatgtaaaatatagaatttgcatgaaataatcaagcctgggtacttttaaccaaaaagttctaaggtgactagaaagatctgaatgctggataattcattgttctaatgagaaaatcttgatctgcagatagggatcattttctaggctatgatggactagtacactaaccagtggactttcttgataccaattttcagttgaatggataaaacacattcacagagagctaggggctacccttctgagcaggcatgggaaatttcttgttgtgatggaagtttttgcctttcaactggaaactctagtcaagcatattttaacaaacttttaaaaaaatgtatatacagctaagaataagagtaaagtttgttaaagaagataactttgtgactttttattagatattattttaatatttcaaattttggatcactttccttatattgcctagaaaagaaggaatcattgtgtttttcaaaatgaatagaatattatttatagtattaaacgaggttttactagatatgtagtaactgcatagaagagtcagtgagtgctaacaaagagtaattaattcccctttcactggtagaaatctctttgtttttctcctttttcttttcctttctctcttttcacttatctttgtattcataaaaccaaatgcagaattcaaaatcaaattgaaaatcaaatgcttcccacatattttgaaaagtgttttaagagattgagctgttagcttttaacaactagttggccagttatttggatagcttcactgacaagaactgagatgtcaggagcattcaattcaccaatctctagctatgctatgaatgggttatttatagaattccttgcatctcagcaactcaagcgccctgatgttgcacccttacagcaacccagggtaaaaaaaatctgaatctttatctttttaaaccttataccacccctttgaggtaggtagatgacatattgcccccattttgcagatgaggaaactgaggcacagagaggtgaagtgacttgcccaaggtcacacagtggtgagtccatgacacagctggcagatgttcatttcttccatgagaaaaagaaaccaggactgctaaaattcctagccttctgctttttccattccacagtttcctctctggactcgccagtccaatttgcatcagtggacttttgtgtctgaagttcctcttggaaggcataactggggggactttgccttctttcccaaatggatggtgttttcagtacccttccccttgtgtcatctttggctccaggcttcccctattgttttgctttcacgtattaccgttttggccagactctttcatataacaaactacaaaatagcaccattatactaaaaaacagagttttacatactgtttgatatatcctgtataattgatatgctaaatttacatagtgctctatatggaaaaaataaaaagaggaaagttactaattaggttgcacattaactcatcatttgaaggaactcttttgagttgaagaaactttctatgtttaaaacatatgcctaaaaatgattggcctcaaagttgcaactatttgcattattcttttttgtaagcatgatgtggaaaaataaagctttgtgtctaaaataaaatgcatccaacttatatttggtacaaatgccacagatggaatcttgtgggttagaattggtgtgcttcttgacgacttgctgctgcttttgaggaggccaaattcggcaaatataaaggttatgaagggaggtggtgggtatagactaacaagattatcagacactgtaaaacaaacagcccgagttgtgtagaaagaagtgcaaataaggaaacaattcataaaccacttagacaaggttgctgaatgaatggctccagcagccaagattcagagaggaatttagtgcaactggatctatacaacacccatgcatttgtggctcttgagaggcagggactaagatatatatatatatatattttttttttcttttctatagaacattattgataaaagatcaacagcaatctaccaactccaggaccatttttgcaaggtgcaaatcactcctaaagacaatgttggaatgtttacttgtgtatttcattgggggaaacgcccatcttttaaatgttatcaaacttattttttggtaggtgttccaaagtttaacaggtaactcgtgcagagcaaaggatcctgcggtggcatgtcactcttcactcctcaggagggtcttcctacatcctgtagttcttgtttcctgcactccctctacttgcgttcttcaaatgtacttcctataaataaaggagaaaaagtgacattaa

SEQ ID NO: 11 - DNA, 70 bp, Homo sapiens
ggcacccacccgtagaaccgaccttgcggggccttcgccgcacacaagctcgtgtctgtgggtccgtgtc

SEQ ID NO: 12 - DNA, 106 bp, Homo sapiens
gcgcagcgccctgtctcccagcctgaggtgcagtgctgcatctctggtcagttgggagtctgagatgaagcactgtagctcaggaagagagaagttgttctgcagc

SEQ ID NO: 13 - DNA, 69 bp, Homo sapiens
cagagtgtagcttaacacaaagcacccaacttacacttaggagatttcaacttaacttgaccgctctga

SEQ ID NO: 14 - DNA, 112 bp, Homo sapiens
ggggcaaagatgactaaaacacttttcctgccctcgaggagctcacagtctagtatgtctcatcccctactagactgaagctccttgaggacagggatggtcatactcacct

SEQ ID NO: 15 - DNA, 113 bp, Homo sapiens
gccaacggctggacagcgggcaacggaatcccaaaagcagctgttgtctccagagcattccagctgcgcttggatttcgtcccctgctctcctgcctgagcagcgccctggcc

SEQ ID NO: 16 - DNA, 150 bp, Homo sapiens
aactcttagcggtggatcactccactcctgcattgatgaagaatgcagccagctgtgagaattaatgtgagttgcaggacacactgatcatcatttcaaatgcacttgtgactccgtgttcctcccagggctacacctgtctgagtcatc

SEQ ID NO: 17 - DNA, 59 bp, Homo sapiens
gagaaagctcacaagaactgctaactcatgcccccatgtctaacaacatggctttctca

SEQ ID NO: 18 - DNA, 110 bp, Homo sapiens
gaactttggccacctggcactgagaactgaattccataggctgtgagctctagcaatgccctgtggactcagttctggtgcccggcagtgctacaacatcaatgccaagg

SEQ ID NO: 19 - DNA, 110 bp, Homo sapiens
tgaacatccaggtctggggcatgaacctggcatacaatgtagatttctgtgttcgttaggcaacagctacattgtctgctgggtttcaggctacctggaaacatgttctc

SEQ ID NO: 20 - DNA, 66 bp, Homo sapiens
ggtaaaatggctgagtgaagcattggactgtaaatctaaagacaggggttaggcctctttttacca

SEQ ID NO: 21 - DNA, 1559 bp, Homo sapiens
  misc_feature (1437)..(1437): n is a, c, g, or t
gctaaacctagccccaaacccactccaccttactaccagacaaccttagccaaaccatttacccaaataaagtataggcgatagaaattgaaacctggcgcaatagatatagtaccgcaagggaaagatgaaaaattataaccaagcataatatagcaaggactaacccctataccttctgcataatgaattaactagaaataactttgcaaggagagccaaagctaagacccccgaaaccagacgagctacctaagaacagctaaaagagcacacccgtctatgtagcaaaatagtgggaagatttataggtagaggcgacaaacctaccgagcctggtgatagctggttgtccaagatagaatcttagttcaactttaaatttgcccacagaaccctctaaatccccttgtaaatttaactgttagtccaaagaggaacagctctttggacactaggaaaaaaccttgtagagagagtaaaaaatttaacacccatagtaggcctaaaagcagccaccaattaagaaagcgttcaagctcaacacccactacctaaaaaatcccaaacatataactgaactcctcacacccaattggaccaatctatcaccctatagaagaactaatgttagtataagtaacatgaaaacattctcctccgcataagcctgcgtcagattaaaacactgaactgacaattaacagcccaatatctacaatcaaccaacaagtcattattaccctcactgtcaacccaacacaggcatgctcataaggaaaggttaaaaaaagtaaaaggaactcggcaaatcttaccccgcctgtttaccaaaaacatcacctctagcatcaccagtattagaggcaccgcctgcccagtgacacatgtttaacggccgcggtaccctaaccgtgcaaaggtagcataatcacttgttccttaaatagggacctgtatgaatggctccacgagggttcagctgtctcttacttttaaccagtgaaattgacctgcccgtgaagaggcgggcataacacagcaagacgagaagaccctatggagctttaatttattaatgcaaacagtacctaacaaacccacaggtcctaaactaccaaacctgcattaaaaatttcggttggggcgacctcggagcagaacccaacctccgagcagtacatgctaagacttcaccagtcaaagcgaactactatactcaattgatccaataacttgaccaacggaacaagttaccctagggataacagcgcaatcctattctagagtccatatcaacaatagggtttacgacctcgatgttggatcaggacatcccgatggtgcagccgctattaaaggttcgtttgttcaacgattaaagtcctacgtgatctgagttcagaccggagtaatccaggtcggtttctatctacnttcaaattcctccctgtacgaaaggacaagagaaataaggcctacttcacaaagcgccttcccccgtaaatgatatcatctcaacttagtattatacccacacccacccaagaacagggttt

SEQ ID NO: 22 - DNA, 111 bp, Homo sapiens
ccttttgcctgattccaggctgaggtagtagtttgtacagtttgagggtctatgataccacccggtacaggagataactgtacaggccactgccttgccaggaacagcgcg

SEQ ID NO: 23 - DNA, 2082 bp, Homo sapiens
atgggttgggcattaggaacggcctggccccacaaatcacacaactggggtgtagaacaaaatggttccacagatgacaccaggctggtccagggccgatgcaggccagaaccccgctgggaggactccccagaacaggcactgagctgaggaaaggcaggacacgtggtctgctaccgaccccaccagatcttgctgggactctgggcagctccggagtaagagcagcatgctctgcaacgaagagctaggtccaaggaccgcaggcggaggcaggaagtgtcaagatcccaggttacggaatggcaccaagtcggtaaccaaaggaagcaacaacccgggtgttcaaggcagtcgtgcaaggcggcgcgggggcgaggccgaggccactccctcccacttccttgacgctatttcctgggaggagccggagctcgcggcccggagccaagagattcccagcccagtgctccaaaatactcggcctgggggaggctggtccgtgagcgtgcgcccggaccgttccgccatgcatagtggacccagcactacagcaagcctggcacgacctctaaggcggttcgcggcaacgtccgcacgtcggctcgttggtctaggggtatgattctcgcttcgggtgcgagaggtcccgggttcaaatcccggacgagccctcctttaccttttactgagacaagagtgtcttcaaggaataggttacctgaccagcgctgcaggaggcttgactgtaagtcatcaatgtacagtaagctcttttgtggcaccgcggtagcagaaagcatctcaatccccagacccgcctggcatgtcaggaagagacgaggcacgcccagacttgggcaggtccctccctttctgcttcctgacttccttcctggtgtctcaactcggccaccacagcctggtttcgctttgattgacacgcgtcaatctatagttgtggatgacagtgttcgggagagcccaggaactgtcaaaacttggttctctgcagtcctgaaggcactctgtctctttcggtcactccatctgacgattggtgcctgaaatacacctacggtttctggtcagcgtttatcagtggttggaagaacagaacccctaggaaccctgctgtcagcacgcagagtgtaaagtctcagatcaaggattcggagaaaggtctctacaggtccctcctcgttagtatagtggttggttgggatgagtcgggttggacccgtgcggatccaggaaaacagcgatcgaggtaaaagtaatggctgccgtcgtctgcccagcgcgcaattgtgagtgaccttcaccgctagcgcgcgccacccaccccacatgaacctgtagggttatgcccagtctacagacgaggaaaccaagatccagggaagctgagtcaccggcagagctgggattacgtctaagatttgtccagggggcgagaactgcagcgacaccatgatttatcatctccagaaaacaaaaaaaaaggcctagacacataaaaatggcttctctgtagagtgagctcaacgagctcaatgtgattccagttaaggaattgggccttaagccaaatgcgcctaaacgcaacttgcctctctattatttatccagaggatgaatttaattcctacgtacatgcgcccacatctcgtcagctggtgcctcagagaaatgcgctgacaaatcttaaaggtggggcttcatgacaaaagtccgcccgttattgctgctcaacagacccatcaagtcacgctgttggacaggcctcgtggcgcaacggtagcgcgtctgactccagatcagaaggttgcgtgttcaaatcacgtcggggtcaaacaaaacattgttttccctaatcaaatagacctacggtgacatttttcaggataggaaaaaaaaaaagcctcctcagtagaaggataggaggggaatgagacaaatatgaacgttattcagaagttgggtgcagactttcaacattatgtgatatatccctgtggcaaaactgcgcatgtatccctaaggtctataaaagtaaaaataaatttaaaaataaaaaaa

SEQ ID NO: 24 - DNA, 112 bp, Homo sapiens
tctccatcctccctggggcatcctgtactgagctgccccgaggcccttcatgctgcccagctcggggcagctcagtacaggatacctcggggtgggagtcagcaggaggtga

SEQ ID NO: 25 - DNA, 2265 bp, Homo sapiens
tgggttaggcattttctgtgcattacctcgttcatccttactacaaccttattaaatagatgtcatcacttctgtatttgcattttacaggcgaggacacaggcttaactcctcaaggccacggagctgacctttgttagtagcttgagcaagtggggtctgaagcacacgtgcctgcacctggcctcagaagtgggactgacacgaggtttcggttaccatggacctctgtgacctccatgaccaatctaggttctggaaggggtggttgggaagccagaatagtcacagcaagtggaacagggctaggtggagaccagcgagcctacgacaagaggctttaggtcatagagggaggttttagtagatgagttttatcagtgggcttcgcccacctcttcctaacatctgaccagctgggctattagttttagaaggctgagctgaggcctgggtgggccaagacatacttccacagattgtcttcatcccactagccaaggtggttgaggacatcaatgaccttcaaagggaattaacaagtcaaaggaaatggtgtcctaggtgtcacaaatggatggcttaatcctgataccagggacaggacatatttgctacatacaaaggattatatgtaacaaaaatattggatgtggagtgtgatttaacaaaccccatggactcatcacttagcccaagaaatggagcatcaggagtaacttgctttttacctgtgttcttttccccatccactcctttgcctcctcccatgaggaagcaatattttatttagtttggcttggattggatttttatatactttgtcatgtatgtattatacctttaaacaataaatattgtttagatttgcctggttttgagctctgtaaaaatggtatcatatgtagttttctggaacttgctttttatattattattgttatttttagagacagggtcttgctgtatcacccaggctggaacttagtgacaggatcatggctcactgcagccttgacctcccaggctcaagtgatcctctcgtttcagcctcccgagtagctgggactacatgcatgtgccacaacactccactaattttttaaatttttagtagagacaaggtcttgctatgttgcccaggcttggaacttgcttttaaacaactcgtcattatgtttctaacattcacccacgttcccgtgtgggactttgttcttccattttcactgttgtatgacatcctactgtgctattgtacagtaggatctgtacaattgatctattctctgtcaattatgtgtggatttcttccccagtttttggatactctggctactgccgctatgaatattcttatgcatgtcctcttgtacatgtcttgtacatatgtgtaagagtttctcataggtatacacccaggagtacaattgctggctgtagggtttgttcagctttgggagtaaatgctaaattgttttccaaaatggttgtagcagttatacattactggtgagagggtaaagaatttttgttgaaatacatgcccttcaactgttcacacttaaaaatttttgccactctgttgggtatgaaatgatatctcattagggtctgaatttgtattttcctggttactaagtaggttgagcttcttttcatatgtgcattgactgtgctgcttttgtaaaatgaccattttggtgggggctgtattgttctatagggttaactttttcttcttgatatgtaagctttcttttatattttatatattatatactaaccctttgttagattatttgtcttcattccttatggtttttttttttttttttttttgagacagagtttcgctcttgttgcccaggctggagtgcaatggtgcggtctcggctcactgcaacctgcgcctcccgggttcatgtgattctcctacctcagcctcccgagtagttgggattacaggcatgcgccaccacacccagcaattttgtatttttagtagacacagggtttctccatgttggtcaggctggtctcaaactcccgacctcaggtgatccgcccacctcggcctcccaaagtgctgggattacaggcatgagccaccgcgcctggcctctcaattttttaaggtcgttaatatttttcaataaagttaaaaagttttctgtattaggatttggtacatcttttgttatatttagtctaaaataatctgtagtatttattgttattataaatggtgtctcttaaaagtta